European Patent Application EP 4 293 125 A2, published December 20, 2023. Title: METHODS FOR TARGETED GENOMIC ANALYSIS. Applicant: Resolution Bioscience, Inc. The sequence listing filed with the application follows.

SEQUENCE LISTING (810 sequences)

SEQ ID NO: 1 - DNA, 24 bp, synthetic construct
  misc_feature 1..24: note = Adaptor sequence - tag, sample code and universal amplification sequence
  source 1..24: mol_type = other DNA
gaccagagaattcgaatacaaaac

SEQ ID NO: 2 - DNA, 24 bp, synthetic construct
  misc_feature 1..24: note = Adaptor sequence - tag, sample code and universal amplification sequence
  source 1..24: mol_type = other DNA
gaccagagaattcgaatacaacac

SEQ ID NO: 3 - DNA, 24 bp, synthetic construct
  misc_feature 1..24: note = Adaptor sequence - tag, sample code and universal amplification sequence
  source 1..24: mol_type = other DNA
gaccagagaattcgaatacaagac

SEQ ID NO: 4 - DNA, 24 bp, synthetic construct
  misc_feature 1..24: note = Adaptor sequence - tag, sample code and universal amplification sequence
  source 1..24: mol_type = other DNA
gaccagagaattcgaatacaatac

SEQ ID NO: 5 - DNA, 24 bp, synthetic construct
  misc_feature 1..24: note = Adaptor sequence - tag, sample code and universal amplification sequence
  source 1..24: mol_type = other DNA
gaccagagaattcgaatacacaac

SEQ ID NO: 6 - DNA, 24 bp, synthetic construct
  misc_feature 1..24: note = Adaptor sequence - tag, sample code and universal amplification sequence
  source 1..24: mol_type = other DNA
gaccagagaattcgaatacaccac

SEQ ID NO: 7 - DNA, 24 bp, synthetic construct
  misc_feature 1..24: note = Adaptor sequence - tag, sample code and universal amplification sequence
  source 1..24: mol_type = other DNA
gaccagagaattcgaatacacgac

SEQ ID NO: 8 - DNA, 24 bp, synthetic construct
  misc_feature 1..24: note = Adaptor sequence - tag, sample code and universal amplification sequence
  source 1..24: mol_type = other DNA
gaccagagaattcgaatacactac

SEQ ID NO: 9 - DNA, 24 bp, synthetic construct
  misc_feature 1..24: note = Adaptor sequence - tag, sample code and universal amplification sequence
  source 1..24: mol_type = other DNA
gaccagagaattcgaatacagaac

SEQ ID NO: 10 - DNA, 24 bp, synthetic construct
  misc_feature 1..24: note = Adaptor sequence - tag, sample code and universal amplification sequence
  source 1..24: mol_type = other DNA
gaccagagaattcgaatacagcac

SEQ ID NO: 11 - DNA, 24 bp, synthetic construct
  misc_feature 1..24: note = Adaptor sequence - tag, sample code and universal amplification sequence
  source 1..24: mol_type = other DNA
gaccagagaattcgaatacaggac

SEQ ID NO: 12 - DNA, 24 bp, synthetic construct
  misc_feature 1..24: note = Adaptor sequence - tag, sample code and universal amplification sequence
  source 1..24: mol_type = other DNA
gaccagagaattcgaatacagtac

SEQ ID NO: 13 - DNA, 24 bp, synthetic construct
  misc_feature 1..24: note = Adaptor sequence - tag, sample code and universal amplification sequence
  source 1..24: mol_type = other DNA
gaccagagaattcgaatacataac

SEQ ID NO: 14 - DNA, 24 bp, synthetic construct
  misc_feature 1..24: note = Adaptor sequence - tag, sample code and universal amplification sequence
  source 1..24: mol_type = other DNA
gaccagagaattcgaatacatcac

SEQ ID NO: 15 - DNA, 24 bp, synthetic construct
  misc_feature 1..24: note = Adaptor sequence - tag, sample code and universal amplification sequence
  source 1..24: mol_type = other DNA
gaccagagaattcgaatacatgac

SEQ ID NO: 16 - DNA, 24 bp, synthetic construct
  misc_feature 1..24: note = Adaptor sequence - tag, sample code and universal amplification sequence
  source 1..24: mol_type = other DNA
gaccagagaattcgaatacattac

SEQ ID NO: 17 - DNA, 24 bp, synthetic construct
  misc_feature 1..24: note = Adaptor sequence - tag, sample code and universal amplification sequence
  source 1..24: mol_type = other DNA
gaccagagaattcgaatacaaaga

SEQ ID NO: 18 - DNA, 24 bp, synthetic construct
  misc_feature 1..24: note = Adaptor sequence - tag, sample code and universal amplification sequence
  source 1..24: mol_type = other DNA
gaccagagaattcgaatacaacga

SEQ ID NO: 19 - DNA, 24 bp, synthetic construct
  misc_feature 1..24: note = Adaptor sequence - tag, sample code and universal amplification sequence
  source 1..24: mol_type = other DNA
gaccagagaattcgaatacaagga

SEQ ID NO: 20 - DNA, 24 bp, synthetic construct
  misc_feature 1..24: note = Adaptor sequence - tag, sample code and universal amplification sequence
  source 1..24: mol_type = other DNA
gaccagagaattcgaatacaatga

SEQ ID NO: 21 - DNA, 24 bp, synthetic construct
  misc_feature 1..24: note = Adaptor sequence - tag, sample code and universal amplification sequence
  source 1..24: mol_type = other DNA
gaccagagaattcgaatacacaga

SEQ ID NO: 22 - DNA, 24 bp, synthetic construct
  misc_feature 1..24: note = Adaptor sequence - tag, sample code and universal amplification sequence
  source 1..24: mol_type = other DNA
gaccagagaattcgaatacaccga

SEQ ID NO: 23 - DNA, 24 bp, synthetic construct
  misc_feature 1..24: note = Adaptor sequence - tag, sample code and universal amplification sequence
  source 1..24: mol_type = other DNA
gaccagagaattcgaatacacgga

SEQ ID NO: 24 - DNA, 24 bp, synthetic construct
  misc_feature 1..24: note = Adaptor sequence - tag, sample code and universal amplification sequence
  source 1..24: mol_type = other DNA
gaccagagaattcgaatacactga

SEQ ID NO: 25 - DNA, 24 bp, synthetic construct
  misc_feature 1..24: note = Adaptor sequence - tag, sample code and universal amplification sequence
  source 1..24: mol_type = other DNA
gaccagagaattcgaatacagaga

SEQ ID NO: 26 - DNA, 24 bp, synthetic construct
  misc_feature 1..24: note = Adaptor sequence - tag, sample code and universal amplification sequence
  source 1..24: mol_type = other DNA
gaccagagaattcgaatacagcga

SEQ ID NO: 27 - DNA, 24 bp, synthetic construct
  misc_feature 1..24: note = Adaptor sequence - tag, sample code and universal amplification sequence
  source 1..24: mol_type = other DNA
gaccagagaattcgaatacaggga

SEQ ID NO: 28 - DNA, 24 bp, synthetic construct
  misc_feature 1..24: note = Adaptor sequence - tag, sample code and universal amplification sequence
  source 1..24: mol_type = other DNA
gaccagagaattcgaatacagtga

SEQ ID NO: 29 - DNA, 24 bp, synthetic construct
  misc_feature 1..24: note = Adaptor sequence - tag, sample code and universal amplification sequence
  source 1..24: mol_type = other DNA
gaccagagaattcgaatacataga

SEQ ID NO: 30 - DNA, 24 bp, synthetic construct
  misc_feature 1..24: note = Adaptor sequence - tag, sample code and universal amplification sequence
  source 1..24: mol_type = other DNA
gaccagagaattcgaatacatcga

SEQ ID NO: 31 - DNA, 24 bp, synthetic construct
  misc_feature 1..24: note = Adaptor sequence - tag, sample code and universal amplification sequence
  source 1..24: mol_type = other DNA
gaccagagaattcgaatacatgga

SEQ ID NO: 32 - DNA, 24 bp, synthetic construct
  misc_feature 1..24: note = Adaptor sequence - tag, sample code and universal amplification sequence
  source 1..24: mol_type = other DNA
gaccagagaattcgaatacattga

SEQ ID NO: 33 - DNA, 24 bp, synthetic construct
  misc_feature 1..24: note = Adaptor sequence - tag, sample code and universal amplification sequence
  source 1..24: mol_type = other DNA
gaccagagaattcgaatacaaact

SEQ ID NO: 34 - DNA, 24 bp, synthetic construct
  misc_feature 1..24: note = Adaptor sequence - tag, sample code and universal amplification sequence
  source 1..24: mol_type = other DNA
gaccagagaattcgaatacaacct

SEQ ID NO: 35 - DNA, 24 bp, synthetic construct
  misc_feature 1..24: note = Adaptor sequence - tag, sample code and universal amplification sequence
  source 1..24: mol_type = other DNA
gaccagagaattcgaatacaagct

SEQ ID NO: 36 - DNA, 24 bp, synthetic construct
  misc_feature 1..24: note = Adaptor sequence - tag, sample code and universal amplification sequence
  source 1..24: mol_type = other DNA
gaccagagaattcgaatacaatct

SEQ ID NO: 37 - DNA, 24 bp, synthetic construct
  misc_feature 1..24: note = Adaptor sequence - tag, sample code and universal amplification sequence
  source 1..24: mol_type = other DNA
gaccagagaattcgaatacacact

SEQ ID NO: 38 - DNA, 24 bp, synthetic construct
  misc_feature 1..24: note = Adaptor sequence - tag, sample code and universal amplification sequence
  source 1..24: mol_type = other DNA
gaccagagaattcgaatacaccct

SEQ ID NO: 39 - DNA, 24 bp, synthetic construct
  misc_feature 1..24: note = Adaptor sequence - tag, sample code and universal amplification sequence
  source 1..24: mol_type = other DNA
gaccagagaattcgaatacacgct

SEQ ID NO: 40 - DNA, 24 bp, synthetic construct
  misc_feature 1..24: note = Adaptor sequence - tag, sample code and universal amplification sequence
  source 1..24: mol_type = other DNA
gaccagagaattcgaatacactct

SEQ ID NO: 41 - DNA, 24 bp, synthetic construct
  misc_feature 1..24: note = Adaptor sequence - tag, sample code and universal amplification sequence
  source 1..24: mol_type = other DNA
gaccagagaattcgaatacagact

SEQ ID NO: 42 - DNA, 24 bp, synthetic construct
  misc_feature 1..24: note = Adaptor sequence - tag, sample code and universal amplification sequence
  source 1..24: mol_type = other DNA
gaccagagaattcgaatacagcct

SEQ ID NO: 43 - DNA, 24 bp, synthetic construct
  misc_feature 1..24: note = Adaptor sequence - tag, sample code and universal amplification sequence
  source 1..24: mol_type = other DNA
gaccagagaattcgaatacaggct

SEQ ID NO: 44 - DNA, 24 bp, synthetic construct
  misc_feature 1..24: note = Adaptor sequence - tag, sample code and universal amplification sequence
  source 1..24: mol_type = other DNA
gaccagagaattcgaatacagtct

SEQ ID NO: 45 - DNA, 24 bp, synthetic construct
  misc_feature 1..24: note = Adaptor sequence - tag, sample code and universal amplification sequence
  source 1..24: mol_type = other DNA
gaccagagaattcgaatacatact

SEQ ID NO: 46 - DNA, 24 bp, synthetic construct
  misc_feature 1..24: note = Adaptor sequence - tag, sample code and universal amplification sequence
  source 1..24: mol_type = other DNA
gaccagagaattcgaatacatcct

SEQ ID NO: 47 - DNA, 24 bp, synthetic construct
  misc_feature 1..24: note = Adaptor sequence - tag, sample code and universal amplification sequence
  source 1..24: mol_type = other DNA
gaccagagaattcgaatacatgct

SEQ ID NO: 48 - DNA, 24 bp, synthetic construct
  misc_feature 1..24: note = Adaptor sequence - tag, sample code and universal amplification sequence
  source 1..24: mol_type = other DNA
gaccagagaattcgaatacattct

SEQ ID NO: 49 - DNA, 24 bp, synthetic construct
  misc_feature 1..24: note = Adaptor sequence - tag, sample code and universal amplification sequence
  source 1..24: mol_type = other DNA
gaccagagaattcgaatacaaatg

SEQ ID NO: 50 - DNA, 24 bp, synthetic construct
  misc_feature 1..24: note = Adaptor sequence - tag, sample code and universal amplification sequence
  source 1..24: mol_type = other DNA
gaccagagaattcgaatacaactg

SEQ ID NO: 51 - DNA, 24 bp, synthetic construct
  misc_feature 1..24: note = Adaptor sequence - tag, sample code and universal amplification sequence
  source 1..24: mol_type = other DNA
gaccagagaattcgaatacaagtg

SEQ ID NO: 52 - DNA, 24 bp, synthetic construct
  misc_feature 1..24: note = Adaptor sequence - tag, sample code and universal amplification sequence
  source 1..24: mol_type = other DNA
gaccagagaattcgaatacaattg

SEQ ID NO: 53 - DNA, 24 bp, synthetic construct
  misc_feature 1..24: note = Adaptor sequence - tag, sample code and universal amplification sequence
  source 1..24: mol_type = other DNA
gaccagagaattcgaatacacatg

SEQ ID NO: 54 - DNA, 24 bp, synthetic construct
  misc_feature 1..24: note = Adaptor sequence - tag, sample code and universal amplification sequence
  source 1..24: mol_type = other DNA
gaccagagaattcgaatacacctg

SEQ ID NO: 55 - DNA, 24 bp, synthetic construct
  misc_feature 1..24: note = Adaptor sequence - tag, sample code and universal amplification sequence
  source 1..24: mol_type = other DNA
gaccagagaattcgaatacacgtg

SEQ ID NO: 56 - DNA, 24 bp, synthetic construct
  misc_feature 1..24: note = Adaptor sequence - tag, sample code and universal amplification sequence
  source 1..24: mol_type = other DNA
gaccagagaattcgaatacacttg

SEQ ID NO: 57 - DNA, 24 bp, synthetic construct
  misc_feature 1..24: note = Adaptor sequence - tag, sample code and universal amplification sequence
  source 1..24: mol_type = other DNA
gaccagagaattcgaatacagatg

SEQ ID NO: 58 - DNA, 24 bp, synthetic construct
  misc_feature 1..24: note = Adaptor sequence - tag, sample code and universal amplification sequence
  source 1..24: mol_type = other DNA
gaccagagaattcgaatacagctg

SEQ ID NO: 59 - DNA, 24 bp, synthetic construct
  misc_feature 1..24: note = Adaptor sequence - tag, sample code and universal amplification sequence
  source 1..24: mol_type = other DNA
gaccagagaattcgaatacaggtg

SEQ ID NO: 60 - DNA, 24 bp, synthetic construct
  misc_feature 1..24: note = Adaptor sequence - tag, sample code and universal amplification sequence
  source 1..24: mol_type = other DNA
gaccagagaattcgaatacagttg

SEQ ID NO: 61 - DNA, 24 bp, synthetic construct
  misc_feature 1..24: note = Adaptor sequence - tag, sample code and universal amplification sequence
  source 1..24: mol_type = other DNA
gaccagagaattcgaatacatatg

SEQ ID NO: 62 - DNA, 24 bp, synthetic construct
  misc_feature 1..24: note = Adaptor sequence - tag, sample code and universal amplification sequence
  source 1..24: mol_type = other DNA
gaccagagaattcgaatacatctg

SEQ ID NO: 63 - DNA, 24 bp, synthetic construct
  misc_feature 1..24: note = Adaptor sequence - tag, sample code and universal amplification sequence
  source 1..24: mol_type = other DNA
gaccagagaattcgaatacatgtg

SEQ ID NO: 64 - DNA, 24 bp, synthetic construct
  misc_feature 1..24: note = Adaptor sequence - tag, sample code and universal amplification sequence
  source 1..24: mol_type = other DNA
gaccagagaattcgaatacatttg

SEQ ID NO: 65 - DNA, 20 bp, synthetic construct
  misc_feature 1..20: note = Primer
  source 1..20: mol_type = other DNA
aatgatacggcgaccaccga

SEQ ID NO: 66 - DNA, 29 bp, synthetic construct
  misc_feature 1..29: note = Primer
  source 1..29: mol_type = other DNA
aatgatacggcgaccaccgagatctacac

SEQ ID NO: 67 - DNA, 25 bp, synthetic construct
  misc_feature 1..25: note = Primer
  source 1..25: mol_type = other DNA
tgcaggaccagagaattcgaataca

SEQ ID NO: 68 - DNA, 33 bp, synthetic construct
  misc_feature 1..33: note = Primer
  source 1..33: mol_type = other DNA
acacgtcatgcaggaccagagaattcgaataca

SEQ ID NO: 69 - DNA, 58 bp, synthetic construct
  misc_feature 1..58: note = Primer
  source 1..58: mol_type = other DNA
aatgatacggcgaccaccgagatctacacgtcatgcaggaccagagaattcgaataca

SEQ ID NO: 70 - DNA, 20 bp, synthetic construct
  misc_feature 1..20: note = Primer
  source 1..20: mol_type = other DNA
caagcagaagacggcatacg

SEQ ID NO: 71 - DNA, 24 bp, synthetic construct
  misc_feature 1..24: note = Primer
  source 1..24: mol_type = other DNA
caagcagaagacggcatacgagat

SEQ ID NO: 72 - DNA, 25 bp, synthetic construct
  misc_feature 1..25: note = Primer
  source 1..25: mol_type = other DNA
cacgggagttgatcctggttttcac

SEQ ID NO: 73 - DNA, 33 bp, synthetic construct
  misc_feature 1..33: note = Primer
  source 1..33: mol_type = other DNA
gtgactggcacgggagttgatcctggttttcac

SEQ ID NO: 74 - DNA, 57 bp, synthetic construct
  misc_feature 1..57: note = Primer
  source 1..57: mol_type = other DNA
caagcagaagacggcatacgagatgtgactggcacgggagttgatcctggttttcac

SEQ ID NO: 75 - DNA, 15 bp, synthetic construct
  misc_feature 1..15: note = Adapter sequence - partner strand for SEQ ID NO:23
  source 1..15: mol_type = other DNA
tccgtgtattcgaat

SEQ ID NO: 76 - DNA, 20 bp, synthetic construct
  misc_feature 1..20: note = Primer
  source 1..20: mol_type = other DNA
gaccagagaattcgaataca

SEQ ID NO: 77 - DNA, 25 bp, synthetic construct
  misc_feature 1..25: note = Primer
  source 1..25: mol_type = other DNA
tgcaggaccagagaattcgaataca

SEQ ID NO: 78 - DNA, 57 bp, synthetic construct
  misc_feature 1..57: note = Primer
  source 1..57: mol_type = other DNA
aatgatacggcgaccaccgagatcacacgtcatgcaggaccagagaattcgaataca

SEQ ID NO: 79 - DNA, 24 bp, synthetic construct
  misc_feature 1..24: note = Primer
  source 1..24: mol_type = other DNA
ttagagtgctgtgcaagatgtctg

SEQ ID NO: 80 - DNA, 22 bp, synthetic construct
  misc_feature 1..22: note = Primer
  source 1..22: mol_type = other DNA
accccaagaaacacaatccagt

SEQ ID NO: 81 - DNA, 22 bp, synthetic construct
  misc_feature 1..22: note = Primer
  source 1..22: mol_type = other DNA
gccactggattgtgtttctttg

SEQ ID NO: 82 - DNA, 24 bp, synthetic construct
  misc_feature 1..24: note = Primer
  source 1..24: mol_type = other DNA
tcaattagcttttctgtgccagtg

SEQ ID NO: 83 - DNA, 22 bp, synthetic construct
  misc_feature 1..22: note = Primer
  source 1..22: mol_type = other DNA
actgttctgtggctgtggacat

SEQ ID NO: 84 - DNA, 27 bp, synthetic construct
  misc_feature 1..27: note = Primer
  source 1..27: mol_type = other DNA
tcttggtagtttttggagaaataggtc

SEQ ID NO: 85 - DNA, 24 bp, synthetic construct
  misc_feature 1..24: note = Primer
  source 1..24: mol_type = other DNA
ttcttcttccccaggcttgttaga

SEQ ID NO: 86 - DNA, 24 bp, synthetic construct
  misc_feature 1..24: note = Primer
  source 1..24: mol_type = other DNA
caccccaaagaaacacaatccagt

SEQ ID NO: 87 - DNA, 23 bp, synthetic construct
  misc_feature 1..23: note = Primer
  source 1..23: mol_type = other DNA
ccctcatggcacagaaaagctaa

SEQ ID NO: 88 - DNA, 24 bp, synthetic construct
  misc_feature 1..24: note = Primer
  source 1..24: mol_type = other DNA
tgggagggcaggtacttacacatt

SEQ ID NO: 89 - DNA, 25 bp, synthetic construct
  misc_feature 1..25: note = Primer
  source 1..25: mol_type = other DNA
ccccttgttttcttacacgtgttct

SEQ ID NO: 90 - DNA, 24 bp, synthetic construct
  misc_feature 1..24: note = Primer
  source 1..24: mol_type = other DNA
cctcccttggcttctccataccta

SEQ ID NO: 91 - DNA, 24 bp, synthetic construct
  misc_feature 1..24: note = Primer
  source 1..24: mol_type = other DNA
gtgtgtcattgtttcccaaaatgg

SEQ ID NO: 92 - DNA, 24 bp, synthetic construct
  misc_feature 1..24: note = Primer
  source 1..24: mol_type = other DNA
caccccttgttattgccacaaaat

SEQ ID NO: 93 - DNA, 24 bp, synthetic construct
  misc_feature 1..24: note = Primer
  source 1..24: mol_type = other DNA
taccagccaagcccatactagagg

SEQ ID NO: 94 - DNA, 24 bp, synthetic construct
  misc_feature 1..24: note = Primer
  source 1..24: mol_type = other DNA
gggatcaacagtggcataattgaa

SEQ ID NO: 95 - DNA, 400 bp, Homo sapiens
  source 1..400: mol_type = unassigned DNA
agtgcccactatctccgagcctgtgagcacagggcctggcagaggggtttgagtggcatgagctacctactggatgtgcctgactgtttccccttcttcttccccaggcttgttagagtgctgtgcaagatgtctggtaggggccccctttgcttccctggtggccactggattgtgtttctttggggtggcactgttctgtggctgtggacatgaagccctcactggcacagaaaagctaattgagacctatttctccaaaaactaccaagactatgagtatctcatcaatgtgtaagtacctgccctcccacacagacccatcttttttttccctctctccatcctggagatagagaactcttcagtaccttagtaactagcaggggactggggtgga

SEQ ID NO: 96 - DNA, 399 bp, Homo sapiens
  source 1..399: mol_type = unassigned DNA
tccaccccagtcccctgctagttactaaggtactgaagagttctctatctccaggatggagagagggaaaaaaaagatgggtctgtgtgggagggcaggtacttacacattgatgagatactcatagtcttggtagtttttggagaaataggtctcaattagcttttctgtgccagtgagggcttcatgtccacagccacagaacagtgccaccccaaagaaacacaatccagtggccaccagggaagcaaagggggcccctaccagacatcttgcacagcactctaacaagcctggggaagaagaaggggaaacagtcaggcacatccagtaggtagctcatgccactcaaacccctctgccaggccctgtgctcacaggctcggagatagtgggcac

SEQ ID NO: 97 - DNA, 400 bp, Homo sapiens; identical to SEQ ID NO: 95
  source 1..400: mol_type = unassigned DNA

SEQ ID NO: 98 - DNA, 400 bp, Homo sapiens; identical to SEQ ID NO: 95
  source 1..400: mol_type = unassigned DNA

SEQ ID NO: 99 - DNA, 400 bp, Homo sapiens; identical to SEQ ID NO: 95
  source 1..400: mol_type = unassigned DNA

SEQ ID NO: 100 - DNA, 400 bp, Homo sapiens; identical to SEQ ID NO: 95
  source 1..400: mol_type = unassigned DNA

SEQ ID NO: 101 - DNA, 400 bp, Homo sapiens; identical to SEQ ID NO: 95
  source 1..400: mol_type = unassigned DNA

SEQ ID NO: 102 - DNA, 100 bp, Homo sapiens
  source 1..100: mol_type = unassigned DNA
ccccttgttttcttacacgtgttctgacttctgctaggtgtggttcatattgcccaagttggagcctccagcgtagtaggtatggagaagccaagggagg

SEQ ID NO: 103 - DNA, 81 bp, Homo sapiens
  source 1..81: mol_type = unassigned DNA
gtgtgtcattgtttgggaaaatggctaggacatcccgacaaggtgatcatcctcaggattttgtggcaataacaaggggtg

SEQ ID NO: 104 - DNA, 96 bp, Homo sapiens
  source 1..96: mol_type = unassigned DNA
taccagccaagcccatactagaggctgtccccagatgctagcaaccatctgattgaataaccatctgtatcattcaattatgccactgttgatccc

SEQ ID NO: 105 - DNA, 34 bp, synthetic construct
  misc_feature 1..34: note = 34 nt binding site of universal oligonucleotide
  modified_base 34: mod_base = OTHER; note = dideoxycytosine
  misc_feature 34: note = n is a, c, g, or t
  source 1..34: mol_type = other DNA
cactggactatgtagtacctcactcagcaatacn

SEQ ID NO: 106 - DNA, 34 bp, synthetic construct
  misc_feature 1..34: note = 34 nt binding site of universal oligonucleotide
  modified_base 34: mod_base = OTHER; note = dideoxycytosine
  misc_feature 34: note = n is a, c, g, or t
  source 1..34: mol_type = other DNA
ggcaacgaacggactggaatctacggtcaccaan

SEQ ID NO: 107 - DNA, 400 bp, Homo sapiens; identical to SEQ ID NO: 95
  source 1..400: mol_type = unassigned DNA

SEQ ID NO: 108 - DNA, 114 bp, synthetic construct
  misc_feature 1..114: note = Ultramer targeted to PLP1 exon 2
  source 1..114: mol_type = other DNA
gagttgatcctggttttcactttgagtggcatgagctacctactggatgtgcctgactgtttccccttcttcttccccagggtattgctgagtgaggtactacatagtccagtg

SEQ ID NO: 109 - DNA, 114 bp, synthetic construct
  misc_feature 1..114: note = Ultramer targeted to PLP1 exon 2
  source 1..114: mol_type = other DNA
gagttgatcctggttttcacatgtctggtaggggccccctttgcttccctggtggccactggattgtgtttctttggggtggtattgctgagtgaggtactacatagtccagtg

SEQ ID NO: 110 - DNA, 114 bp, synthetic construct
  misc_feature 1..114: note = Ultramer targeted to PLP1 exon 2
  source 1..114: mol_type = other DNA
gagttgatcctggttttcaccttggtagtttttggagaaataggtctcaattagcttttctgtgccagtgagggcttcatggtattgctgagtgaggtactacatagtccagtg

SEQ ID NO: 111 - DNA, 114 bp, synthetic construct
  misc_feature 1..114: note = Ultramer targeted to PLP1 exon 2
  source 1..114: mol_type = other DNA
gagttgatcctggttttcacatctccaggatggagagagggaaaaaaaagatgggtctgtgtgggagggcaggtacttacggtattgctgagtgaggtactacatagtccagtg

SEQ ID NO: 112 - DNA, 114 bp, synthetic construct
  misc_feature 1..114: note = Ultramer targeted to PLP1 exon 2
  source 1..114: mol_type = other DNA
gagttgatcctggttttcactttgagtggcatgagctacctactggatgtgcctgactgtttccccttcttcttccccaggttggtgaccgtagattccagtccgttcgttgcc

SEQ ID NO: 113 - DNA, 114 bp, synthetic construct
  misc_feature 1..114: note = Ultramer targeted to PLP1 exon 2
  source 1..114: mol_type = other DNA
gagttgatcctggttttcacatgtctggtaggggccccctttgcttccctggtggccactggattgtgtttctttggggtgttggtgaccgtagattccagtccgttcgttgcc

SEQ ID NO: 114 - DNA, 114 bp, synthetic construct
  misc_feature 1..114: note = Ultramer targeted to PLP1 exon 2
  source 1..114: mol_type = other DNA
gagttgatcctggttttcaccttggtagtttttggagaaataggtctcaattagcttttctgtgccagtgagggcttcatgttggtgaccgtagattccagtccgttcgttgcc

SEQ ID NO: 115 - DNA, 114 bp, synthetic construct
  misc_feature 1..114: note = Ultramer targeted to PLP1 exon 2
  source 1..114: mol_type = other DNA
gagttgatcctggttttcacatctccaggatggagagagggaaaaaaaagatgggtctgtgtgggagggcaggtacttacgttggtgaccgtagattccagtccgttcgttgcc

SEQ ID NO: 116 - DNA, 400 bp, Homo sapiens; identical to SEQ ID NO: 95
  source 1..400: mol_type = unassigned DNA

SEQ ID NO: 117 - DNA, 400 bp, Homo sapiens; identical to SEQ ID NO: 95
  source 1..400: mol_type = unassigned DNA

SEQ ID NO: 118 - DNA, 400 bp, Homo sapiens; identical to SEQ ID NO: 95
  source 1..400: mol_type = unassigned DNA

SEQ ID NO: 119 - DNA, 400 bp, Homo sapiens; identical to SEQ ID NO: 95
  source 1..400: mol_type = unassigned DNA

SEQ ID NO: 120 - DNA, 400 bp, Homo sapiens; identical to SEQ ID NO: 95
  source 1..400: mol_type = unassigned DNA

SEQ ID NO: 121 - DNA, 400 bp, Homo sapiens; identical to SEQ ID NO: 95
  source 1..400: mol_type = unassigned DNA

SEQ ID NO: 122 - DNA, 21 bp, synthetic construct
  misc_feature 1..21: note = Primer
  source 1..21: mol_type = other DNA
ggcttcgactgaacgtctcca

SEQ ID NO: 123 - DNA, 22 bp, synthetic construct
  misc_feature 1..22: note = Primer
  source 1..22: mol_type = other DNA
agtgctccatggctgctcagtt

SEQ ID NO: 124 - DNA, 25 bp, synthetic construct
  misc_feature 1..25: note = Primer
  source 1..25: mol_type = other DNA
gaaccagaggaacgctgtggtaact

SEQ ID NO: 125 - DNA, 23 bp, synthetic construct
  misc_feature 1..23: note = Primer
  source 1..23: mol_type = other DNA
gacgtgtgcctagatgcgttttc

SEQ ID NO: 126 - DNA, 25 bp, synthetic construct
  misc_feature 1..25: note = Primer
  source 1..25: mol_type = other DNA
tggctgaaaagtctccttgaaactg

SEQ ID NO: 127 - DNA, 25 bp, synthetic construct
  misc_feature 1..25: note = Primer
  source 1..25: mol_type = other DNA
ctcagtgggtctccttgagagaggt

SEQ ID NO: 128 - DNA, 25 bp, synthetic construct
  misc_feature 1..25: note = Primer
  source 1..25: mol_type = other DNA
ctttcctccagtcacaagccatcta

SEQ ID NO: 129 - DNA, 25 bp, synthetic construct
  misc_feature 1..25: note = Primer
  source 1..25: mol_type = other DNA
catgctgatagaaagtcccctggta

SEQ ID NO: 130 - DNA, 25 bp, synthetic construct
  misc_feature 1..25: note = Primer
  source 1..25: mol_type = other DNA
ttttcacacagccaggagtcttttc

SEQ ID NO: 131 - DNA, 25 bp, synthetic construct
  misc_feature 1..25: note = Primer
  source 1..25: mol_type = other DNA
gggagatccgacaatacagattgaa

SEQ ID NO: 132 - DNA, 25 bp, synthetic construct
  misc_feature 1..25: note = Primer
  source 1..25: mol_type = other DNA
cctgtcttgtctttgctgatgtttc

SEQ ID NO: 133 - DNA, 25 bp, synthetic construct
  misc_feature 1..25: note = Primer
  source 1..25: mol_type = other DNA
acaaaacaggctcaggacttagcaa

SEQ ID NO: 134 - DNA, 25 bp, synthetic construct
  misc_feature 1..25: note = Primer
  source 1..25: mol_type = other DNA
caacgttagcttcaccaacaggaac

SEQ ID NO: 135 - DNA, 25 bp, synthetic construct
  misc_feature 1..25: note = Primer
  source 1..25: mol_type = other DNA
gctggtagaagttctcctcctcgtc

SEQ ID NO: 136 - DNA, 23 bp, synthetic construct
  misc_feature 1..23: note = Primer
  source 1..23: mol_type = other DNA
gtctgctccacctccagcttgta

SEQ ID NO: 137 - DNA, 24 bp, synthetic construct
  misc_feature 1..24: note = Primer
  source 1..24: mol_type = other DNA
gttgagagggtaggggaagaccac

SEQ ID NO: 138 - DNA, 25 bp, synthetic construct
  misc_feature 1..25: note = Primer
  source 1..25: mol_type = other DNA
gaaccagaggaacgctgtggtaact

SEQ ID NO: 139 - DNA, 23 bp, synthetic construct
  misc_feature 1..23: note = Primer
  source 1..23: mol_type = other DNA
gacgtgtgcctagatgcgttttc

SEQ ID NO: 140 - DNA, 25 bp, synthetic construct
  misc_feature 1..25: note = Primer
  source 1..25: mol_type = other DNA
cctgtcttgtctttgctgatgtttc

SEQ ID NO: 141 - DNA, 25 bp, synthetic construct
  misc_feature 1..25: note = Primer
  source 1..25: mol_type = other DNA
acaaaacaggctcaggacttagcaa

SEQ ID NO: 142 - DNA, 25 bp, synthetic construct
  misc_feature 1..25: note = Primer
  source 1..25: mol_type = other DNA
caacgttagcttcaccaacaggaac

SEQ ID NO: 143 - DNA, 25 bp, synthetic construct
  misc_feature 1..25: note = Primer
  source 1..25: mol_type = other DNA
gctggtagaagttctcctcctcgtc

SEQ ID NO: 144 - DNA, 23 bp, synthetic construct
  misc_feature 1..23: note = Primer
  source 1..23: mol_type = other DNA
gtctgctccacctccagcttgta

SEQ ID NO: 145 - DNA, 24 bp, synthetic construct
  misc_feature 1..24: note = Primer
  source 1..24: mol_type = other DNA
gttgagagggtaggggaagaccac

SEQ ID NO: 146 - DNA, 60 bp, Homo sapiens
  source 1..60: mol_type = unassigned DNA
agaattcattgccagctataaatctgtggaaacgctgccacacaatcttagcacacaaga

SEQ ID NO: 147 - DNA, 60 bp, Homo sapiens
  source 1..60: mol_type = unassigned DNA
taaatgacataacagttatgattttgcagaaaacagatctgtatttatttcagtgttact

SEQ ID NO: 148 - DNA, 60 bp, Homo sapiens
  source 1..60: mol_type = unassigned DNA
aggtttccgcaccaagacccctttaactcaagactgcctcccgctttgtgtgccccgctc

SEQ ID NO: 149 - DNA, 60 bp, Homo sapiens
  source 1..60: mol_type = unassigned DNA
agagcagagaatccgaggacggagagaaggcgctggagtcttgcgaggcgcaggacttgg

SEQ ID NO: 150 - DNA, 95 bp, Homo sapiens
  source 1..95: mol_type = unassigned DNA
atgtgactggcacgggagttgatcctggttttcacaagcacctagccccattcctgctgagcaggaggtggcaggtaccccagactgggaggtaa

SEQ ID NO: 151 - DNA, 95 bp, Homo sapiens
  source 1..95: mol_type = unassigned DNA
atgtgactggcacgggagttgatcctggttttcacagtcggtggggccaggatgaggcccagtctgttcacacatggctgctgcctctcagctct

SEQ ID NO: 152 - DNA, 95 bp, Homo sapiens
  source 1..95: mol_type = unassigned DNA
atgtgactggcacgggagttgatcctggttttcacacctgagtagcatcattgtagttctcgatatctccacttccagttttacatttaccatca

SEQ ID NO: 153 - DNA, 95 bp, Homo sapiens
  source 1..95: mol_type = unassigned DNA
atgtgactggcacgggagttgatcctggttttcaccctggccctcagccagtacagaaagtcatttgtcaaggccttcagttggcagacgtgctc

SEQ ID NO: 154 - DNA, 95 bp, Homo sapiens
  source 1..95: mol_type = unassigned DNA
atgtgactggcacgggagttgatcctggttttcacagaattcattgccagctataaatctgtggaaacgctgccacacaatcttagcacacaaga

SEQ ID NO: 155 - DNA, 95 bp, Homo sapiens
  source 1..95: mol_type = unassigned DNA
atgtgactggcacgggagttgatcctggttttcacgacttcaaagaaattacaagttgacatcttggactctacccctcgtactttatctcctat

SEQ ID NO: 156 - DNA, 95 bp, Homo sapiens
  source 1..95: mol_type = unassigned DNA
atgtgactggcacgggagttgatcctggttttcactctctttggggtcaagaaagaatccctagtggatttgggattctagaggaggtgttataa

SEQ ID NO: 157 - DNA, 95 bp, Homo sapiens
  source 1..95: mol_type = unassigned DNA
atgtgactggcacgggagttgatcctggttttcactgcgataccatgctgaagatgagctaacccaaccagccaagcaggcagggctgcgaagga

SEQ ID NO: 158 - DNA, 95 bp, Homo sapiens
  source 1..95: mol_type = unassigned DNA
atgtgactggcacgggagttgatcctggttttcacggggtaggtggaaaacccaagtaatgtgattttgtaacatccactgctgcatttgtttgc

SEQ ID NO: 159 - DNA, 95 bp, Homo sapiens
  source 1..95: mol_type = unassigned DNA
atgtgactggcacgggagttgatcctggttttcacttacttccctccagttttgttgcttgcaaaacaacagaatcttctctccatgaaatcatg

SEQ ID NO: 160 - DNA, 95 bp, Homo sapiens
  source 1..95: mol_type = unassigned DNA
atgtgactggcacgggagttgatcctggttttcaccaggggtatctattatccccattttctcacaaaggaaaccaagataaaaggtttaaatgg

SEQ ID NO: 161 - DNA, 95 bp, Homo sapiens
  source 1..95: mol_type = unassigned DNA
atgtgactggcacgggagttgatcctggttttcacgaaattctcttgtgaattcctgtgtcctcttgaatcttcaatgctaaagtttttgaaact

SEQ ID NO: 162 - DNA, 95 bp, Homo sapiens
  source 1..95: mol_type = unassigned DNA
atgtgactggcacgggagttgatcctggttttcacgggtttgagtggcatgagctacctactggatgtgcctgactgtttccccttcttcttccc

SEQ ID NO: 163 - DNA, 95 bp, Homo sapiens
  source 1..95: mol_type = unassigned DNA
atgtgactggcacgggagttgatcctggttttcacctatctccaggatggagagagggaaaaaaaagatgggtctgtgtgggagggcaggtactt

SEQ ID NO: 164 - DNA, 95 bp, Homo sapiens
  source 1..95: mol_type = unassigned DNA
atgtgactggcacgggagttgatcctggttttcacgaaagaagccaggtcttcaattaataagattccctggtctcgtttgtctacctgttaatg

SEQ ID NO: 165 - DNA, 95 bp, Homo sapiens
  source 1..95: mol_type = unassigned DNA
atgtgactggcacgggagttgatcctggttttcaccagactcgcgcccaattttcccccaccccttgttattgccacaaaatcctgaggatgatc

SEQ ID NO: 166 - DNA, 95 bp, Homo sapiens
  source 1..95: mol_type = unassigned DNA
atgtgactggcacgggagttgatcctggttttcactctttcttcttcctttatggggccctcctgctggctgagggcttctacaccaccggcgca

SEQ ID NO: 167 - DNA, 95 bp, Homo sapiens
  source 1..95: mol_type = unassigned DNA
atgtgactggcacgggagttgatcctggttttcacgtttgtgtttctacatctgcaggctgatgctgatttctaaccaccccatgtcaatcattt

SEQ ID NO: 168 - DNA, 95 bp, Homo sapiens
  source 1..95: mol_type = unassigned DNA
atgtgactggcacgggagttgatcctggttttcacaaccaaatatatagtgcttccatagtgggtaggagagccaaagcacccgtaccctaactc

SEQ ID NO: 169 - DNA, 95 bp, Homo sapiens
  source 1..95: mol_type = unassigned DNA
atgtgactggcacgggagttgatcctggttttcacagtctccatgtggccccgtaactccataaagcttaccctgcttgctttttgtgtcttact

SEQ ID NO: 170 - DNA, 95 bp, Homo sapiens
  source 1..95: mol_type = unassigned DNA
atgtgactggcacgggagttgatcctggttttcacccatgggtgtaatttgtatggtattagctactcccttgtaaaataacccaaataacccac

SEQ ID NO: 171 - DNA, 95 bp, Homo sapiens
  source 1..95: mol_type = unassigned DNA
atgtgactggcacgggagttgatcctggttttcactttacagtggagcatattactgctgttgcaagaaacagttcttcctctttcattttcctg

SEQ ID NO: 172 - DNA, 95 bp, Homo sapiens
  source 1..95: mol_type = unassigned DNA
atgtgactggcacgggagttgatcctggttttcacatagctgtacccacactatctcaggcctatttacttgccaagatcattcaaagtcaactc

SEQ ID NO: 173 - DNA, 95 bp, Homo sapiens
  source 1..95: mol_type = unassigned DNA
atgtgactggcacgggagttgatcctggttttcacgatttgaggagggagtgctttcttttctactctcattcacattctctcttctgttcccta

SEQ ID NO: 174 - DNA, 95 bp, Homo sapiens
  source 1..95: mol_type = unassigned DNA
atgtgactggcacgggagttgatcctggttttcaccagcattgtaggctgtgtggttagagcctcgctattagagaaagggggatttctacgggg

SEQ ID NO: 175 - DNA, 95 bp, Homo sapiens
  source 1..95: mol_type = unassigned DNA
atgtgactggcacgggagttgatcctggttttcactgttacctttaaaagacatctgctttctgccaaaattaatgtgctgaacttaaacttacc

SEQ ID NO: 176 - DNA, 95 bp, Homo sapiens
  source 1..95: mol_type = unassigned DNA
atgtgactggcacgggagttgatcctggttttcacttcccagtaaattactcttaccaatgcaacagactttaaagaagttgtgttttacaatgc

SEQ ID NO: 177 - DNA, 95 bp, Homo sapiens
  source 1..95: mol_type = unassigned DNA
atgtgactggcacgggagttgatcctggttttcactaaatgacataacagttatgattttgcagaaaacagatctgtatttatttcagtgttact

SEQ ID NO: 178 - DNA, 95 bp, Homo sapiens
  source 1..95: mol_type = unassigned DNA
atgtgactggcacgggagttgatcctggttttcacgacaggttttgaaagatatttgtgttactaatgactgtgctataacttttttttctttcc

SEQ ID NO: 179 - DNA, 95 bp, Homo sapiens
  source 1..95: mol_type = unassigned DNA
atgtgactggcacgggagttgatcctggttttcacactcaaaaaataaaaactataattactccttaatgtcagcttattatattcaatttaaac

SEQ ID NO: 180 - DNA, 95 bp, Homo sapiens
  source 1..95: mol_type = unassigned DNA
atgtgactggcacgggagttgatcctggttttcacaacaccttttttgaagtaaaaggtgcactgtaataatccagactgtgtttctcccttctc

SEQ ID NO: 181 - DNA, 95 bp, Homo sapiens
  source 1..95: mol_type = unassigned DNA
atgtgactggcacgggagttgatcctggttttcacgaaacctttatctgtatcaaagaatggtcctgcaccagtaatatgcatattaaaacaaga

SEQ ID NO: 182 - DNA, 95 bp, Homo sapiens
  source 1..95: mol_type = unassigned DNA
atgtgactggcacgggagttgatcctggttttcacgtgtattaaccttatgtgtgacatgttctaatatagtcacattttcattatttttattat

SEQ ID NO: 183 - DNA, 95 bp, Homo sapiens
  source 1..95: mol_type = unassigned DNA
atgtgactggcacgggagttgatcctggttttcacccccagccagcggtccgcaacccttgccgcatccacgaaactttgcccatagcagcgggc

SEQ ID NO: 184 - DNA, 95 bp, Homo sapiens
  source 1..95: mol_type = unassigned DNA
atgtgactggcacgggagttgatcctggttttcaccgactcatctcagcattaaagtgataaaaaaataaattaaaaggcaagtggacttcggtg

SEQ ID NO: 185 - DNA, 95 bp, Homo sapiens
  source 1..95: mol_type = unassigned DNA
atgtgactggcacgggagttgatcctggttttcacctgtggcgcgcactgcgcgctgcgccaggtttccgcaccaagacccctttaactcaagac

SEQ ID NO: 186 - DNA, 95 bp, Homo sapiens
  source 1..95: mol_type = unassigned DNA
atgtgactggcacgggagttgatcctggttttcacttctactgcgacgaggaggagaacttctaccagcagcagcagcagagcgagctgcagccc

SEQ ID NO: 187 - DNA, 95 bp, Homo sapiens
  source 1..95: mol_type = unassigned DNA
atgtgactggcacgggagttgatcctggttttcacaccgagctgctgggaggagacatggtgaaccagagtttcatctgcgacccggacgacgag

SEQ ID NO: 188 - DNA, 95 bp, Homo sapiens
  source 1..95: mol_type = unassigned DNA
atgtgactggcacgggagttgatcctggttttcacgccgccgcctcagagtgcatcgacccctcggtggtcttcccctaccctctcaacgacagc

SEQ ID NO: 189 - DNA, 95 bp, Homo sapiens
  source 1..95: mol_type = unassigned DNA
atgtgactggcacgggagttgatcctggttttcacggcggctaggggacaggggcggggtgggcagcagctcgaatttcttccagatatcctcgc

SEQ ID NO: 190 - DNA, 95 bp, Homo sapiens
  source 1..95: mol_type = unassigned DNA
atgtgactggcacgggagttgatcctggttttcacagacgagcttggcggcggccgagaagccgctccacatacagtcctggatgatgatgtttt

SEQ ID NO: 191 - DNA, 95 bp, Homo sapiens
  source 1..95: mol_type = unassigned DNA
atgtgactggcacgggagttgatcctggttttcacaggagagcagagaatccgaggacggagagaaggcgctggagtcttgcgaggcgcaggact

SEQ ID NO: 192 - DNA, 95 bp, Homo sapiens
  source 1..95: mol_type = unassigned DNA
atgtgactggcacgggagttgatcctggttttcactaagagtggcccgttaaataagctgccaatgaaaatgggaaaggtatccagccgcccact

SEQ ID NO: 193 - DNA, 95 bp, Homo sapiens
  source 1..95: mol_type = unassigned DNA
atgtgactggcacgggagttgatcctggttttcacttgtatttgtacagcattaatctggtaattgattattttaatgtaaccttgctaaaggag

SEQ ID NO: 194 - DNA, 95 bp, Homo sapiens
  source 1..95: mol_type = unassigned DNA
atgtgactggcacgggagttgatcctggttttcacgaggccacagcaaacctcctcacagcccactggtcctcaagaggtgccacgtctccacac

SEQ ID NO: 195 - DNA, 95 bp, Homo sapiens
  source 1..95: mol_type = unassigned DNA
atgtgactggcacgggagttgatcctggttttcacagaggaggaacgagctaaaacggagcttttttgccctgcgtgaccagatcccggagttgg

SEQ ID NO: 196 - DNA, 95 bp, Homo sapiens
  source 1..95: mol_type = unassigned DNA
atgtgactggcacgggagttgatcctggttttcactccaacttgaccctcttggcagcaggatagtccttccgagtggagggaggcgctgcgtag

SEQ ID NO: 197 - DNA, 95 bp, Homo sapiens
  source 1..95: mol_type = unassigned DNA
atgtgactggcacgggagttgatcctggttttcacgcttggacggacaggatgtatgctgtggcttttttaaggataactaccttgggggccttt

SEQ ID NO: 198 - DNA, 95 bp, Homo sapiens
  source 1..95: mol_type = unassigned DNA
atgtgactggcacgggagttgatcctggttttcacgcatttgatcatgcatttgaaacaagttcataggtgattgctcaggacatttctgttaga

SEQ ID NO: 199 - DNA, 46 bp, synthetic construct
  misc_feature 1..46: note = Primer
  source 1..46: mol_type = other DNA
aatgatacggcgaccaccgagatctacacgtcatgcaggaccagag

SEQ ID NO: 200 - DNA, 57 bp, synthetic construct
  misc_feature 1..57: note = Primer
  source 1..57: mol_type = other DNA
caagcagaagacggcatacgagatgtgactggcacgggagttgagaattcgaataca

SEQ ID NO: 201 - DNA, 60 bp, synthetic construct
  misc_feature 1..60: note = Oligonucleotide probe
  source 1..60: mol_type = other DNA
aagcacctagccccattcctgctgagcaggaggtggcaggtaccccagactgggaggtaa

SEQ ID NO: 202 - DNA, 60 bp, synthetic construct
  misc_feature 1..60: note = Oligonucleotide probe
  source 1..60: mol_type = other DNA
agtcggtggggccaggatgaggcccagtctgttcacacatggctgctgcctctcagctct

SEQ ID NO: 203 - DNA, 60 bp, synthetic construct
  misc_feature 1..60: note = Oligonucleotide probe
  source 1..60: mol_type = other DNA
acctgagtagcatcattgtagttctcgatatctccacttccagttttacatttaccatca

SEQ ID NO: 204 - DNA, 60 bp, synthetic construct
  misc_feature 1..60: note = Oligonucleotide probe
  source 1..60: mol_type = other DNA
cctggccctcagccagtacagaaagtcatttgtcaaggccttcagttggcagacgtgctc

SEQ ID NO: 205 - DNA, 60 bp, synthetic construct; identical to SEQ ID NO: 146
  misc_feature 1..60: note = Oligonucleotide probe
  source 1..60: mol_type = other DNA

SEQ ID NO: 206 - DNA, 60 bp, synthetic construct
  misc_feature 1..60: note = Oligonucleotide probe
  source 1..60: mol_type = other DNA
gacttcaaagaaattacaagttgacatcttggactctacccctcgtactttatctcctat

SEQ ID NO: 207 - DNA, 60 bp, synthetic construct
  misc_feature 1..60: note = Oligonucleotide probe
  source 1..60: mol_type = other DNA
tctctttggggtcaagaaagaatccctagtggatttgggattctagaggaggtgttataa

SEQ ID NO: 208 - DNA, 60 bp, synthetic construct
  misc_feature 1..60: note = Oligonucleotide probe
  source 1..60: mol_type = other DNA
tgcgataccatgctgaagatgagctaacccaaccagccaagcaggcagggctgcgaagga

SEQ ID NO: 209 - DNA, 60 bp, synthetic construct
  misc_feature 1..60: note = Oligonucleotide probe
  source 1..60: mol_type = other DNA
ggggtaggtggaaaacccaagtaatgtgattttgtaacatccactgctgcatttgtttgc

SEQ ID NO: 210 - DNA, 60 bp, synthetic construct
  misc_feature 1..60: note = Oligonucleotide probe
  source 1..60: mol_type = other DNA
ttacttccctccagttttgttgcttgcaaaacaacagaatcttctctccatgaaatcatg

SEQ ID NO: 211 - DNA, 60 bp, synthetic construct
  misc_feature 1..60: note = Oligonucleotide probe
  source 1..60: mol_type = other DNA
caggggtatctattatccccattttctcacaaaggaaaccaagataaaaggtttaaatgg

SEQ ID NO: 212 - DNA, 60 bp, synthetic construct
  misc_feature 1..60: note = Oligonucleotide probe
  source 1..60: mol_type = other DNA
gaaattctcttgtgaattcctgtgtcctcttgaatcttcaatgctaaagtttttgaaact

SEQ ID NO: 213 - DNA, 60 bp, synthetic construct
  misc_feature 1..60: note = Oligonucleotide probe
  source 1..60: mol_type = other DNA
gggtttgagtggcatgagctacctactggatgtgcctgactgtttccccttcttcttccc

SEQ ID NO: 214 - DNA, 60 bp, synthetic construct
  misc_feature 1..60: note = Oligonucleotide probe
  source 1..60: mol_type = other DNA
ctatctccaggatggagagagggaaaaaaaagatgggtctgtgtgggagggcaggtactt

SEQ ID NO: 215 - DNA, 60 bp, synthetic construct
  misc_feature 1..60: note = Oligonucleotide probe
  source 1..60: mol_type = other DNA
gaaagaagccaggtcttcaattaataagattccctggtctcgtttgtctacctgttaatg

SEQ ID NO: 216 - DNA, 60 bp, synthetic construct
  misc_feature 1..60: note = Oligonucleotide probe
  source 1..60: mol_type = other DNA
cagactcgcgcccaattttcccccaccccttgttattgccacaaaatcctgaggatgatc

SEQ ID NO: 217 - DNA, 60 bp, synthetic construct
  misc_feature 1..60: note = Oligonucleotide probe
  source 1..60: mol_type = other DNA
tctttcttcttcctttatggggccctcctgctggctgagggcttctacaccaccggcgca

SEQ ID NO: 218 - DNA, 60 bp, synthetic construct
  misc_feature 1..60: note = Oligonucleotide probe
  source 1..60: mol_type = other DNA
gtttgtgtttctacatctgcaggctgatgctgatttctaaccaccccatgtcaatcattt

SEQ ID NO: 219 - DNA, 60 bp, synthetic construct
  misc_feature 1..60: note = Oligonucleotide probe
  source 1..60: mol_type = other DNA
aaccaaatatatagtgcttccatagtgggtaggagagccaaagcacccgtaccctaactc

SEQ ID NO: 220 - DNA, 60 bp, synthetic construct
  misc_feature 1..60: note = Oligonucleotide probe
  source 1..60: mol_type = other DNA
agtctccatgtggccccgtaactccataaagcttaccctgcttgctttttgtgtcttact

SEQ ID NO: 221 - DNA, 60 bp, synthetic construct
  misc_feature 1..60: note = Oligonucleotide probe
  source 1..60: mol_type = other DNA
ccatgggtgtaatttgtatggtattagctactcccttgtaaaataacccaaataacccac

SEQ ID NO: 222 - DNA, 60 bp, synthetic construct
  misc_feature 1..60: note = Oligonucleotide probe
  source 1..60: mol_type = other DNA
tttacagtggagcatattactgctgttgcaagaaacagttcttcctctttcattttcctg

SEQ ID NO: 223 - DNA, 60 bp, synthetic construct
  misc_feature 1..60: note = Oligonucleotide probe
  source 1..60: mol_type = other DNA
atagctgtacccacactatctcaggcctatttacttgccaagatcattcaaagtcaactc

SEQ ID NO: 224 - DNA, 60 bp, synthetic construct
  misc_feature 1..60: note = Oligonucleotide probe
  source 1..60: mol_type = other DNA
gatttgaggagggagtgctttcttttctactctcattcacattctctcttctgttcccta

SEQ ID NO: 225 - DNA, 60 bp, synthetic construct
  misc_feature 1..60: note = Oligonucleotide probe
  source 1..60: mol_type = other DNA
cagcattgtaggctgtgtggttagagcctcgctattagagaaagggggatttctacgggg

SEQ ID NO: 226 - DNA, 60 bp, synthetic construct
  misc_feature 1..60: note = Oligonucleotide probe
  source 1..60: mol_type = other DNA
tgttacctttaaaagacatctgctttctgccaaaattaatgtgctgaacttaaacttacc

SEQ ID NO: 227 - DNA, 60 bp, synthetic construct
  misc_feature 1..60: note = Oligonucleotide probe
  source 1..60: mol_type = other DNA
ttcccagtaaattactcttaccaatgcaacagactttaaagaagttgtgttttacaatgc

SEQ ID NO: 228 - DNA, 60 bp, synthetic construct; identical to SEQ ID NO: 147
  misc_feature 1..60: note = Oligonucleotide probe
  source 1..60: mol_type = other DNA

SEQ ID NO: 229 - DNA, 60 bp, synthetic construct
  misc_feature 1..60: note = Oligonucleotide probe
  source 1..60: mol_type = other DNA
gacaggttttgaaagatatttgtgttactaatgactgtgctataacttttttttctttcc

SEQ ID NO: 230 - DNA, 60 bp, synthetic construct
  misc_feature 1..60: note = Oligonucleotide probe
  source 1..60: mol_type = other DNA
actcaaaaaataaaaactataattactccttaatgtcagcttattatattcaatttaaac

SEQ ID NO: 231 - DNA, 60 bp, synthetic construct
  misc_feature 1..60: note = Oligonucleotide probe
  source 1..60: mol_type = other DNA
aacaccttttttgaagtaaaaggtgcactgtaataatccagactgtgtttctcccttctc

SEQ ID NO: 232 - DNA, 60 bp, synthetic construct
  misc_feature 1..60: note = Oligonucleotide probe
  source 1..60: mol_type = other DNA
gaaacctttatctgtatcaaagaatggtcctgcaccagtaatatgcatattaaaacaaga

SEQ ID NO: 233 - DNA, 60 bp, synthetic construct
  misc_feature 1..60: note = Oligonucleotide probe
  source 1..60: mol_type = other DNA
gtgtattaaccttatgtgtgacatgttctaatatagtcacattttcattatttttattat

SEQ ID NO: 234 - DNA, 60 bp, synthetic construct
  misc_feature 1..60: note = Oligonucleotide probe
  source 1..60: mol_type = other DNA
ccccagccagcggtccgcaacccttgccgcatccacgaaactttgcccatagcagcgggc

SEQ ID NO: 235 - DNA, 60 bp, synthetic construct
  misc_feature 1..60: note = Oligonucleotide probe
  source 1..60: mol_type = other DNA
cgactcatctcagcattaaagtgataaaaaaataaattaaaaggcaagtggacttcggtg

SEQ ID NO: 236 - DNA, 60 bp, synthetic construct
  misc_feature 1..60: note = Oligonucleotide probe
  source 1..60: mol_type = other DNA
ctgtggcgcgcactgcgcgctgcgccaggtttccgcaccaagacccctttaactcaagac

SEQ ID NO: 237 - DNA, 60 bp, synthetic construct
  misc_feature 1..60: note = Oligonucleotide probe
  source 1..60: mol_type = other DNA
ttctactgcgacgaggaggagaacttctaccagcagcagcagcagagcgagctgcagccc

SEQ ID NO: 238 - DNA, 60 bp, synthetic construct
  misc_feature 1..60: note = Oligonucleotide probe
  source 1..60: mol_type = other DNA
accgagctgctgggaggagacatggtgaaccagagtttcatctgcgacccggacgacgag

SEQ ID NO: 239 - DNA, 60 bp, synthetic construct
  misc_feature 1..60: note = Oligonucleotide probe
  source 1..60: mol_type = other DNA
gccgccgcctcagagtgcatcgacccctcggtggtcttcccctaccctctcaacgacagc

SEQ ID NO: 240 - DNA, 60 bp, synthetic construct
  misc_feature 1..60: note = Oligonucleotide probe
  source 1..60: mol_type = other DNA
ggcggctaggggacaggggcggggtgggcagcagctcgaatttcttccagatatcctcgc

SEQ ID NO: 241 - DNA, 60 bp, synthetic construct
  misc_feature 1..60: note = Oligonucleotide probe
  source 1..60: mol_type = other DNA
agacgagcttggcggcggccgagaagccgctccacatacagtcctggatgatgatgtttt

SEQ ID NO: 242 - DNA, 60 bp, synthetic construct
  misc_feature 1..60: note = Oligonucleotide probe
  source 1..60: mol_type = other DNA
aggagagcagagaatccgaggacggagagaaggcgctggagtcttgcgaggcgcaggact

SEQ ID NO: 243 - DNA, 60 bp, synthetic construct
  misc_feature 1..60: note = Oligonucleotide probe
  source 1..60: mol_type = other DNA
taagagtggcccgttaaataagctgccaatgaaaatgggaaaggtatccagccgcccact

SEQ ID NO: 244 - DNA, 60 bp, synthetic construct
  misc_feature 1..60: note = Oligonucleotide probe
  source 1..60: mol_type = other DNA
ttgtatttgtacagcattaatctggtaattgattattttaatgtaaccttgctaaaggag

SEQ ID NO: 245 - DNA, 60 bp, synthetic construct
  misc_feature 1..60: note = Oligonucleotide probe
  source 1..60: mol_type = other DNA
gaggccacagcaaacctcctcacagcccactggtcctcaagaggtgccacgtctccacac

SEQ ID NO: 246 - DNA, 60 bp, synthetic construct
  misc_feature 1..60: note = Oligonucleotide probe
  source 1..60: mol_type = other DNA
agaggaggaacgagctaaaacggagcttttttgccctgcgtgaccagatcccggagttgg

SEQ ID NO: 247 - DNA, 60 bp, synthetic construct
  misc_feature 1..60: note = Oligonucleotide probe
  source 1..60: mol_type = other DNA
tccaacttgaccctcttggcagcaggatagtccttccgagtggagggaggcgctgcgtag

SEQ ID NO: 248 - DNA, 60 bp, synthetic construct
  misc_feature 1..60: note = Oligonucleotide probe
  source 1..60: mol_type = other DNA
gcttggacggacaggatgtatgctgtggcttttttaaggataactaccttgggggccttt

SEQ ID NO: 249 - DNA, 60 bp, synthetic construct
  misc_feature 1..60: note = Oligonucleotide probe
  source 1..60: mol_type = other DNA
gcatttgatcatgcatttgaaacaagttcataggtgattgctcaggacatttctgttaga

SEQ ID NO: 250 - DNA, 60 bp, synthetic construct
  misc_feature 1..60: note = Oligonucleotide probe
  source 1..60: mol_type = other DNA
catcattgttgaaaacaatgaatcctctgtttcctctcccaaaagccacttggttgctcc

SEQ ID NO: 251 - DNA, 60 bp, synthetic construct
  misc_feature 1..60: note = Oligonucleotide probe
  source 1..60: mol_type = other DNA
tttatctccagaaatgacatcacagtatgtgccagcaggaagaccagtttgcaaagttaa

SEQ ID NO: 252 - DNA, 60 bp, synthetic construct
  misc_feature 1..60: note = Oligonucleotide probe
  source 1..60: mol_type = other DNA
ctattagaggacatgtctaaatacatattctcaccttatttggcgccatcgatgttcaca

SEQ ID NO: 253 - DNA, 60 bp, synthetic construct
  misc_feature 1..60: note = Oligonucleotide probe
  source 1..60: mol_type = other DNA
tctgagcaagagaaggggaggcggggtaagggaagtaggtggaagattcagccaagctca

SEQ ID NO: 254 - DNA, 60 bp, synthetic construct
  misc_feature 1..60: note = Oligonucleotide probe
  source 1..60: mol_type = other DNA
ccagaacacagagtgactctgccctgggccgaaaggcgacatttctggaaggaaaaactt

SEQ ID NO: 255 - DNA, 60 bp, synthetic construct
  misc_feature 1..60: note = Oligonucleotide probe
  source 1..60: mol_type = other DNA
cttcacttgcctatttctgccattcagtgacatgtgttgcattggttttttgtgtctttc

SEQ ID NO: 256 - DNA, 60 bp, synthetic construct
  misc_feature 1..60: note = Oligonucleotide probe
  source 1..60: mol_type = other DNA
gtgtctctctctggaaggtaaaggagaaagggaaagagaagtgcatgtgcaagacccttt

SEQ ID NO: 257 - DNA, 60 bp, synthetic construct
  misc_feature 1..60: note = Oligonucleotide probe
  source 1..60: mol_type = other DNA
ccgaagaaagagactctggaaactcattatcaggtctatcaactcttgtatttgttctcc

SEQ ID NO: 258 - DNA, 60 bp, synthetic construct
  misc_feature 1..60: note = Oligonucleotide probe
  source 1..60: mol_type = other DNA
actagaaaatgagggagaagggggagagaggaaggaggaggaagagaaagaaaagtatct

SEQ ID NO: 259 - DNA, 60 bp, synthetic construct
  misc_feature 1..60: note = Oligonucleotide probe
  source 1..60: mol_type = other DNA
gtagttgcattgtgtgtttttgaccactgatgataaattcaagtctctcttccttcccaa

SEQ ID NO: 260 - DNA, 60 bp, synthetic construct
  misc_feature 1..60: note = Oligonucleotide probe
  source 1..60: mol_type = other DNA
cataggagcgttcactaaatatgatcccccttatctcatgctcccacttcccttttcctt

SEQ ID NO: 261 - DNA, 60 bp, synthetic construct
  misc_feature 1..60: note = Oligonucleotide probe
  source 1..60: mol_type = other DNA
ctcagacttagctcaacccgtcagtacccagactgaccactgcctctgcctcttcttctc

SEQ ID NO: 262 - DNA, 60 bp, synthetic construct
  misc_feature 1..60: note = Oligonucleotide probe
  source 1..60: mol_type = other DNA
caccaaccaggtctggccaagctgctgtattttagtgaggtctgggccccaggagcactt

SEQ ID NO: 263 - DNA, 60 bp, synthetic construct
  misc_feature 1..60: note = Oligonucleotide probe
  source 1..60: mol_type = other DNA
ggaagatacagttgttgagaaaaggaaattgagagaaaacacaattagtaagagtaactc

SEQ ID NO: 264 - DNA, 60 bp, synthetic construct
  misc_feature 1..60: note = Oligonucleotide probe
  source 1..60: mol_type = other DNA
ttttagatttatattggcctcatatgtatatggatatttcataggcattgtgtttctttt

SEQ ID NO: 265 - DNA, 60 bp, synthetic construct
  misc_feature 1..60: note = Oligonucleotide probe
  source 1..60: mol_type = other DNA
tgtaggggccaataattatattcgaggttactgttaaattatttacaaagtataggtgat

SEQ ID NO: 266 - DNA, 60 bp, synthetic construct
  misc_feature 1..60: note = Oligonucleotide probe
  source 1..60: mol_type = other DNA
tttgagtaaagatttttaaattctaacattgttagtttgtaataaaatgtattgtttcta

SEQ ID NO: 267 - DNA, 60 bp, synthetic construct
  misc_feature 1..60: note = Oligonucleotide probe
  source 1..60: mol_type = other DNA
catatcaagttcatttgtagagatgaggactacagcccatatcaagctataccttctact

SEQ ID NO: 268 - DNA, 60 bp, synthetic construct
  misc_feature 1..60: note = Oligonucleotide probe
  source 1..60: mol_type = other DNA
atgtcagcaagatttcttcttgcaaagataacatcataccataatatttgtttcaatttt

SEQ ID NO: 269 - DNA, 60 bp, synthetic construct
  misc_feature 1..60: note = Oligonucleotide probe
  source 1..60: mol_type = other DNA
caaccacagattcataccaaatgcattacttttagattattaacatattcttttacataa

SEQ ID NO: 270 - DNA, 60 bp, synthetic construct
  misc_feature 1..60: note = Oligonucleotide probe
  source 1..60: mol_type = other DNA
aagaaaggtagtaattccaaattattaacatctgtttttggttttatgtttcttcttttt

SEQ ID NO: 271 - DNA, 60 bp, synthetic construct
  misc_feature 1..60: note = Oligonucleotide probe
  source 1..60: mol_type = other DNA
ggcctatgtgtggccaccccagtccagctccgggtgttccgcgagttccacctgcacctc

SEQ ID NO: 272 - DNA, 60 bp, synthetic construct
  misc_feature 1..60: note = Oligonucleotide probe
  source 1..60: mol_type = other DNA
aggcgtggcctccctcttgaggcttcctcgaggctgtggggagcaaaccatgatctactt

SEQ ID NO: 273 - DNA, 60 bp, synthetic construct
  misc_feature 1..60: note = Oligonucleotide probe
  source 1..60: mol_type = other DNA
cctagcttggccagaaggtagcagacagacagacggatctaacctctcttggatcctcca

SEQ ID NO: 274 - DNA, 60 bp, synthetic construct
  misc_feature 1..60: note = Oligonucleotide probe
  source 1..60: mol_type = other DNA
tgaatcgggtcccgatgccagccctgccccaatccaagcacccagcatcccgcctccagg

SEQ ID NO: 275 - DNA, 60 bp, synthetic construct
  misc_feature 1..60: note = Oligonucleotide probe
  source 1..60: mol_type = other DNA
agggagagcaggggtggaggtgtcagagcgaagtctgactgctgatcctgtctgttctcc

SEQ ID NO: 276 - DNA, 60 bp, synthetic construct
  misc_feature 1..60: note = Oligonucleotide probe
  source 1..60: mol_type = other DNA
tgacacttacaagacagatgggaacagggcaggaggcccccacaagcagcaggagggcat

SEQ ID NO: 277 - DNA, 60 bp, synthetic construct
  misc_feature 1..60: note = Oligonucleotide probe
  source 1..60: mol_type = other DNA
cctttttggtcagctgtctcttgctctgtgacccgctccctctccctctccctctcctga

SEQ ID NO: 278 - DNA, 60 bp, synthetic construct
  misc_feature 1..60: note = Oligonucleotide probe
  source 1..60: mol_type = other DNA
caaactcatcctgagagggctcggagggggttaaaggttgaggccctggggctgagactc

SEQ ID NO: 279 - DNA, 60 bp, synthetic construct
  misc_feature 1..60: note = Oligonucleotide probe
  source 1..60: mol_type = other DNA
agtttgacccaccctccccttgcacatggacccctgctcacctctctcctcctccactcc

SEQ ID NO: 280 - DNA, 60 bp, synthetic construct
  misc_feature 1..60: note = Oligonucleotide probe
  source 1..60: mol_type = other DNA
aaggggagaagtgctcacaggcaggaggtcacatcagtggccaggatcaggaaggccaga

SEQ ID NO: 281 - DNA, 60 bp, synthetic construct
  misc_feature 1..60: note = Oligonucleotide probe
  source 1..60: mol_type = other DNA
gttctgaagcttctgagttctgcagcctcacctctgagaaaacctctttgccaccaatac

SEQ ID NO: 282 - DNA, 60 bp, synthetic construct
  misc_feature 1..60: note = Oligonucleotide probe
  source 1..60: mol_type = other DNA
ggcagtgttgatctcaccctggcctttcctttcagtgggctcagaccctcccaccgcctg

SEQ ID NO: 283 - DNA, 60 bp, synthetic construct
  misc_feature 1..60: note = Oligonucleotide probe
  source 1..60: mol_type = other DNA
accacagctggctgggagcagaggctgctggtctcatagtaatctaccacaaagttgcga

SEQ ID NO: 284 - DNA, 60 bp, synthetic construct
  misc_feature 1..60: note = Oligonucleotide probe
  source 1..60: mol_type = other DNA
tcaggtgaccttccctgaagacttcctgtctctgagcagctcagttcagttccaggtcat

SEQ ID NO: 285 - DNA, 60 bp, synthetic construct
  misc_feature 1..60: note = Oligonucleotide probe
  source 1..60: mol_type = other DNA
ggagcatatagtgggcctaggtgattggccactttatccatcaaagaggcacacacactt

SEQ ID NO: 286 - DNA, 60 bp, synthetic construct
  misc_feature 1..60: note = Oligonucleotide probe
  source 1..60: mol_type = other DNA
cctttcaaagtattttactttacaatgatctcttgtaacattgtacctctagggatatac

SEQ ID NO: 287 - DNA, 60 bp, synthetic construct
  misc_feature 1..60: note = Oligonucleotide probe
  source 1..60: mol_type = other DNA
atggggaggatggaaaacagactagcagagcttctcgggcagagcttggcccatccacat

SEQ ID NO: 288 - DNA, 60 bp, synthetic construct
  misc_feature 1..60: note = Oligonucleotide probe
  source 1..60: mol_type = other DNA
gatctggccacccctgaaatgtttccaagaatgtcagtagagaggagagcagtccagaaa

SEQ ID NO: 289 - DNA, 62 bp, synthetic construct
  misc_feature 1..62: note = Oligonucleotide probe
  source 1..62: mol_type = other DNA
agcaaccagagcttggcatattgtatctatacctttattaaatgcttttaatttaataaatt

SEQ ID NO: 290 - DNA, 60 bp, synthetic construct
  misc_feature 1..60: note = Oligonucleotide probe
  source 1..60: mol_type = other DNA
caaaactagtcaatgaatcacaaatacgcaagcagtcacataactaagcttttgttaaca

SEQ ID NO: 291 - DNA, 60 bp, synthetic construct
  misc_feature 1..60: note = Oligonucleotide probe
  source 1..60: mol_type = other DNA
aaggagcatatagtggacctaggtgattggtcaatttatccatcaaagaggcacacaccg

SEQ ID NO: 292 - DNA, 60 bp, synthetic construct
  misc_feature 1..60: note = Oligonucleotide probe
  source 1..60: mol_type = other DNA
agcctttcaaagtattttactttaccattacctcttgtaacatgtacctctagggataca

SEQ ID NO: 293 - DNA, 60 bp, synthetic construct
  misc_feature 1..60: note = Oligonucleotide probe
  source 1..60: mol_type = other DNA
ggggaggatggaaaacagagacttacagagctcctcgggcagagcttggcccatccacat

SEQ ID NO: 294 - DNA, 60 bp, synthetic construct
  misc_feature 1..60: note = Oligonucleotide probe
  source 1..60: mol_type = other DNA
gatatggccacccctgaaatgtttccaagaatgtcagtagagaagatagtagtccagtaa

SEQ ID NO: 295 - DNA, 62 bp, synthetic construct
  misc_feature 1..62: note = Oligonucleotide probe
  source 1..62: mol_type = other DNA
ctcaaccagagcttggtatatggtatgtatgcttttattaaaatcttttaatttaataaatt

SEQ ID NO: 296 - DNA, 60 bp, synthetic construct
  misc_feature 1..60: note = Oligonucleotide probe
  source 1..60: mol_type = other DNA
cagaactagtcaacaaatcacaaattcacaagcagtcacataactaagcttttgtttaca

SEQ ID NO: 297 - DNA, 60 bp, synthetic construct
  misc_feature 1..60: note = Oligonucleotide probe
  source 1..60: mol_type = other DNA
ggaagtcccccaaacctgcttccccttctcagcctggcttctggtccagcctgtggtttc

SEQ ID NO: 298 - DNA, 60 bp, synthetic construct
  misc_feature 1..60: note = Oligonucleotide probe
  source 1..60: mol_type = other DNA
gcctggtggggtgggggtgccaggtgtgtccagaggagcccatttggtagtgaggcaggt

SEQ ID NO: 299 - DNA, 60 bp, synthetic construct
  misc_feature 1..60: note = Oligonucleotide probe
  source 1..60: mol_type = other DNA
gcccagctcggactacggtcatcacccacccgggtcccacggaaatctgtctctgtcccc

SEQ ID NO: 300 - DNA, 60 bp, synthetic construct
  misc_feature 1..60: note = Oligonucleotide probe
  source 1..60: mol_type = other DNA
aataggactaggacctgtagtctggggggatcctggcttgacaagaggccctgaccctcc

SEQ ID NO: 301 - DNA, 60 bp, synthetic construct
  misc_feature 1..60: note = Oligonucleotide probe
  source 1..60: mol_type = other DNA
aagttcatgggcccccgcctgtacccttcctccctcggcccctgcactgtttcccagatg

SEQ ID NO: 302 - DNA, 60 bp, synthetic construct
  misc_feature 1..60: note = Oligonucleotide probe
  source 1..60: mol_type = other DNA
gggctgacaggtgcagaattggaggtcatttgggggctaccccgttctgtcccgagtatg

SEQ ID NO: 303 - DNA, 60 bp, synthetic construct
  misc_feature 1..60: note = Oligonucleotide probe
  source 1..60: mol_type = other DNA
cattgctttattgtacattagagcctctggctagggagcaggctggggactaggtacccc

SEQ ID NO: 304 - DNA, 60 bp, synthetic construct
  misc_feature 1..60: note = Oligonucleotide probe
  source 1..60: mol_type = other DNA
tggagtcttgcaggggtatcacccaggagccaggctcactgacgcccctcccctccccac

SEQ ID NO: 305 - DNA, 60 bp, synthetic construct
  misc_feature 1..60: note = Oligonucleotide probe
  source 1..60: mol_type = other DNA
agtgcatgtgtgtgagtgctgccgctgcccgcgacccctggccccgaaggtgttggctga

SEQ ID NO: 306 - DNA, 60 bp, synthetic construct
  misc_feature 1..60: note = Oligonucleotide probe
  source 1..60: mol_type = other DNA
aatgagaagggaagtggggtacggaagggggtgcgacgagaagaaaggaaagagccactt

SEQ ID NO: 307 - DNA, 60 bp, synthetic construct
  misc_feature 1..60: note = Oligonucleotide probe
  source 1..60: mol_type = other DNA
ggaatctaagcctgagatttatttgaatacatgaacatatttccctgtgctctcttgttc

SEQ ID NO: 308 - DNA, 60 bp, synthetic construct
  misc_feature 1..60: note = Oligonucleotide probe
  source 1..60: mol_type = other DNA
aagatggcattcatctggccttgggaatggatgaaaggaagcagcaactttcaaatgggt

SEQ ID NO: 309 - DNA, 60 bp, synthetic construct
  misc_feature 1..60: note = Oligonucleotide probe
  source 1..60: mol_type = other DNA
ggtaaagtccctcatctggcttgtggtgtctggaatgaagtatgttttgtatcagcagag

SEQ ID NO: 310 - DNA, 60 bp, synthetic construct
  misc_feature 1..60: note = Oligonucleotide probe
  source 1..60: mol_type = other DNA
tttattggcgattattgtgctttatttggaagacttattcttccttctttgtttttctcc

SEQ ID NO: 311 - DNA, 60 bp, synthetic construct
  misc_feature 1..60: note = Oligonucleotide probe
  source 1..60: mol_type = other DNA
gaaaaaaattgtttttcaacttattccagagaatatcattctgaaggcaacaaagagcat

SEQ ID NO: 312 - DNA, 60 bp, synthetic construct
  misc_feature 1..60: note = Oligonucleotide probe
  source 1..60: mol_type = other DNA
atatatcatttatctttgcaatgtttttcatatatcatatgatactgtgttttcccctca

SEQ ID NO: 313 - DNA, 60 bp, synthetic construct
  misc_feature 1..60: note = Oligonucleotide probe
  source 1..60: mol_type = other DNA
attagagaaatataaatagcagcatataccatacaaaagtacactttacaaaaaagtctt

SEQ ID NO: 314 - DNA, 60 bp, synthetic construct
  misc_feature 1..60: note = Oligonucleotide probe
  source 1..60: mol_type = other DNA
atactccatctcccgtaaaaatagtgagacttgagtaatgtttgatgtcacttgtctttc

SEQ ID NO: 315 - DNA, 60 bp, synthetic construct
  misc_feature 1..60: note = Oligonucleotide probe
  source 1..60: mol_type = other DNA
cagtcaccactatattattctaggtatcccagaaaagttaaagtcaaatctgaaacacat

SEQ ID NO: 316 - DNA, 60 bp, synthetic construct
  misc_feature 1..60: note = Oligonucleotide probe
  source 1..60: mol_type = other DNA
ttcttactgttctagcttgtccttaaggcctctgtgctttttaacaaatggtttcttttg

SEQ ID NO: 317 - DNA, 60 bp, synthetic construct
  misc_feature 1..60: note = Oligonucleotide probe
  source 1..60: mol_type = other DNA
tccgcatgcactccctggacatgtggacacatggaccatggtccacacctggccaagctt

SEQ ID NO: 318 - DNA, 60 bp, synthetic construct
  misc_feature 1..60: note = Oligonucleotide probe
  source 1..60: mol_type = other DNA
cttggcttgggctgtgttgtgtgaacggaacagttcaccccagtatggccttcttgccga

SEQ ID NO: 319 - DNA, 60 bp, synthetic construct
  misc_feature 1..60: note = Oligonucleotide probe
  source 1..60: mol_type = other DNA
gctgtgcataatcactggacaacaaactaattagcacttttcaaaataatgcagttactt

SEQ ID NO: 320 - DNA, 60 bp, synthetic construct
  misc_feature 1..60: note = Oligonucleotide probe
  source 1..60: mol_type = other DNA
gaacagcagtcagattgctcatctctatcactttttctcattgtgtcccttttctctcct

SEQ ID NO: 321 - DNA, 60 bp, synthetic construct
  misc_feature 1..60: note = Oligonucleotide probe
  source 1..60: mol_type = other DNA
agagaatgaaagggaaaaagaaaagccaaagcgtactgactattcaaggggatcgtactt

SEQ ID NO: 322 - DNA, 60 bp, synthetic construct
  misc_feature 1..60: note = Oligonucleotide probe
  source 1..60: mol_type = other DNA
tattgcaagttttcatttggttaaggtttggggttaattttggaattggctctgctcttc

SEQ ID NO: 323 - DNA, 60 bp, synthetic construct
  misc_feature 1..60: note = Oligonucleotide probe
  source 1..60: mol_type = other DNA
aaaacttgttaatattcacgataaagaaaaattccagagaaagtaacaacgttaagactt

SEQ ID NO: 324 - DNA, 60 bp, synthetic construct
  misc_feature 1..60: note = Oligonucleotide probe
  source 1..60: mol_type = other DNA
gcagaagaagccccgccaccagcagcttctgccatctctctcctcctttttcttcagcca

SEQ ID NO: 325 - DNA, 60 bp, synthetic construct
  misc_feature 1..60: note = Oligonucleotide probe
  source 1..60: mol_type = other DNA
ctactcccacgttctaagagagtgacagaaaggtaaagaggagcagccgcagaaatggat

SEQ ID NO: 326 - DNA, 60 bp, synthetic construct
  misc_feature 1..60: note = Oligonucleotide probe
  source 1..60: mol_type = other DNA
agtattcttttagtttgattgctgcatatttcagatatttctttccttaactaaagtact

SEQ ID NO: 327 - DNA, 60 bp, synthetic construct
  misc_feature 1..60: note = Oligonucleotide probe
  source 1..60: mol_type = other DNA
aatgaaaacacaacatgaatataaacatcaatatttgaaatagaaaatcaaagcattctt

SEQ ID NO: 328 - DNA, 60 bp, synthetic construct
  misc_feature 1..60: note = Oligonucleotide probe
  source 1..60: mol_type = other DNA
gtaatttcaaatgttagctcatttttgttaatggtggctttttgtttgtttgttttgttt

SEQ ID NO: 329 - DNA, 60 bp, synthetic construct
  misc_feature 1..60: note = Oligonucleotide probe
  source 1..60: mol_type = other DNA
ctttcacttaatagttgttttagaagatatttgcaagcatacaaataagaaaacatactt

SEQ ID NO: 330 - DNA, 60 bp, synthetic construct
  misc_feature 1..60: note = Oligonucleotide probe
  source 1..60: mol_type = other DNA
gtacttttttttcttcctaagtgcaaaagataactttatatcacttttaaacttttcttt

SEQ ID NO: 331 - DNA, 60 bp, synthetic construct
  misc_feature 1..60: note = Oligonucleotide probe
  source 1..60: mol_type = other DNA
acagtaagatacagtctatcgggtttaagttatacaacatagtacagtacattcatacct

SEQ ID NO: 332 - DNA, 60 bp, synthetic construct
  misc_feature 1..60: note = Oligonucleotide probe
  source 1..60: mol_type = other DNA
tacttgttaattaaaaattcaagagtttttttttcttattctgaggttatctttttacca

SEQ ID NO: 333 - DNA, 60 bp, synthetic construct
  misc_feature 1..60: note = Oligonucleotide probe
  source 1..60: mol_type = other DNA
ccaaaatctgttttccaataaattctcagatccaggaagaggaaaggaaaaacatcaaaa

SEQ ID NO: 334 - DNA, 60 bp, synthetic construct
  misc_feature 1..60: note = Oligonucleotide probe
  source 1..60: mol_type = other DNA
tcaagtaggtgttggagagaggggtgatgcctggtgctggtggaacccctgcacagagac

SEQ ID NO: 335 - DNA, 60 bp, synthetic construct
  misc_feature 1..60: note = Oligonucleotide probe
  source 1..60: mol_type = other DNA
cctgtcctttcggggtccattccctctatgacccagaagtgatccagccaccatcccaat

SEQ ID NO: 336 - DNA, 60 bp, synthetic construct
  misc_feature 1..60: note = Oligonucleotide probe
  source 1..60: mol_type = other DNA
aacccctcgaggctcagacctttggagcaggagtgtgattctggccaaccaccctctctg

SEQ ID NO: 337 - DNA, 60 bp, synthetic construct
  misc_feature 1..60: note = Oligonucleotide probe
  source 1..60: mol_type = other DNA
cataaatatgtgtgctagtcctgttagacccaagtgctgcccaagggcagcgccctgctc

SEQ ID NO: 338 - DNA, 60 bp, synthetic construct
  misc_feature 1..60: note = Oligonucleotide probe
  source 1..60: mol_type = other DNA
ttgcagcaagatggtgttctctctctaccttgcttcctttacccacacgctatttctttg

SEQ ID NO: 339 - DNA, 60 bp, synthetic construct
  misc_feature 1..60: note = Oligonucleotide probe
  source 1..60: mol_type = other DNA
gagatcaagccaaaatcagtatgtgggttcatctgcaataaaaatgtttgttttgctttt

SEQ ID NO: 340 - DNA, 60 bp, synthetic construct
  misc_feature 1..60: note = Oligonucleotide probe
  source 1..60: mol_type = other DNA
gcaacagtgagaggaagttgtcttgtttttgaacaggccttgtttttcttggatgctttt

SEQ ID NO: 341 - DNA, 60 bp, synthetic construct
  misc_feature 1..60: note = Oligonucleotide probe
  source 1..60: mol_type = other DNA
ctgccatttcattacaggcaaagctgagcaaaagtagatattacaagaccagcatgtact

SEQ ID NO: 342 - DNA, 60 bp, synthetic construct
  misc_feature 1..60: note = Oligonucleotide probe
  source 1..60: mol_type = other DNA
aaggtaaaagaaatcattgagtcccccgccttcagaagagggtgcattttcaggaggaag

SEQ ID NO: 343 - DNA, 60 bp, synthetic construct
  misc_feature 1..60: note = Oligonucleotide probe
  source 1..60: mol_type = other DNA
gcggatctcccccggcctcgccggcctccgcctgtcctcccaccaccctctccgggccag

SEQ ID NO: 344 - DNA, 60 bp, synthetic construct
  misc_feature 1..60: note = Oligonucleotide probe
  source 1..60: mol_type = other DNA
ctggtaggagctgtttgcagggtcctaactcaatcggcttgttgtgatgcgtatccccgt

SEQ ID NO: 345 - DNA, 60 bp, synthetic construct
  misc_feature 1..60: note = Oligonucleotide probe
  source 1..60: mol_type = other DNA
ttttgaaatgtgggtttgttgccatgaaacgtgtttcaagcatagttttgacagataacg

SEQ ID NO: 346 - DNA, 60 bp, synthetic construct
  misc_feature 1..60: note = Oligonucleotide probe
  source 1..60: mol_type = other DNA
tgccctaaaagtgtatgtataacatccctgatgtctgcatttgtcctttgactggtgttt

SEQ ID NO: 347 - DNA, 60 bp, synthetic construct
  misc_feature 1..60: note = Oligonucleotide probe
  source 1..60: mol_type = other DNA
gtataccagcctggagggtgtaccagcctggagggtgtaccagccccaagtggatgcact

SEQ ID NO: 348 - DNA, 60 bp, synthetic construct
  misc_feature 1..60: note = Oligonucleotide probe
  source 1..60: mol_type = other DNA
ttcaacagatatgttcaggccaccaacctcattctgttttgttctctatcgtgtccccac

SEQ ID NO: 349 - DNA, 60 bp, synthetic construct
  misc_feature 1..60: note = Oligonucleotide probe
  source 1..60: mol_type = other DNA
aggatgtgtctgggtggtgcttggggacagaggcaccttcccgacacccgcctgcccctc

SEQ ID NO: 350 - DNA, 60 bp, synthetic construct
  misc_feature 1..60: note = Oligonucleotide probe
  source 1..60: mol_type = other DNA
cctcagccagtgccacccccacagcccacagggaggaggcacagaaagcgactcacacgt

SEQ ID NO: 351 - DNA, 60 bp, synthetic construct
  misc_feature 1..60: note = Oligonucleotide probe
  source 1..60: mol_type = other DNA
ctggtgtggagctgccgggcacttccatgactttgtttctgtctctgcttcctcctcagt

SEQ ID NO: 352 - DNA, 60 bp, synthetic construct
  misc_feature 1..60: note = Oligonucleotide probe
  source 1..60: mol_type = other DNA
ctggtgcaggctgtgctcactgcccgtgccctggacctcccagcaccactcgccccgctc

SEQ ID NO: 353 - DNA, 60 bp, synthetic construct
  misc_feature 1..60: note = Oligonucleotide probe
  source 1..60: mol_type = other DNA
gtcatggtgaggggtgtgctgggaccggctgggcagtgaccccgagccgcctccggcccc

SEQ ID NO: 354 - DNA, 60 bp, synthetic construct
  misc_feature 1..60: note = Oligonucleotide probe
  source 1..60: mol_type = other DNA
ccggggcccacggcggctccacgcccaccgtgctgcgtgcctcagtctccccacccgcat

SEQ ID NO: 355 - DNA, 60 bp, synthetic construct
  misc_feature 1..60: note = Oligonucleotide probe
  source 1..60: mol_type = other DNA
ctgtaagttatcgtaaaaaggagcatctaggtaggtctttgtagccaatgttacccgatt

SEQ ID NO: 356 - DNA, 60 bp, synthetic construct
  misc_feature 1..60: note = Oligonucleotide probe
  source 1..60: mol_type = other DNA
agtaaaataagtttcgaactctggcacctttcaattttgtcgcactctccttgtttttga

SEQ ID NO: 357 - DNA, 60 bp, synthetic construct
  misc_feature 1..60: note = Oligonucleotide probe
  source 1..60: mol_type = other DNA
gaagcaaactgcaattcttcggcagcatcttcgccttccgacgaggtcgatacttataat

SEQ ID NO: 358 - DNA, 60 bp, synthetic construct
  misc_feature 1..60: note = Oligonucleotide probe
  source 1..60: mol_type = other DNA
aatggccattcttccaggaggcacagaaattacaggccatgcacagagagaaatacccga

SEQ ID NO: 359 - DNA, 60 bp, synthetic construct
  misc_feature 1..60: note = Oligonucleotide probe
  source 1..60: mol_type = other DNA
cttgcgcctctgatcgcgagaccacacgatgaatgcgttcatgggtcgcttcactctatc

SEQ ID NO: 360 - DNA, 60 bp, synthetic construct
  misc_feature 1..60: note = Oligonucleotide probe
  source 1..60: mol_type = other DNA
gaaagctgtaactctaagtatcagtgtgaaacgggagaaaacagtaaaggcaacgtccag

SEQ ID NO: 361 - DNA, 60 bp, synthetic construct
  misc_feature 1..60: note = Oligonucleotide probe
  source 1..60: mol_type = other DNA
agttcctctgctggagttcatcctgctagctgggttcccgagctgccggtctgagcctga

SEQ ID NO: 362 - DNA, 60 bp, synthetic construct
  misc_feature 1..60: note = Oligonucleotide probe
  source 1..60: mol_type = other DNA
tctgtgggaggccctggggtcagaactgggatctgcgagcagacggagaggaggctcggg

SEQ ID NO: 363 - DNA, 60 bp, synthetic construct
  misc_feature 1..60: note = Oligonucleotide probe
  source 1..60: mol_type = other DNA
caagcctggcagagcccacagggcagccagggcatctcccaatgcctgtcctgaccccct

SEQ ID NO: 364 - DNA, 60 bp, synthetic construct
  misc_feature 1..60: note = Oligonucleotide probe
  source 1..60: mol_type = other DNA
tgtctggggcagaagggggcaagagtgtctgccctcggcccacagagctggcccgccaaa

SEQ ID NO: 365 - DNA, 60 bp, synthetic construct
  misc_feature 1..60: note = Oligonucleotide probe
  source 1..60: mol_type = other DNA
tgatgggtgggctcccgaaggggcctcccgcagacttgcgaagttcccactctctgggcg

SEQ ID NO: 366 - DNA, 60 bp, synthetic construct
  misc_feature 1..60: note = Oligonucleotide probe
  source 1..60: mol_type = other DNA
cagggtgcgggggcatccaggctgcccaagcggaggctgggccggctgtgctggcctctt

SEQ ID NO: 367 - DNA, 60 bp, synthetic construct
  misc_feature 1..60: note = Oligonucleotide probe
  source 1..60: mol_type = other DNA
ctccaccttctttatctctgaaagtgaactccctgctacctttgtggactgacagctttt

SEQ ID NO: 368 - DNA, 60 bp, synthetic construct
  misc_feature 1..60: note = Oligonucleotide probe
  source 1..60: mol_type = other DNA
tcgatccaaagtaatacatctgaaagaatatacgcatgtaaaagtcccactccaatacac

SEQ ID NO: 369 - DNA, 60 bp, synthetic construct
  misc_feature 1..60: note = Oligonucleotide probe
  source 1..60: mol_type = other DNA
ctgcagcagaggggacatgaaatagttgtcctagcacctgacgcctcgttgtacatcaga

SEQ ID NO: 370 - DNA, 60 bp, synthetic construct
  misc_feature 1..60: note = Oligonucleotide probe
  source 1..60: mol_type = other DNA
actctttcacatcctccctttggaatggcacagggtacgtcttcaaggtgtaaaatgctc

SEQ ID NO: 371 - DNA, 60 bp, synthetic construct
  misc_feature 1..60: note = Oligonucleotide probe
  source 1..60: mol_type = other DNA
gcgtgtgatcaaaacatacaagaaaataaaaaaggactctgctatgcttttgtctggctg

SEQ ID NO: 372 - DNA, 60 bp, synthetic construct
  misc_feature 1..60: note = Oligonucleotide probe
  source 1..60: mol_type = other DNA
acatcaaagctgctttctgccagggaggccatgagctccttgttgtgcagtaagtgggaa

SEQ ID NO: 373 - DNA, 60 bp, synthetic construct
  misc_feature 1..60: note = Oligonucleotide probe
  source 1..60: mol_type = other DNA
ctctgcccactgtattcttcttgcatgcactgccatgcagcctggaatttgaggctaccc

SEQ ID NO: 374 - DNA, 60 bp, synthetic construct
  misc_feature 1..60: note = Oligonucleotide probe
  source 1..60: mol_type = other DNA
tcatgtgatctgaatgagaggagagaggcctgggcacgtaggagaatgggttggggcact

SEQ ID NO: 375 - DNA, 60 bp, synthetic construct
  misc_feature 1..60: note = Oligonucleotide probe
  source 1..60: mol_type = other DNA
tgcgacgtggtttattccccgtatgcaacccttgcctcagaattccttcagagagaggtg

SEQ ID NO: 376 - DNA, 60 bp, synthetic construct
  misc_feature 1..60: note = Oligonucleotide probe
  source 1..60: mol_type = other DNA
cttcacaaagtcacttctaaacagccagacagatgcagagctcaataggtcctggacagt

SEQ ID NO: 377 - DNA, 60 bp, synthetic construct
  misc_feature 1..60: note = Oligonucleotide probe
  source 1..60: mol_type = other DNA
actgtatgtagtcatcaaagaatatgagaaaaaattaactgaaaatttttcttctggctc

SEQ ID NO: 378 - DNA, 60 bp, synthetic construct
  misc_feature 1..60: note = Oligonucleotide probe
  source 1..60: mol_type = other DNA
attaatctggaagctggaagtctgggattagcgctcctgtgaaaatagatatgaggccat

SEQ ID NO: 379 - DNA, 60 bp, synthetic construct
  misc_feature 1..60: note = Oligonucleotide probe
  source 1..60: mol_type = other DNA
cagatttgttttctaatcatattatgttctttctttacgttctgctctttttgcccctcc

SEQ ID NO: 380 - DNA, 60 bp, synthetic construct
  misc_feature 1..60: note = Oligonucleotide probe
  source 1..60: mol_type = other DNA
gcttaagccattttcttaatttgaccctggtttgacctatacatccaatccgcccaacat

SEQ ID NO: 381 - DNA, 60 bp, synthetic construct
  misc_feature 1..60: note = Oligonucleotide probe
  source 1..60: mol_type = other DNA
tgtgtccagctgtgaaactcagagatgtaactgctgacatcctccctattttgcatctca

SEQ ID NO: 382 - DNA, 60 bp, synthetic construct
  misc_feature 1..60: note = Oligonucleotide probe
  source 1..60: mol_type = other DNA
atttgaaacaattttatcatgaatgccatgaccaaagtattcttctgtatcttctttctt

SEQ ID NO: 383 - DNA, 60 bp, synthetic construct
  misc_feature 1..60: note = Oligonucleotide probe
  source 1..60: mol_type = other DNA
ataaagagaggattgttcataccacaggtgttccaggcataacgaaactgtctttgtgtt

SEQ ID NO: 384 - DNA, 60 bp, synthetic construct
  misc_feature 1..60: note = Oligonucleotide probe
  source 1..60: mol_type = other DNA
ttttcaagtttggaaatgactagggaatggttcaaaattttaccttatttcccacccact

SEQ ID NO: 385 - DNA, 60 bp, synthetic construct
  misc_feature 1..60: note = Oligonucleotide probe
  source 1..60: mol_type = other DNA
cgccccgcgtccgacccgcggatcccgcggcgtccggcccgggtggtctggatcgcggag

SEQ ID NO: 386 - DNA, 60 bp, synthetic construct
  misc_feature 1..60: note = Oligonucleotide probe
  source 1..60: mol_type = other DNA
tagaggggcttcagaccgtgctatcgtccctgctgggtcgggcctaagcgccgggcccgt

SEQ ID NO: 387 - DNA, 60 bp, synthetic construct
  misc_feature 1..60: note = Oligonucleotide probe
  source 1..60: mol_type = other DNA
ggcgccgaggaggagatggaggccgggcggccgcggcccgtgctgcgctcggtgaactcg

SEQ ID NO: 388 - DNA, 60 bp, synthetic construct
  misc_feature 1..60: note = Oligonucleotide probe
  source 1..60: mol_type = other DNA
ccatacgggcagcacgacgcgcggactgcgattgcagaagatgacctgggagggctcgcg

SEQ ID NO: 389 - DNA, 60 bp, synthetic construct
  misc_feature 1..60: note = Oligonucleotide probe
  source 1..60: mol_type = other DNA
ggtgtgggccaccgtgcccagccaccggtgtggctctttaacaacctttgcttgtcccga

SEQ ID NO: 390 - DNA, 60 bp, synthetic construct
  misc_feature 1..60: note = Oligonucleotide probe
  source 1..60: mol_type = other DNA
aagtggtctatcctgtacttaccacaacaaccttatctttttaaaaagtaaaacgtcagt

SEQ ID NO: 391 - DNA, 60 bp, synthetic construct
  misc_feature 1..60: note = Oligonucleotide probe
  source 1..60: mol_type = other DNA
cttgttcgttccttgtactgagaccctagtctgccactgaggatttggtttttgcccttc

SEQ ID NO: 392 - DNA, 60 bp, synthetic construct
  misc_feature 1..60: note = Oligonucleotide probe
  source 1..60: mol_type = other DNA
atcaagactcatcagtaccatcaaaagctgagatgaaacagtgtaagtttcaacagaaat

SEQ ID NO: 393 - DNA, 10 bp, synthetic construct
  misc_feature 1..10: note = 10 nt read_2 sequence
  source 1..10: mol_type = other DNA
aagcacctag

SEQ ID NO: 394 - DNA, 10 bp, synthetic construct
  misc_feature 1..10: note = 10 nt read_2 sequence
  source 1..10: mol_type = other DNA
agtcggtggg

SEQ ID NO: 395 - DNA, 10 bp, synthetic construct
  misc_feature 1..10: note = 10 nt read_2 sequence
  source 1..10: mol_type = other DNA
acctgagtag

SEQ ID NO: 396 - DNA, 10 bp, synthetic construct
  misc_feature 1..10: note = 10 nt read_2 sequence
  source 1..10: mol_type = other DNA
cctggccctc

SEQ ID NO: 397 - DNA, 10 bp, synthetic construct
  misc_feature 1..10: note = 10 nt read_2 sequence
  source 1..10: mol_type = other DNA
agaattcatt

SEQ ID NO: 398 - DNA, 10 bp, synthetic construct
  misc_feature 1..10: note = 10 nt read_2 sequence
  source 1..10: mol_type = other DNA
gacttcaaag

SEQ ID NO: 399 - DNA, 10 bp, synthetic construct
  misc_feature 1..10: note = 10 nt read_2 sequence
  source 1..10: mol_type = other DNA
tctctttggg

SEQ ID NO: 400 - DNA, 10 bp, synthetic construct
  misc_feature 1..10: note = 10 nt read_2 sequence
  source 1..10: mol_type = other DNA
tgcgatacca

SEQ ID NO: 401 - DNA, 10 bp, synthetic construct
  misc_feature 1..10: note = 10 nt read_2 sequence
  source 1..10: mol_type = other DNA
ggggtaggtg

SEQ ID NO: 402 - DNA, 10 bp, synthetic construct
  misc_feature 1..10: note = 10 nt read_2 sequence
  source 1..10: mol_type = other DNA
ttacttccct

SEQ ID NO: 403 - DNA, 10 bp, synthetic construct
  misc_feature 1..10: note = 10 nt read_2 sequence
  source 1..10: mol_type = other DNA
caggggtatc

SEQ ID NO: 404 - DNA, 10 bp, synthetic construct
  misc_feature 1..10: note = 10 nt read_2 sequence
  source 1..10: mol_type = other DNA
gaaattctct

SEQ ID NO: 405 - DNA, 10 bp, synthetic construct
  misc_feature 1..10: note = 10 nt read_2 sequence
  source 1..10: mol_type = other DNA
gggtttgagt

SEQ ID NO: 406 - DNA, 10 bp, synthetic construct
  misc_feature 1..10: note = 10 nt read_2 sequence
  source 1..10: mol_type = other DNA
ctatctccag

SEQ ID NO: 407 - DNA, 10 bp, synthetic construct
  misc_feature 1..10: note = 10 nt read_2 sequence
  source 1..10: mol_type = other DNA
gaaagaagcc

SEQ ID NO: 408 - DNA, 10 bp, synthetic construct
  misc_feature 1..10: note = 10 nt read_2 sequence
  source 1..10: mol_type = other DNA
cagactcgcg

SEQ ID NO: 409 - DNA, 10 bp, synthetic construct
  misc_feature 1..10: note = 10 nt read_2 sequence
  source 1..10: mol_type = other DNA
tctttcttct

SEQ ID NO: 410 - DNA, 10 bp, synthetic construct
  misc_feature 1..10: note = 10 nt read_2 sequence
  source 1..10: mol_type = other DNA
gtttgtgttt

SEQ ID NO: 411 - DNA, 10 bp, synthetic construct
  misc_feature 1..10: note = 10 nt read_2 sequence
  source 1..10: mol_type = other DNA
aaccaaatat

SEQ ID NO: 412 - DNA, 10 bp, synthetic construct
  misc_feature 1..10: note = 10 nt read_2 sequence
  source 1..10: mol_type = other DNA
agtctccatg

SEQ ID NO: 413 - DNA, 10 bp, synthetic construct
  misc_feature 1..10: note = 10 nt read_2 sequence
  source 1..10: mol_type = other DNA
ccatgggtgt

SEQ ID NO: 414 - DNA, 10 bp, synthetic construct
  misc_feature 1..10: note = 10 nt read_2 sequence
  source 1..10: mol_type = other DNA
tttacagtgg

SEQ ID NO: 415 - DNA, 10 bp, synthetic construct
  misc_feature 1..10: note = 10 nt read_2 sequence
  source 1..10: mol_type = other DNA
atagctgtac

SEQ ID NO: 416 - DNA, 10 bp, synthetic construct
  misc_feature 1..10: note = 10 nt read_2 sequence
  source 1..10: mol_type = other DNA
gatttgagga

SEQ ID NO: 417 - DNA, 10 bp, synthetic construct
  misc_feature 1..10: note = 10 nt read_2 sequence
  source 1..10: mol_type = other DNA
cagcattgta

SEQ ID NO: 418 - DNA, 10 bp, synthetic construct
  misc_feature 1..10: note = 10 nt read_2 sequence
  source 1..10: mol_type = other DNA
tgttaccttt

SEQ ID NO: 419 - DNA, 10 bp, synthetic construct
  misc_feature 1..10: note = 10 nt read_2 sequence
  source 1..10: mol_type = other DNA
ttcccagtaa

SEQ ID NO: 420 - DNA, 10 bp, synthetic construct
  misc_feature 1..10: note = 10 nt read_2 sequence
  source 1..10: mol_type = other DNA
taaatgacat

SEQ ID NO: 421 - DNA, 10 bp, synthetic construct
  misc_feature 1..10: note = 10 nt read_2 sequence
  source 1..10: mol_type = other DNA
gacaggtttt

SEQ ID NO: 422 - DNA, 10 bp, synthetic construct
  misc_feature 1..10: note = 10 nt read_2 sequence
  source 1..10: mol_type = other DNA
actcaaaaaa

SEQ ID NO: 423 - DNA, 10 bp, synthetic construct
  misc_feature 1..10: note = 10 nt read_2 sequence
  source 1..10: mol_type = other DNA
aacacctttt

SEQ ID NO: 424 - DNA, 10 bp, synthetic construct
  misc_feature 1..10: note = 10 nt read_2 sequence
  source 1..10: mol_type = other DNA
gaaaccttta

SEQ ID NO: 425 - DNA, 10 bp, synthetic construct
  misc_feature 1..10: note = 10 nt read_2 sequence
  source 1..10: mol_type = other DNA
gtgtattaac

SEQ ID NO: 426 - DNA, 10 bp, synthetic construct
  misc_feature 1..10: note = 10 nt read_2 sequence
  source 1..10: mol_type = other DNA
ccccagccag

SEQ ID NO: 427 - DNA, 10 bp, synthetic construct
  misc_feature 1..10: note = 10 nt read_2 sequence
  source 1..10: mol_type = other DNA
cgactcatct

SEQ ID NO: 428 - DNA, 10 bp, synthetic construct
  misc_feature 1..10: note = 10 nt read_2 sequence
  source 1..10: mol_type = other DNA
ctgtggcgcg

SEQ ID NO: 429 - DNA, 10 bp, synthetic construct
  misc_feature 1..10: note = 10 nt read_2 sequence
  source 1..10: mol_type = other DNA
ttctactgcg

SEQ ID NO: 430 - DNA, 10 bp, synthetic construct
  misc_feature 1..10: note = 10 nt read_2 sequence
  source 1..10: mol_type = other DNA
accgagctgc

SEQ ID NO: 431 - DNA, 10 bp, synthetic construct
  misc_feature 1..10: note = 10 nt read_2 sequence
  source 1..10: mol_type = other DNA
gccgccgcct

SEQ ID NO: 432 - DNA, 10 bp, synthetic construct
  misc_feature 1..10: note = 10 nt read_2 sequence
  source 1..10: mol_type = other DNA
ggcggctagg

SEQ ID NO: 433 - DNA, 10 bp, synthetic construct
  misc_feature 1..10: note = 10 nt read_2 sequence
  source 1..10: mol_type = other DNA
agacgagctt

SEQ ID NO: 434 - DNA, 10 bp, synthetic construct
  misc_feature 1..10: note = 10 nt read_2 sequence
  source 1..10: mol_type = other DNA
aggagagcag

SEQ ID NO: 435 - DNA, 10 bp, synthetic construct
  misc_feature 1..10: note = 10 nt read_2 sequence
  source 1..10: mol_type = other DNA
taagagtggc

SEQ ID NO: 436 - DNA, 10 bp, synthetic construct
  misc_feature 1..10: note = 10 nt read_2 sequence
  source 1..10: mol_type = other DNA
ttgtatttgt

SEQ ID NO: 437 - DNA, 10 bp, synthetic construct
  misc_feature 1..10: note = 10 nt read_2 sequence
  source 1..10: mol_type = other DNA
gaggccacag

SEQ ID NO: 438 - DNA, 10 bp, synthetic construct
  misc_feature 1..10: note = 10 nt read_2 sequence
  source 1..10: mol_type = other DNA
agaggaggaa

SEQ ID NO: 439 - DNA, 10 bp, synthetic construct
  misc_feature 1..10: note = 10 nt read_2 sequence
  source 1..10: mol_type = other DNA
tccaacttga

SEQ ID NO: 440 - DNA, 10 bp, synthetic construct
  misc_feature 1..10: note = 10 nt read_2 sequence
  source 1..10: mol_type = other DNA
gcttggacgg

SEQ ID NO: 441 - DNA, 10 bp, synthetic construct
  misc_feature 1..10: note = 10 nt read_2 sequence
  source 1..10: mol_type = other DNA
gcatttgatc

SEQ ID NO: 442 - DNA, 10 bp, synthetic construct
  misc_feature 1..10: note = 10 nt read_2 sequence
  source 1..10: mol_type = other DNA
catcattgtt

SEQ ID NO: 443 - DNA, 10 bp, synthetic construct
  misc_feature 1..10: note = 10 nt read_2 sequence
  source 1..10: mol_type = other DNA
tttatctcca

SEQ ID NO: 444 - DNA, 10 bp, synthetic construct
  misc_feature 1..10: note = 10 nt read_2 sequence
  source 1..10: mol_type = other DNA
ctattagagg

SEQ ID NO: 445 - DNA, 10 bp, synthetic construct
  misc_feature 1..10: note = 10 nt read_2 sequence
  source 1..10: mol_type = other DNA
tctgagcaag

SEQ ID NO: 446 - DNA, 10 bp, synthetic construct
  misc_feature 1..10: note = 10 nt read_2 sequence
  source 1..10: mol_type = other DNA
ccagaacaca

SEQ ID NO: 447 - DNA, 10 bp, synthetic construct
  misc_feature 1..10: note = 10 nt read_2 sequence
  source 1..10: mol_type = other DNA
cttcacttgc

SEQ ID NO: 448 - DNA, 10 bp, synthetic construct
  misc_feature 1..10: note = 10 nt read_2 sequence
  source 1..10: mol_type = other DNA
gtgtctctct

SEQ ID NO: 449 - DNA, 10 bp, synthetic construct
  misc_feature 1..10: note = 10 nt read_2 sequence
  source 1..10: mol_type = other DNA
ccgaagaaag

SEQ ID NO: 450 - DNA, 10 bp, synthetic construct
  misc_feature 1..10: note = 10 nt read_2 sequence
  source 1..10: mol_type = other DNA
actagaaaat

SEQ ID NO: 451 - DNA, 10 bp, synthetic construct
  misc_feature 1..10: note = 10 nt read_2 sequence
  source 1..10: mol_type = other DNA
gtagttgcat

SEQ ID NO: 452 - DNA, 10 bp, synthetic construct
  misc_feature 1..10: note = 10 nt read_2 sequence
  source 1..10: mol_type = other DNA
cataggagcg

SEQ ID NO: 453 - DNA, 10 bp, synthetic construct
  misc_feature 1..10: note = 10 nt read_2 sequence
  source 1..10: mol_type = other DNA
ctcagactta

SEQ ID NO: 454 - DNA, 10 bp, synthetic construct
  misc_feature 1..10: note = 10 nt read_2 sequence
  source 1..10: mol_type = other DNA
caccaaccag

SEQ ID NO: 455 - DNA, 10 bp, synthetic construct
  misc_feature 1..10: note = 10 nt read_2 sequence
  source 1..10: mol_type = other DNA
ggaagataca

SEQ ID NO: 456 - DNA, 10 bp, synthetic construct
  misc_feature 1..10: note = 10 nt read_2 sequence
  source 1..10: mol_type = other DNA
ttttagattt

SEQ ID NO: 457 - DNA, 10 bp, synthetic construct
  misc_feature 1..10: note = 10 nt read_2 sequence
  source 1..10: mol_type = other DNA
tgtaggggcc

SEQ ID NO: 458 - DNA, 10 bp, synthetic construct
  misc_feature 1..10: note = 10 nt read_2 sequence
  source 1..10: mol_type = other DNA
tttgagtaaa

SEQ ID NO: 459 - DNA, 10 bp, synthetic construct
  misc_feature 1..10: note = 10 nt read_2 sequence
  source 1..10: mol_type = other DNA
catatcaagt

SEQ ID NO: 460 - DNA, 10 bp, synthetic construct
  misc_feature 1..10: note = 10 nt read_2 sequence
  source 1..10: mol_type = other DNA
atgtcagcaa

SEQ ID NO: 461 - DNA, 10 bp, synthetic construct
  misc_feature 1..10: note = 10 nt read_2 sequence
  source 1..10: mol_type = other DNA
caaccacaga

SEQ ID NO: 462 - DNA, 10 bp, synthetic construct
  misc_feature 1..10: note = 10 nt read_2 sequence
  source 1..10: mol_type = other DNA
aagaaaggta

SEQ ID NO: 463 - DNA, 10 bp, synthetic construct
  misc_feature 1..10: note = 10 nt read_2 sequence
  source 1..10: mol_type = other DNA
ggcctatgtg

SEQ ID NO: 464 - DNA, 10 bp, synthetic construct
  misc_feature 1..10: note = 10 nt read_2 sequence
  source 1..10: mol_type = other DNA
aggcgtggcc

SEQ ID NO: 465 - DNA, 10 bp, synthetic construct
  misc_feature 1..10: note = 10 nt read_2 sequence
  source 1..10: mol_type = other DNA
cctagcttgg

SEQ ID NO: 466 - DNA, 10 bp, synthetic construct
  misc_feature 1..10: note = 10 nt read_2 sequence
  source 1..10: mol_type = other DNA
tgaatcgggt

SEQ ID NO: 467 - DNA, 10 bp, synthetic construct
  misc_feature 1..10: note = 10 nt read_2 sequence
  source 1..10: mol_type = other DNA
agggagagca

SEQ ID NO: 468 - DNA, 10 bp, synthetic construct
  misc_feature 1..10: note = 10 nt read_2 sequence
  source 1..10: mol_type = other DNA
tgacacttac

SEQ ID NO: 469 - DNA, 10 bp, synthetic construct
  misc_feature 1..10: note = 10 nt read_2 sequence
  source 1..10: mol_type = other DNA
cctttttggt

SEQ ID NO: 470 - DNA, 10 bp, synthetic construct
  misc_feature 1..10: note = 10 nt read_2 sequence
  source 1..10: mol_type = other DNA
caaactcatc

SEQ ID NO: 471 - DNA, 10 bp, synthetic construct
  misc_feature 1..10: note = 10 nt read_2 sequence
  source 1..10: mol_type = other DNA
agtttgaccc

SEQ ID NO: 472 - DNA, 10 bp, synthetic construct
  misc_feature 1..10: note = 10 nt read_2 sequence
  source 1..10: mol_type = other DNA
aaggggagaa

SEQ ID NO: 473 - DNA, 10 bp, synthetic construct
  misc_feature 1..10: note = 10 nt read_2 sequence
  source 1..10: mol_type = other DNA
gttctgaagc

SEQ ID NO: 474 - DNA, 10 bp, synthetic construct
  misc_feature 1..10: note = 10 nt read_2 sequence
  source 1..10: mol_type = other DNA
ggcagtgttg

SEQ ID NO: 475 - DNA, 10 bp, synthetic construct
  misc_feature 1..10: note = 10 nt read_2 sequence
  source 1..10: mol_type = other DNA
accacagctg

SEQ ID NO: 476 - DNA, 10 bp, synthetic construct
  misc_feature 1..10: note = 10 nt read_2 sequence
  source 1..10: mol_type = other DNA
tcaggtgacc

SEQ ID NO: 477 - DNA, 10 bp, synthetic construct
  misc_feature 1..10: note = 10 nt read_2 sequence
  source 1..10: mol_type = other DNA
ggagcatata

SEQ ID NO: 478 - DNA, 10 bp, synthetic construct
  misc_feature 1..10: note = 10 nt read_2 sequence
  source 1..10: mol_type = other DNA
cctttcaaag

SEQ ID NO: 479 - DNA, 10 bp, synthetic construct
  misc_feature 1..10: note = 10 nt read_2 sequence
  source 1..10: mol_type = other DNA
atggggagga

SEQ ID NO: 480 - DNA, 10 bp, synthetic construct
  misc_feature 1..10: note = 10 nt read_2 sequence
  source 1..10: mol_type = other DNA
gatctggcca

SEQ ID NO: 481 - DNA, 10 bp, synthetic construct
  misc_feature 1..10: note = 10 nt read_2 sequence
  source 1..10: mol_type = other DNA
agcaaccaga

SEQ ID NO: 482 - DNA, 10 bp, synthetic construct
  misc_feature 1..10: note = 10 nt read_2 sequence
  source 1..10: mol_type = other DNA
caaaactagt

SEQ ID NO: 483 - DNA, 10 bp, synthetic construct
  misc_feature 1..10: note = 10 nt read_2 sequence
  source 1..10: mol_type = other DNA
aaggagcata

SEQ ID NO: 484 - DNA, 10 bp, synthetic construct
  misc_feature 1..10: note = 10 nt read_2 sequence
  source 1..10: mol_type = other DNA
agcctttcaa

SEQ ID NO: 485 - DNA, 10 bp, synthetic construct
  misc_feature 1..10: note = 10 nt read_2 sequence
  source 1..10: mol_type = other DNA
ggggaggatg

SEQ ID NO: 486 - DNA, 10 bp, synthetic construct
  misc_feature 1..10: note = 10 nt read_2 sequence
  source 1..10: mol_type = other DNA
gatatggcca

SEQ ID NO: 487 - DNA, 10 bp, synthetic construct
  misc_feature 1..10: note = 10 nt read_2 sequence
  source 1..10: mol_type = other DNA
ctcaaccaga

SEQ ID NO: 488 - DNA, 10 bp, synthetic construct
  misc_feature 1..10: note = 10 nt read_2 sequence
  source 1..10: mol_type = other DNA
cagaactagt

SEQ ID NO: 489 - DNA, 10 bp, synthetic construct
  misc_feature 1..10: note = 10 nt read_2 sequence
  source 1..10: mol_type = other DNA
ggaagtcccc

SEQ ID NO: 490 - DNA, 10 bp, synthetic construct
  misc_feature 1..10: note = 10 nt read_2 sequence
  source 1..10: mol_type = other DNA
gcctggtggg

SEQ ID NO: 491 - DNA, 10 bp, synthetic construct
  misc_feature 1..10: note = 10 nt read_2 sequence
  source 1..10: mol_type = other DNA
gcccagctcg

SEQ ID NO: 492 - DNA, 10 bp, synthetic construct
  misc_feature 1..10: note = 10 nt read_2 sequence
  source 1..10: mol_type = other DNA
aataggacta

SEQ ID NO: 493 - DNA, 10 bp, synthetic construct
  misc_feature 1..10: note = 10 nt read_2 sequence
  source 1..10: mol_type = other DNA
aagttcatgg

SEQ ID NO: 494 - DNA, 10 bp, synthetic construct
  misc_feature 1..10: note = 10 nt read_2 sequence
  source 1..10: mol_type = other DNA
gggctgacag

SEQ ID NO: 495 - DNA, 10 bp, synthetic construct
  misc_feature 1..10: note = 10 nt read_2 sequence
  source 1..10: mol_type = other DNA
cattgcttta

SEQ ID NO: 496 - DNA, 10 bp, synthetic construct
  misc_feature 1..10: note = 10 nt read_2 sequence
  source 1..10: mol_type = other DNA
tggagtcttg

SEQ ID NO: 497 - DNA, 10 bp, synthetic construct
  misc_feature 1..10: note = 10 nt read_2 sequence
  source 1..10: mol_type = other DNA
agtgcatgtg

SEQ ID NO: 498 - DNA, 10 bp, synthetic construct
  misc_feature 1..10: note = 10 nt read_2 sequence
  source 1..10: mol_type = other DNA
aatgagaagg

SEQ ID NO: 499 - DNA, 10 bp, synthetic construct
  misc_feature 1..10: note = 10 nt read_2 sequence
  source 1..10: mol_type = other DNA
ggaatctaag

SEQ ID NO: 500 - DNA, 10 bp, synthetic construct
  misc_feature 1..10: note = 10 nt read_2 sequence
  source 1..10: mol_type = other DNA
aagatggcat

SEQ ID NO: 501 - DNA, 10 bp, synthetic construct
  misc_feature 1..10: note = 10 nt read_2 sequence
  source 1..10: mol_type = other DNA
ggtaaagtcc

SEQ ID NO: 502 - DNA, 10 bp, synthetic construct
  misc_feature 1..10: note = 10 nt read_2 sequence
  source 1..10: mol_type = other DNA
tttattggcg

SEQ ID NO: 503 - DNA, 10 bp, synthetic construct
  misc_feature 1..10: note = 10 nt read_2 sequence
  source 1..10: mol_type = other DNA
gaaaaaaatt

SEQ ID NO: 504 - DNA, 10 bp, synthetic construct
  misc_feature 1..10: note = 10 nt read_2 sequence
  source 1..10: mol_type = other DNA
atatatcatt

SEQ ID NO: 505 - DNA, 10 bp, synthetic construct
  misc_feature 1..10: note = 10 nt read_2 sequence
  source 1..10: mol_type = other DNA
attagagaaa

SEQ ID NO: 506 - DNA, 10 bp, synthetic construct
  misc_feature 1..10: note = 10 nt read_2 sequence
  source 1..10: mol_type = other DNA
atactccatc

SEQ ID NO: 507 - DNA, 10 bp, synthetic construct
  misc_feature 1..10: note = 10 nt read_2 sequence
  source 1..10: mol_type = other DNA
cagtcaccac

SEQ ID NO: 508 - DNA, 10 bp, synthetic construct
  misc_feature 1..10: note = 10 nt read_2 sequence
  source 1..10: mol_type = other DNA
ttcttactgt

SEQ ID NO: 509 - DNA, 10 bp, synthetic construct
  misc_feature 1..10: note = 10 nt read_2 sequence
  source 1..10: mol_type = other DNA
tccgcatgca

SEQ ID NO: 510 - DNA, 10 bp, synthetic construct
  misc_feature 1..10: note = 10 nt read_2 sequence
  source 1..10: mol_type = other DNA
cttggcttgg

SEQ ID NO: 511 - DNA, 10 bp, synthetic construct
  misc_feature 1..10: note = 10 nt read_2 sequence
  source 1..10: mol_type = other DNA
gctgtgcata

SEQ ID NO: 512 - DNA, 10 bp, synthetic construct
  misc_feature 1..10: note = 10 nt read_2 sequence
  source 1..10: mol_type = other DNA
gaacagcagt

SEQ ID NO: 513 - DNA, 10 bp, synthetic construct
  misc_feature 1..10: note = 10 nt read_2 sequence
  source 1..10: mol_type = other DNA
agagaatgaa

SEQ ID NO: 514 - DNA, 10 bp, synthetic construct
  misc_feature 1..10: note = 10 nt read_2 sequence
  source 1..10: mol_type = other DNA
tattgcaagt

SEQ ID NO: 515 - DNA, 10 bp, synthetic construct
  misc_feature 1..10: note = 10 nt read_2 sequence
  source 1..10: mol_type = other DNA
aaaacttgtt

SEQ ID NO: 516 - DNA, 10 bp, synthetic construct
  misc_feature 1..10: note = 10 nt read_2 sequence
  source 1..10: mol_type = other DNA
gcagaagaag

SEQ ID NO: 517 - DNA, 10 bp, synthetic construct
  misc_feature 1..10: note = 10 nt read_2 sequence
  source 1..10: mol_type = other DNA
ctactcccac

SEQ ID NO: 518 - DNA, 10 bp, synthetic construct
  misc_feature 1..10: note = 10 nt read_2 sequence
  source 1..10: mol_type = other DNA
agtattcttt

SEQ ID NO: 519 - DNA, 10 bp, synthetic construct
  misc_feature 1..10: note = 10 nt read_2 sequence
  source 1..10: mol_type = other DNA
aatgaaaaca

SEQ ID NO: 520 - DNA, 10 bp, synthetic construct
  misc_feature 1..10: note = 10 nt read_2 sequence
  source 1..10: mol_type = other DNA
gtaatttcaa

SEQ ID NO: 521 - DNA, 10 bp, synthetic construct
  misc_feature 1..10: note = 10 nt read_2 sequence
  source 1..10: mol_type = other DNA
ctttcactta

SEQ ID NO: 522 - DNA, 10 bp, synthetic construct
  misc_feature 1..10: note = 10 nt read_2 sequence
  source 1..10: mol_type = other DNA
gtactttttt

SEQ ID NO: 523 - DNA, 10 bp, synthetic construct
  misc_feature 1..10: note = 10 nt read_2 sequence
  source 1..10: mol_type = other DNA
acagtaagat

SEQ ID NO: 524 - DNA, 10 bp, synthetic construct
  misc_feature 1..10: note = 10 nt read_2 sequence
  source 1..10: mol_type = other DNA
tacttgttaa

SEQ ID NO: 525 - DNA, 10 bp, synthetic construct
  misc_feature 1..10: note = 10 nt read_2 sequence
  source 1..10: mol_type = other DNA
ccaaaatctg

SEQ ID NO: 526 - DNA, 10 bp, synthetic construct
  misc_feature 1..10: note = 10 nt read_2 sequence
  source 1..10: mol_type = other DNA
tcaagtaggt

SEQ ID NO: 527 - DNA, 10 bp, synthetic construct
  misc_feature 1..10: note = 10 nt read_2 sequence
  source 1..10: mol_type = other DNA
cctgtccttt

SEQ ID NO: 528 - DNA, 10 bp, synthetic construct
  misc_feature 1..10: note = 10 nt read_2 sequence
  source 1..10: mol_type = other DNA
aacccctcga

SEQ ID NO: 529 - DNA, 10 bp, synthetic construct
  misc_feature 1..10: note = 10 nt read_2 sequence
  source 1..10: mol_type = other DNA
cataaatatg

SEQ ID NO: 530 - DNA, 10 bp, synthetic construct
  misc_feature 1..10: note = 10 nt read_2 sequence
  source 1..10: mol_type = other DNA
ttgcagcaag

SEQ ID NO: 531 - DNA, 10 bp, synthetic construct
  misc_feature 1..10: note = 10 nt read_2 sequence
  source 1..10: mol_type = other DNA
gagatcaagc

SEQ ID NO: 532 - DNA, 10 bp, synthetic construct
  misc_feature 1..10: note = 10 nt read_2 sequence
  source 1..10: mol_type = other DNA
gcaacagtga

SEQ ID NO: 533 - DNA, 10 bp, synthetic construct
  misc_feature 1..10: note = 10 nt read_2 sequence
  source 1..10: mol_type = other DNA
ctgccatttc

SEQ ID NO: 534 - DNA, 10 bp, synthetic construct
  misc_feature 1..10: note = 10 nt read_2 sequence
  source 1..10: mol_type = other DNA
aaggtaaaag

SEQ ID NO: 535 - DNA, 10 bp, synthetic construct
  misc_feature 1..10: note = 10 nt read_2 sequence
  source 1..10: mol_type = other DNA
gcggatctcc

SEQ ID NO: 536 - DNA, 10 bp, synthetic construct
  misc_feature 1..10: note = 10 nt read_2 sequence
  source 1..10: mol_type = other DNA
ctggtaggag

SEQ ID NO: 537 - DNA, 10 bp, synthetic construct
  misc_feature 1..10: note = 10 nt read_2 sequence
  source 1..10: mol_type = other DNA
ttttgaaatg

SEQ ID NO: 538 - DNA, 10 bp, synthetic construct
  misc_feature 1..10: note = 10 nt read_2 sequence
  source 1..10: mol_type = other DNA
tgccctaaaa

SEQ ID NO: 539 - DNA, 10 bp, synthetic construct
  misc_feature 1..10: note = 10 nt read_2 sequence
  source 1..10: mol_type = other DNA
gtataccagc

SEQ ID NO: 540 - DNA, 10 bp, synthetic construct
  misc_feature 1..10: note = 10 nt read_2 sequence
  source 1..10: mol_type = other DNA
ttcaacagat

SEQ ID NO: 541 - DNA, 10 bp, synthetic construct
  misc_feature 1..10: note = 10 nt read_2 sequence
  source 1..10: mol_type = other DNA
aggatgtgtc

SEQ ID NO: 542 - DNA, 10 bp, synthetic construct
  misc_feature 1..10: note = 10 nt read_2 sequence
  source 1..10: mol_type = other DNA
cctcagccag

SEQ ID NO: 543 - DNA, 10 bp, synthetic construct
  misc_feature 1..10: note = 10 nt read_2 sequence
  source 1..10: mol_type = other DNA
ctggtgtgga

SEQ ID NO: 544 - DNA, 10 bp, synthetic construct
  misc_feature 1..10: note = 10 nt read_2 sequence
  source 1..10: mol_type = other DNA
ctggtgcagg

SEQ ID NO: 545 - DNA, 10 bp, synthetic construct
  misc_feature 1..10: note = 10 nt read_2 sequence
  source 1..10: mol_type = other DNA
gtcatggtga

SEQ ID NO: 546 - DNA, 10 bp, synthetic construct
  misc_feature 1..10: note = 10 nt read_2 sequence
  source 1..10: mol_type = other DNA
ccggggccca

SEQ ID NO: 547 - DNA, 10 bp, synthetic construct
  misc_feature 1..10: note = 10 nt read_2 sequence
  source 1..10: mol_type = other DNA
ctgtaagtta

SEQ ID NO: 548 - DNA, 10 bp, synthetic construct
  misc_feature 1..10: note = 10 nt read_2 sequence
  source 1..10: mol_type = other DNA
agtaaaataa

SEQ ID NO: 549 - DNA, 10 bp, synthetic construct
  misc_feature 1..10: note = 10 nt read_2 sequence
  source 1..10: mol_type = other DNA
gaagcaaact

SEQ ID NO: 550 - DNA, 10 bp, synthetic construct
  misc_feature 1..10: note = 10 nt read_2 sequence
  source 1..10: mol_type = other DNA
aatggccatt

SEQ ID NO: 551 - DNA, 10 bp, synthetic construct
  misc_feature 1..10: note = 10 nt read_2 sequence
  source 1..10: mol_type = other DNA
cttgcgcctc

SEQ ID NO: 552 - DNA, 10 bp, synthetic construct
  misc_feature 1..10: note = 10 nt read_2 sequence
  source 1..10: mol_type = other DNA
gaaagctgta

SEQ ID NO: 553 - DNA, 10 bp, synthetic construct
  misc_feature 1..10: note = 10 nt read_2 sequence
  source 1..10: mol_type = other DNA
agttcctctg

SEQ ID NO: 554 - DNA, 10 bp, synthetic construct
  misc_feature 1..10: note = 10 nt read_2 sequence
  source 1..10: mol_type = other DNA
tctgtgggag

SEQ ID NO: 555 - DNA, 10 bp, synthetic construct
  misc_feature 1..10: note = 10 nt read_2 sequence
  source 1..10: mol_type = other DNA
caagcctggc

SEQ ID NO: 556 - DNA, 10 bp, synthetic construct
  misc_feature 1..10: note = 10 nt read_2 sequence
  source 1..10: mol_type = other DNA
tgtctggggc

SEQ ID NO: 557 - DNA, 10 bp, synthetic construct
  misc_feature 1..10: note = 10 nt read_2 sequence
  source 1..10: mol_type = other DNA
tgatgggtgg

SEQ ID NO: 558 - DNA, 10 bp, synthetic construct
  misc_feature 1..10: note = 10 nt read_2 sequence
  source 1..10: mol_type = other DNA
cagggtgcgg

SEQ ID NO: 559 - DNA, 10 bp, synthetic construct
  misc_feature 1..10: note = 10 nt read_2 sequence
  source 1..10: mol_type = other DNA
ctccaccttc

SEQ ID NO: 560 - DNA, 10 bp, synthetic construct
  misc_feature 1..10: note = 10 nt read_2 sequence
  source 1..10: mol_type = other DNA
tcgatccaaa

SEQ ID NO: 561 - DNA, 10 bp, synthetic construct
  misc_feature 1..10: note = 10 nt read_2 sequence
  source 1..10: mol_type = other DNA
ctgcagcaga

SEQ ID NO: 562 - DNA, 10 bp, synthetic construct
  misc_feature 1..10: note = 10 nt read_2 sequence
  source 1..10: mol_type = other DNA
actctttcac

SEQ ID NO: 563 - DNA, 10 bp, synthetic construct
  misc_feature 1..10: note = 10 nt read_2 sequence
  source 1..10: mol_type = other DNA
gcgtgtgatc

SEQ ID NO: 564 - DNA, 10 bp, synthetic construct
  misc_feature 1..10: note = 10 nt read_2 sequence
  source 1..10: mol_type = other DNA
acatcaaagc

SEQ ID NO: 565 - DNA, 10 bp, synthetic construct
  misc_feature 1..10: note = 10 nt read_2 sequence
  source 1..10: mol_type = other DNA
ctctgcccac

SEQ ID NO: 566 - DNA, 10 bp, synthetic construct
  misc_feature 1..10: note = 10 nt read_2 sequence
  source 1..10: mol_type = other DNA
tcatgtgatc

SEQ ID NO: 567 - DNA, 10 bp, synthetic construct
  misc_feature 1..10: note = 10 nt read_2 sequence
  source 1..10: mol_type = other DNA
tgcgacgtgg

SEQ ID NO: 568 - DNA, 10 bp, synthetic construct
  misc_feature 1..10: note = 10 nt read_2 sequence
  source 1..10: mol_type = other DNA
cttcacaaag

SEQ ID NO: 569 - DNA, 10 bp, synthetic construct
  misc_feature 1..10: note = 10 nt read_2 sequence
  source 1..10: mol_type = other DNA
actgtatgta

SEQ ID NO: 570 - DNA, 10 bp, synthetic construct
  misc_feature 1..10: note = 10 nt read_2 sequence
  source 1..10: mol_type = other DNA
attaatctgg

SEQ ID NO: 571 - DNA, 10 bp, synthetic construct
  misc_feature 1..10: note = 10 nt read_2 sequence
  source 1..10: mol_type = other DNA
cagatttgtt

SEQ ID NO: 572 - DNA, 10 bp, synthetic construct
  misc_feature 1..10: note = 10 nt read_2 sequence
  source 1..10: mol_type = other DNA
gcttaagcca

SEQ ID NO: 573 - DNA, 10 bp, synthetic construct
  misc_feature 1..10: note = 10 nt read_2 sequence
  source 1..10: mol_type = other DNA
tgtgtccagc

SEQ ID NO: 574 - DNA, 10 bp, synthetic construct
  misc_feature 1..10: note = 10 nt read_2 sequence
  source 1..10: mol_type = other DNA
atttgaaaca

SEQ ID NO: 575 - DNA, 10 bp, synthetic construct
  misc_feature 1..10: note = 10 nt read_2 sequence
  source 1..10: mol_type = other DNA
ataaagagag

SEQ ID NO: 576 - DNA, 10 bp, synthetic construct
  misc_feature 1..10: note = 10 nt read_2 sequence
  source 1..10: mol_type = other DNA
ttttcaagtt

SEQ ID NO: 577 - DNA, 10 bp, synthetic construct
  misc_feature 1..10: note = 10 nt read_2 sequence
  source 1..10: mol_type = other DNA
cgccccgcgt

SEQ ID NO: 578 - DNA, 10 bp, synthetic construct
  misc_feature 1..10: note = 10 nt read_2 sequence
  source 1..10: mol_type = other DNA
tagaggggct

SEQ ID NO: 579 - DNA, 10 bp, synthetic construct
  misc_feature 1..10: note = 10 nt read_2 sequence
  source 1..10: mol_type = other DNA
ggcgccgagg

SEQ ID NO: 580 - DNA, 10 bp, synthetic construct
  misc_feature 1..10: note = 10 nt read_2 sequence
  source 1..10: mol_type = other DNA
ccatacgggc

SEQ ID NO: 581 - DNA, 10 bp, synthetic construct
  misc_feature 1..10: note = 10 nt read_2 sequence
  source 1..10: mol_type = other DNA
ggtgtgggcc

SEQ ID NO: 582 - DNA, 10 bp, synthetic construct
  misc_feature 1..10: note = 10 nt read_2 sequence
  source 1..10: mol_type = other DNA
aagtggtcta

SEQ ID NO: 583 - DNA, 10 bp, synthetic construct
  misc_feature 1..10: note = 10 nt read_2 sequence
  source 1..10: mol_type = other DNA
cttgttcgtt

SEQ ID NO: 584 - DNA, 10 bp, synthetic construct
  misc_feature 1..10: note = 10 nt read_2 sequence
  source 1..10: mol_type = other DNA
atcaagactc

SEQ ID NO: 585 - DNA, 24 bp, Homo sapiens
  source 1..24: mol_type = unassigned DNA
ctggtgctccattcttgagtgtgt

SEQ ID NO: 586 - DNA, 24 bp, Homo sapiens
  source 1..24: mol_type = unassigned DNA
ggacaacaggttgtacagggatga

SEQ ID NO: 587 - DNA, 24 bp, Homo sapiens
  source 1..24: mol_type = unassigned DNA
tacaggagactggacatcgtcagg

SEQ ID NO: 588 - DNA, 24 bp, Homo sapiens
  source 1..24: mol_type = unassigned DNA
ctttctgcacatttgggtggtctt

SEQ ID NO: 589 - DNA, 24 bp, Homo sapiens
  source 1..24: mol_type = unassigned DNA
ggtgatcagatggacaatgcaaag

SEQ ID NO: 590 - DNA, 24 bp, Homo sapiens
  source 1..24: mol_type = unassigned DNA
tcatttccagaacattcagggtca

SEQ ID NO: 591 - DNA, 24 bp, Homo sapiens
  source 1..24: mol_type = unassigned DNA
acctcaatggcctaagcaagtgtc

SEQ ID NO: 592 - DNA, 24 bp, Homo sapiens
  source 1..24: mol_type = unassigned DNA
gcctcttacctgggtcacacattt

SEQ ID NO: 593 - DNA, 24 bp, Homo sapiens
  source 1..24: mol_type = unassigned DNA
atcttgcaacctggttcttcatgg

SEQ ID NO: 594 - DNA, 24 bp, Homo sapiens
  source 1..24: mol_type = unassigned DNA
gctggcaatgatgaaaactactcg

SEQ ID NO: 595 - DNA, 24 bp, Homo sapiens
  source 1..24: mol_type = unassigned DNA
ccaagtttcaactctgctctgctg

SEQ ID NO: 596 - DNA, 24 bp, Homo sapiens
  source 1..24: mol_type = unassigned DNA
gttgaacacggcattcttcctttc

SEQ ID NO: 597 - DNA, 24 bp, Homo sapiens
  source 1..24: mol_type = unassigned DNA
ggaaagggacgaactggtgtaatg

SEQ ID NO: 598 - DNA, 24 bp, Homo sapiens
  source 1..24: mol_type = unassigned DNA
aaatctagggcctcttgtgccttt

SEQ ID NO: 599 - DNA, 24 bp, Homo sapiens
  source 1..24: mol_type = unassigned DNA
agccccatggatctttctaccatt

SEQ ID NO: 600 - DNA, 24 bp, Homo sapiens
  source 1..24: mol_type = unassigned DNA
atactgccagggctcctgatactg

SEQ ID NO: 601 - DNA, 100 bp, synthetic construct
  misc_feature 1..100: note = Oligonucleotide capture probe
  source 1..100: mol_type = other DNA
aatcgggtaacattggctacaaagacctacctagatgctcctttttacgataacttacaggtgaaaaccaggatcaactcccgtgccagtcacatctcgt

SEQ ID NO: 602 - DNA, 100 bp, synthetic construct
  misc_feature 1..100: note = Oligonucleotide capture probe
  source 1..100: mol_type = other DNA
attataagtatcgacctcgtcggaaggcgaagatgctgccgaagaattgcagtttgcttcgtgaaaaccaggatcaactcccgtgccagtcacatctcgt

SEQ ID NO: 603 - DNA, 24 bp, Homo sapiens
  source 1..24: mol_type = unassigned DNA
ctggtgctccattcttgagtgtgt

SEQ ID NO: 604 - DNA, 24 bp, Homo sapiens
  source 1..24: mol_type = unassigned DNA
ggacaacaggttgtacagggatga

SEQ ID NO: 605 - DNA, 61 bp, synthetic construct
  misc_feature 1..61: note = qPCR Amplicon
  source 1..61: mol_type = other DNA
ctggtgctccattcttgagtgtgtggctttcgtacagtcatccctgtacaacctgttgtcc

SEQ ID NO: 606 - DNA, 60 bp, synthetic construct; identical to SEQ ID NO: 355
  misc_feature 1..60: note = Oligonucleotide probe
  source 1..60: mol_type = other DNA

SEQ ID NO: 607 - DNA, 60 bp, synthetic construct; identical to SEQ ID NO: 357
  misc_feature 1..60: note = Oligonucleotide probe
  source 1..60: mol_type = other DNA

SEQ ID NO: 608 - DNA, 60 bp, synthetic construct
  misc_feature 1..60: note = Oligonucleotide probe
  source 1..60: mol_type = other DNA
aatcgggtaacattggctacaaagacctacctagatgctcctttttacgataacttacag

SEQ ID NO: 609 - DNA, 60 bp, synthetic construct
  misc_feature 1..60: note = Oligonucleotide probe
  source 1..60: mol_type = other DNA
attataagtatcgacctcgtcggaaggcgaagatgctgccgaagaattgcagtttgcttc

SEQ ID NO: 610 - DNA, 24 bp, Homo sapiens
  source 1..24: mol_type = unassigned DNA
tacaggagactggacatcgtcagg

SEQ ID NO: 611 - DNA, 24 bp, Homo sapiens
  source 1..24: mol_type = unassigned DNA
ctttctgcacatttgggtggtctt

SEQ ID NO: 612 - DNA, 67 bp, synthetic construct
  misc_feature 1..67: note = qPCR amplicon
  source 1..67: mol_type = other DNA
tacaggagactggacatcgtcaggtcgctctacgaagatctggaagaccacccaaatgtgcagaaag

SEQ ID NO: 613 - DNA, 60 bp, synthetic construct; identical to SEQ ID NO: 391
  misc_feature 1..60: note = Oligonucleotide probe
  source 1..60: mol_type = other DNA

SEQ ID NO: 614 - DNA, 60 bp, synthetic construct; identical to SEQ ID NO: 392
  misc_feature 1..60: note = Oligonucleotide probe
  source 1..60: mol_type = other DNA

SEQ ID NO: 615 - DNA, 60 bp, synthetic construct
  misc_feature 1..60: note = Oligonucleotide probe
  source 1..60: mol_type = other DNA
gaagggcaaaaaccaaatcctcagtggcagactagggtctcagtacaaggaacgaacaag

SEQ ID NO: 616 - DNA, 60 bp, synthetic construct
  misc_feature 1..60: note = Oligonucleotide probe
  source 1..60: mol_type = other DNA
atttctgttgaaacttacactgtttcatctcagcttttgatggtactgatgagtcttgat

SEQ ID NO: 617 - DNA, 24 bp, Homo sapiens
  source 1..24: mol_type = unassigned DNA
ggtgatcagatggacaatgcaaag

SEQ ID NO: 618 - DNA, 24 bp, Homo sapiens
  source 1..24: mol_type = unassigned DNA
tcatttccagaacattcagggtca

SEQ ID NO: 619 - DNA, 73 bp, synthetic construct
  misc_feature 1..73: note = qPCR amplicon
  source 1..73: mol_type = other DNA
ggtgatcagatggacaatgcaaagcgcatggagactaagggagctggagtgaccctgaatgttctggaaatga

SEQ ID NO: 620 - DNA, 60 bp, synthetic construct; identical to SEQ ID NO: 381
  misc_feature 1..60: note = Oligonucleotide probe
  source 1..60: mol_type = other DNA

SEQ ID NO: 621 - DNA, 60 bp, synthetic construct; identical to SEQ ID NO: 382
  misc_feature 1..60: note = Oligonucleotide probe
  source 1..60: mol_type = other DNA

SEQ ID NO: 622 - DNA, 60 bp, synthetic construct
  misc_feature 1..60: note = Oligonucleotide probe
  source 1..60: mol_type = other DNA
tgagatgcaaaatagggaggatgtcagcagttacatctctgagtttcacagctggacaca

SEQ ID NO: 623 - DNA, 60 bp, synthetic construct
  misc_feature 1..60: note = Oligonucleotide probe
  source 1..60: mol_type = other DNA
aagaaagaagatacagaagaatactttggtcatggcattcatgataaaattgtttcaaat

SEQ ID NO: 624 - DNA, 24 bp, Homo sapiens
  source 1..24: mol_type = unassigned DNA
acctcaatggcctaagcaagtgtc

SEQ ID NO: 625 - DNA, 24 bp, Homo sapiens
  source 1..24: mol_type = unassigned DNA
gcctcttacctgggtcacacattt

SEQ ID NO: 626 - DNA, 57 bp, synthetic construct
  misc_feature 1..57: note = qPCR amplicon
  source 1..57: mol_type = other DNA
acctcaatggcctaagcaagtgtctgcagtgccaaatgtgtgacccaggtaagaggc

SEQ ID NO: 627 - DNA, 60 bp, synthetic construct; identical to SEQ ID NO: 365
  misc_feature 1..60: note = Oligonucleotide probe
  source 1..60: mol_type = other DNA

SEQ ID NO: 628 - DNA, 60 bp, synthetic construct; identical to SEQ ID NO: 366
  misc_feature 1..60: note = Oligonucleotide probe
  source 1..60: mol_type = other DNA

SEQ ID NO: 629 - DNA, 60 bp, synthetic construct
  misc_feature 1..60: note = Oligonucleotide probe
  source 1..60: mol_type = other DNA
cgcccagagagtgggaacttcgcaagtctgcgggaggccccttcgggagcccacccatca

SEQ ID NO: 630 - DNA, 60 bp, synthetic construct
  misc_feature 1..60: note = Oligonucleotide probe
  source 1..60: mol_type = other DNA
aagaggccagcacagccggcccagcctccgcttgggcagcctggatgcccccgcaccctg

SEQ ID NO: 631 - DNA, 24 bp, Homo sapiens
  source 1..24: mol_type = unassigned DNA
atcttgcaacctggttcttcatgg

SEQ ID NO: 632 - DNA, 24 bp, Homo sapiens
  source 1..24: mol_type = unassigned DNA
gctggcaatgatgaaaactactcg

SEQ ID NO: 633 - DNA, 74 bp, synthetic construct
  misc_feature 1..74: note = qPCR amplicon
  source 1..74: mol_type = other DNA
aatcttgcaacctggttcttcatggctgcggtagcatttctcagctcagccgagtagttttcatcattgccagc

SEQ ID NO: 634 - DNA, 60 bp, synthetic construct; identical to SEQ ID NO: 345
  misc_feature 1..60: note = Oligonucleotide probe
  source 1..60: mol_type = other DNA

SEQ ID NO: 635 - DNA, 60 bp, synthetic construct; identical to SEQ ID NO: 346
  misc_feature 1..60: note = Oligonucleotide probe
  source 1..60: mol_type = other DNA

SEQ ID NO: 636 - DNA, 60 bp, synthetic construct
  misc_feature 1..60: note = Oligonucleotide probe
  source 1..60: mol_type = other DNA
cgttatctgtcaaaactatgcttgaaacacgtttcatggcaacaaacccacatttcaaaa

SEQ ID NO: 637 - DNA, 60 bp, synthetic construct
  misc_feature 1..60: note = Oligonucleotide probe
  source 1..60: mol_type = other DNA
aaacaccagtcaaaggacaaatgcagacatcagggatgttatacatacacttttagggca

SEQ ID NO: 638 - DNA, 24 bp, Homo sapiens
  source 1..24: mol_type = unassigned DNA
ccaagtttcaactctgctctgctg

SEQ ID NO: 639 - DNA, 24 bp, Homo sapiens
  source 1..24: mol_type = unassigned DNA
gttgaacacggcattcttcctttc

SEQ ID NO: 640 - DNA, 60 bp, synthetic construct
  misc_feature 1..60: note = qPCR amplicon
  source 1..60: mol_type = other DNA
ccaagtttcaactctgctctgctgagaagtccaatcgaaaggaagaatgccgtgttcaac

SEQ ID NO: 641 - DNA, 60 bp, synthetic construct; identical to SEQ ID NO: 336
  misc_feature 1..60: note = Oligonucleotide probe
  source 1..60: mol_type = other DNA

SEQ ID NO: 642 - DNA, 60 bp, synthetic construct; identical to SEQ ID NO: 337
  misc_feature 1..60: note = Oligonucleotide probe
  source 1..60: mol_type = other DNA

SEQ ID NO: 643 - DNA, 60 bp, synthetic construct
  misc_feature 1..60: note = Oligonucleotide probe
  source 1..60: mol_type = other DNA
cagagagggtggttggccagaatcacactcctgctccaaaggtctgagcctcgaggggtt

SEQ ID NO: 644 - DNA, 60 bp, synthetic construct
  misc_feature 1..60: note = Oligonucleotide probe
  source 1..60: mol_type = other DNA
gagcagggcgctgcccttgggcagcacttgggtctaacaggactagcacacatatttatg

SEQ ID NO: 645 - DNA, 24 bp, Homo sapiens
  source 1..24: mol_type = unassigned DNA
ggaaagggacgaactggtgtaatg

SEQ ID NO: 646 - DNA, 24 bp, Homo sapiens
  source 1..24: mol_type = unassigned DNA
aaatctagggcctcttgtgccttt

SEQ ID NO: 647 - DNA, 83 bp, synthetic construct
  misc_feature 1..83: note = qPCR amplicon
  source 1..83: mol_type = other DNA
ggaaagggacgaactggtgtaatgatatgtgcatatttattacatcggggcaaatttttaaaggcacaagaggccctagattt

SEQ ID NO: 648 - DNA, 60 bp, synthetic construct; identical to SEQ ID NO: 332
  misc_feature 1..60: note = Oligonucleotide probe
  source 1..60: mol_type = other DNA

SEQ ID NO: 649 - DNA, 60 bp, synthetic construct; identical to SEQ ID NO: 333
  misc_feature 1..60: note = Oligonucleotide probe
  source 1..60: mol_type = other DNA

SEQ ID NO: 650 - DNA, 60 bp, synthetic construct
  misc_feature 1..60: note = Oligonucleotide probe
  source 1..60: mol_type = other DNA
tggtaaaaagataacctcagaataagaaaaaaaaactcttgaatttttaattaacaagta

SEQ ID NO: 651 - DNA, 60 bp, synthetic construct
  misc_feature 1..60: note = Oligonucleotide probe
  source 1..60: mol_type = other DNA
ttttgatgtttttcctttcctcttcctggatctgagaatttattggaaaacagattttgg

SEQ ID NO: 652 - DNA, 24 bp, Homo sapiens
  source 1..24: mol_type = unassigned DNA
agccccatggatctttctaccatt

SEQ ID NO: 653 - DNA, 24 bp, Homo sapiens
  source 1..24: mol_type = unassigned DNA
atactgccagggctcctgatactg

SEQ ID NO: 654 - DNA, 69 bp, synthetic construct
  misc_feature 1..69: note = qPCR amplicon
  source 1..69: mol_type = other DNA
agccccatggatctttctaccattaagaggaagttagacactggacagtatcaggagccctggcagtat

SEQ ID NO: 655 - DNA, 60 bp, synthetic construct; identical to SEQ ID NO: 314
  misc_feature 1..60: note = Oligonucleotide probe
  source 1..60: mol_type = other DNA

SEQ ID NO: 656 - DNA, 60 bp, synthetic construct; identical to SEQ ID NO: 315
  misc_feature 1..60: note = Oligonucleotide probe
  source 1..60: mol_type = other DNA

SEQ ID NO: 657 - DNA, 60 bp, synthetic construct
  misc_feature 1..60: note = Oligonucleotide probe
  source 1..60: mol_type = other DNA
gaaagacaagtgacatcaaacattactcaagtctcactatttttacgggagatggagtat

SEQ ID NO: 658 - DNA, 60 bp, synthetic construct
  misc_feature 1..60: note = Oligonucleotide probe
  source 1..60: mol_type = other DNA
atgtgtttcagatttgactttaacttttctgggatacctagaataatatagtggtgactg

SEQ ID NO: 659 - DNA, 40 bp, synthetic construct
  misc_feature 1..40: note = Oligonucleotide probe
  source 1..40: mol_type = other DNA
gtgaaaaccaggatcaactcccgtgccagtcacatctcgt

SEQ ID NO: 660 - DNA, 40 bp, synthetic construct
  misc_feature 1..40: note = Oligonucleotide probe
  source 1..40: mol_type = other DNA
acgagatgtgactggcacgggagttgatcctggttttcac

SEQ ID NO: 661 - DNA, 58 bp, synthetic construct; identical to SEQ ID NO: 69
  misc_feature 1..58: note = Primer
  source 1..58: mol_type = other DNA

SEQ ID NO: 662 - DNA, 57 bp, synthetic construct; identical to SEQ ID NO: 74
  misc_feature 1..57: note = Primer
  source 1..57: mol_type = other DNA

SEQ ID NO: 663 - DNA, 20 bp, synthetic construct
  misc_feature 1..20: note = Oligonucleotide probe
  modified_base 20: mod_base = OTHER; note = dideoxycytosine
  misc_feature 20: note = n is a, c, g, or t
  source 1..20: mol_type = other DNA
agttgatcctggttatacan

SEQ ID NO: 664 - DNA, 31 bp, synthetic construct
  misc_feature 1..31: note = Adaptor ligation strand oligonucleotide
  source 1..31: mol_type = other DNA
gtgtataaccaggatcaactcccgtgccagt

SEQ ID NO: 665 - DNA, 33 bp, synthetic construct
  misc_feature 1..33: note = Index 1 sequencing primer
  source 1..33: mol_type = other DNA
gtgaaaaccaggatcaactcccgtgccagtcac

SEQ ID NO: 666 - DNA, 30 bp, synthetic construct
  misc_feature 1..30: note = Library-free Forward sequencing primer
  source 1..30: mol_type = other DNA
gtcatgcaggagttgatcctggttatacac

SEQ ID NO: 667 - DNA, 25 bp, synthetic construct
  misc_feature 1..25: note = Post-processing amplification primer
  source 1..25: mol_type = other DNA
actggcacgggagttgatcctggtt

SEQ ID NO: 668 - DNA, 59 bp, synthetic construct
  misc_feature 1..59: note = Library-free forward amplification primer
  source 1..59: mol_type = other DNA
aatgatacggcgaccaccgagatctacacgtcatgcaggagttgatcctggttatacac

SEQ ID NO: 669 - DNA, 65 bp, synthetic construct
  misc_feature 1..65: note = Index N701 reverse primer
  source 1..65: mol_type = other DNA
caagcagaagacggcatacgagattcgccttagtgactggcacgggagttgatcctggttttcac

SEQ ID NO: 670 - DNA, 65 bp, synthetic construct
  misc_feature 1..65: note = Index N702 reverse primer
  source 1..65: mol_type = other DNA
caagcagaagacggcatacgagatctagtacggtgactggcacgggagttgatcctggttttcac

SEQ ID NO: 671 - DNA, 65 bp, synthetic construct
  misc_feature 1..65: note = Index N703 reverse primer
  source 1..65: mol_type = other DNA
caagcagaagacggcatacgagatttctgcctgtgactggcacgggagttgatcctggttttcac

SEQ ID NO: 672 - DNA, 65 bp, synthetic construct
  misc_feature 1..65: note = Index N704 reverse primer
  source 1..65: mol_type = other DNA
caagcagaagacggcatacgagatgctcaggagtgactggcacgggagttgatcctggttttcac

SEQ ID NO: 673 - DNA, 101 bp, synthetic construct
  misc_feature 1..101: note = Oligonucleotide probe
  modified_base 36..41: mod_base = OTHER; note = n = any nucleotide
  misc_feature 36..41: note = n is a, c, g, or t
  source 1..101: mol_type = other DNA
atgtgactggcacgggagttgatcctggttttcacnnnnnnaagcacctagccccattcctgctgagcaggaggtggcaggtaccccagactgggaggtaa

SEQ ID NO: 674 - DNA, 101 bp, synthetic construct
  misc_feature 1..101: note = Oligonucleotide probe
  misc_feature 36..41: note = n is a, c, g, or t
  source 1..101: mol_type = other DNA
atgtgactggcacgggagttgatcctggttttcacnnnnnnagtcggtggggccaggatgaggcccagtctgttcacacatggctgctgcctctcagctct

SEQ ID NO: 675 - DNA, 101 bp, synthetic construct
  misc_feature 1..101: note = Oligonucleotide probe
  misc_feature 36..41: note = n is a, c, g, or t
  source 1..101: mol_type = other DNA
atgtgactggcacgggagttgatcctggttttcacnnnnnnacctgagtagcatcattgtagttctcgatatctccacttccagttttacatttaccatca

SEQ ID NO: 676 - DNA, 101 bp, synthetic construct
  misc_feature 1..101: note = Oligonucleotide probe
  misc_feature 36..41: note = n is a, c, g, or t
  source 1..101: mol_type = other DNA
atgtgactggcacgggagttgatcctggttttcacnnnnnncctggccctcagccagtacagaaagtcatttgtcaaggccttcagttggcagacgtgctc

SEQ ID NO: 677 - DNA, 101 bp, synthetic construct
  misc_feature 1..101: note = Oligonucleotide probe
  misc_feature 36..41: note = n is a, c, g, or t
  source 1..101: mol_type = other DNA
atgtgactggcacgggagttgatcctggttttcacnnnnnnagaattcattgccagctataaatctgtggaaacgctgccacacaatcttagcacacaaga

SEQ ID NO: 678 - DNA, 101 bp, synthetic construct
  misc_feature 1..101: note = Oligonucleotide probe
  misc_feature 36..41: note = n is a, c, g, or t
  source 1..101: mol_type = other DNA
atgtgactggcacgggagttgatcctggttttcacnnnnnngacttcaaagaaattacaagttgacatcttggactctacccctcgtactttatctcctat

SEQ ID NO: 679 - DNA, 101 bp, synthetic construct
  misc_feature 1..101: note = Oligonucleotide probe
  misc_feature 36..41: note = n is a, c, g, or t
  source 1..101: mol_type = other DNA
atgtgactggcacgggagttgatcctggttttcacnnnnnntctctttggggtcaagaaagaatccctagtggatttgggattctagaggaggtgttataa

SEQ ID NO: 680 - DNA, 101 bp, synthetic construct
  misc_feature 1..101: note = Oligonucleotide probe
  misc_feature 36..41: note = n is a, c, g, or t
  source 1..101: mol_type = other DNA
atgtgactggcacgggagttgatcctggttttcacnnnnnntgcgataccatgctgaagatgagctaacccaaccagccaagcaggcagggctgcgaagga

SEQ ID NO: 681 - DNA, 101 bp, synthetic construct
  misc_feature 1..101: note = Oligonucleotide probe
  misc_feature 36..41: note = n is a, c, g, or t
  source 1..101: mol_type = other DNA
atgtgactggcacgggagttgatcctggttttcacnnnnnnggggtaggtggaaaacccaagtaatgtgattttgtaacatccactgctgcatttgtttgc

SEQ ID NO: 682 - DNA, 101 bp, synthetic construct
  misc_feature 1..101: note = Oligonucleotide probe
  misc_feature 36..41: note = n is a, c, g, or t
  source 1..101: mol_type = other DNA
atgtgactggcacgggagttgatcctggttttcacnnnnnnttacttccctccagttttgttgcttgcaaaacaacagaatcttctctccatgaaatcatg

SEQ ID NO: 683 - DNA, 101 bp, synthetic construct
  misc_feature 1..101: note = Oligonucleotide probe
  misc_feature 36..41: note = n is a, c, g, or t
  source 1..101: mol_type = other DNA
atgtgactggcacgggagttgatcctggttttcacnnnnnncaggggtatctattatccccattttctcacaaaggaaaccaagataaaaggtttaaatgg

SEQ ID NO: 684 - DNA, 101 bp, synthetic construct
  misc_feature 1..101: note = Oligonucleotide probe
  misc_feature 36..41: note = n is a, c, g, or t
  source 1..101: mol_type = other DNA
atgtgactggcacgggagttgatcctggttttcacnnnnnngaaattctcttgtgaattcctgtgtcctcttgaatcttcaatgctaaagtttttgaaact

SEQ ID NO: 685 - DNA, 101 bp, synthetic construct
  misc_feature 1..101: note = Oligonucleotide probe
  misc_feature 36..41: note = n is a, c, g, or t
  source 1..101: mol_type = other DNA
atgtgactggcacgggagttgatcctggttttcacnnnnnngggtttgagtggcatgagctacctactggatgtgcctgactgtttccccttcttcttccc

SEQ ID NO: 686 - DNA, 101 bp, synthetic construct
  misc_feature 1..101: note = Oligonucleotide probe
  misc_feature 36..41: note = n is a, c, g, or t
  source 1..101: mol_type = other DNA
atgtgactggcacgggagttgatcctggttttcacnnnnnnctatctccaggatggagagagggaaaaaaaagatgggtctgtgtgggagggcaggtactt

SEQ ID NO: 687 - DNA, 101 bp, synthetic construct
  misc_feature 1..101: note = Oligonucleotide probe
  misc_feature 36..41: note = n is a, c, g, or t
  source 1..101: mol_type = other DNA
atgtgactggcacgggagttgatcctggttttcacnnnnnngaaagaagccaggtcttcaattaataagattccctggtctcgtttgtctacctgttaatg

SEQ ID NO: 688 - DNA, 101 bp, synthetic construct
  misc_feature 1..101: note = Oligonucleotide probe
  misc_feature 36..41: note = n is a, c, g, or t
  source 1..101: mol_type = other DNA
atgtgactggcacgggagttgatcctggttttcacnnnnnncagactcgcgcccaattttcccccaccccttgttattgccacaaaatcctgaggatgatc

SEQ ID NO: 689 - DNA, 101 bp, synthetic construct
  misc_feature 1..101: note = Oligonucleotide probe
  misc_feature 36..41: note = n is a, c, g, or t
  source 1..101: mol_type = other DNA
atgtgactggcacgggagttgatcctggttttcacnnnnnntctttcttcttcctttatggggccctcctgctggctgagggcttctacaccaccggcgca

SEQ ID NO: 690 - DNA, 101 bp, synthetic construct
  misc_feature 1..101: note = Oligonucleotide probe
  misc_feature 36..41: note = n is a, c, g, or t
  source 1..101: mol_type = other DNA
atgtgactggcacgggagttgatcctggttttcacnnnnnngtttgtgtttctacatctgcaggctgatgctgatttctaaccaccccatgtcaatcattt

SEQ ID NO: 691 - DNA, 101 bp, synthetic construct
  misc_feature 1..101: note = Oligonucleotide probe
  misc_feature 36..41: note = n is a, c, g, or t
  source 1..101: mol_type = other DNA
atgtgactggcacgggagttgatcctggttttcacnnnnnnaaccaaatatatagtgcttccatagtgggtaggagagccaaagcacccgtaccctaactc

SEQ ID NO: 692 - DNA, 101 bp, synthetic construct
  misc_feature 1..101: note = Oligonucleotide probe
  misc_feature 36..41: note = n is a, c, g, or t
  source 1..101: mol_type = other DNA
atgtgactggcacgggagttgatcctggttttcacnnnnnnagtctccatgtggccccgtaactccataaagcttaccctgcttgctttttgtgtcttact

SEQ ID NO: 693 - DNA, 101 bp, synthetic construct
  misc_feature 1..101: note = Oligonucleotide probe
  misc_feature 36..41: note = n is a, c, g, or t
  source 1..101: mol_type = other DNA
atgtgactggcacgggagttgatcctggttttcacnnnnnnccatgggtgtaatttgtatggtattagctactcccttgtaaaataacccaaataacccac

SEQ ID NO: 694 - DNA, 101 bp, synthetic construct
  misc_feature 1..101: note = Oligonucleotide probe
  misc_feature 36..41: note = n is a, c, g, or t
  source 1..101: mol_type = other DNA
atgtgactggcacgggagttgatcctggttttcacnnnnnntttacagtggagcatattactgctgttgcaagaaacagttcttcctctttcattttcctg

SEQ ID NO: 695 - DNA, 101 bp, synthetic construct
  misc_feature 1..101: note = Oligonucleotide probe
  misc_feature 36..41: note = n is a, c, g, or t
  source 1..101: mol_type = other DNA
atgtgactggcacgggagttgatcctggttttcacnnnnnnatagctgtacccacactatctcaggcctatttacttgccaagatcattcaaagtcaactc

SEQ ID NO: 696 - DNA, 101 bp, synthetic construct
  misc_feature 1..101: note = Oligonucleotide probe
  misc_feature 36..41: note = n is a, c, g, or t
  source 1..101: mol_type = other DNA
atgtgactggcacgggagttgatcctggttttcacnnnnnngatttgaggagggagtgctttcttttctactctcattcacattctctcttctgttcccta

SEQ ID NO: 697 - DNA, 101 bp, synthetic construct
  misc_feature 1..101: note = Oligonucleotide probe
  misc_feature 36..41: note = n is a, c, g, or t
  source 1..101: mol_type = other DNA
atgtgactggcacgggagttgatcctggttttcacnnnnnncagcattgtaggctgtgtggttagagcctcgctattagagaaagggggatttctacgggg

SEQ ID NO: 698 - DNA, 101 bp, synthetic construct
  misc_feature 1..101: note = Oligonucleotide probe
  misc_feature 36..41: note = n is a, c, g, or t
  source 1..101: mol_type = other DNA
atgtgactggcacgggagttgatcctggttttcacnnnnnntgttacctttaaaagacatctgctttctgccaaaattaatgtgctgaacttaaacttacc

SEQ ID NO: 699 - DNA, 101 bp, synthetic construct
  misc_feature 1..101: note = Oligonucleotide probe
  misc_feature 36..41: note = n is a, c, g, or t
  source 1..101: mol_type = other DNA
atgtgactggcacgggagttgatcctggttttcacnnnnnnttcccagtaaattactcttaccaatgcaacagactttaaagaagttgtgttttacaatgc

SEQ ID NO: 700 - DNA, 101 bp, synthetic construct
  misc_feature 1..101: note = Oligonucleotide probe
  misc_feature 36..41: note = n is a, c, g, or t
  source 1..101: mol_type = other DNA
atgtgactggcacgggagttgatcctggttttcacnnnnnntaaatgacataacagttatgattttgcagaaaacagatctgtatttatttcagtgttact

SEQ ID NO: 701 - DNA, 101 bp, synthetic construct
  misc_feature 1..101: note = Oligonucleotide probe
  misc_feature 36..41: note = n is a, c, g, or t
  source 1..101: mol_type = other DNA
atgtgactggcacgggagttgatcctggttttcacnnnnnngacaggttttgaaagatatttgtgttactaatgactgtgctataacttttttttctttcc

SEQ ID NO: 702 - DNA, 101 bp, synthetic construct
  misc_feature 1..101: note = Oligonucleotide probe
  misc_feature 36..41: note = n is a, c, g, or t
  source 1..101: mol_type = other DNA
atgtgactggcacgggagttgatcctggttttcacnnnnnnactcaaaaaataaaaactataattactccttaatgtcagcttattatattcaatttaaac

SEQ ID NO: 703 - DNA, 101 bp, synthetic construct
  misc_feature 1..101: note = Oligonucleotide probe
  misc_feature 36..41: note = n is a, c, g, or t
  source 1..101: mol_type = other DNA
atgtgactggcacgggagttgatcctggttttcacnnnnnnaacaccttttttgaagtaaaaggtgcactgtaataatccagactgtgtttctcccttctc

SEQ ID NO: 704 - DNA, 101 bp, synthetic construct
  misc_feature 1..101: note = Oligonucleotide probe
  misc_feature 36..41: note = n is a, c, g, or t
  source 1..101: mol_type = other DNA
atgtgactggcacgggagttgatcctggttttcacnnnnnngaaacctttatctgtatcaaagaatggtcctgcaccagtaatatgcatattaaaacaaga

SEQ ID NO: 705 - DNA, 101 bp, synthetic construct
  misc_feature 1..101: note = Oligonucleotide probe
  misc_feature 36..41: note = n is a, c, g, or t
  source 1..101: mol_type = other DNA
atgtgactggcacgggagttgatcctggttttcacnnnnnngtgtattaaccttatgtgtgacatgttctaatatagtcacattttcattatttttattat

SEQ ID NO: 706 - DNA, 101 bp, synthetic construct
  misc_feature 1..101: note = Oligonucleotide probe
  misc_feature 36..41: note = n is a, c, g, or t
  source 1..101: mol_type = other DNA
atgtgactggcacgggagttgatcctggttttcacnnnnnnccccagccagcggtccgcaacccttgccgcatccacgaaactttgcccatagcagcgggc

SEQ ID NO: 707 - DNA, 101 bp, synthetic construct
  misc_feature 1..101: note = Oligonucleotide probe
  misc_feature 36..41: note = n is a, c, g, or t
  source 1..101: mol_type = other DNA
atgtgactggcacgggagttgatcctggttttcacnnnnnncgactcatctcagcattaaagtgataaaaaaataaattaaaaggcaagtggacttcggtg

SEQ ID NO: 708 - DNA, 101 bp, synthetic construct
  misc_feature 1..101: note = Oligonucleotide probe
  misc_feature 36..41: note = n is a, c, g, or t
  source 1..101: mol_type = other DNA
atgtgactggcacgggagttgatcctggttttcacnnnnnnctgtggcgcgcactgcgcgctgcgccaggtttccgcaccaagacccctttaactcaagac

SEQ ID NO: 709 - DNA, 101 bp, synthetic construct
  misc_feature 1..101: note = Oligonucleotide probe
  misc_feature 36..41: note = n is a, c, g, or t
  source 1..101: mol_type = other DNA
atgtgactggcacgggagttgatcctggttttcacnnnnnnttctactgcgacgaggaggagaacttctaccagcagcagcagcagagcgagctgcagccc

SEQ ID NO: 710 - DNA, 101 bp, synthetic construct
  misc_feature 1..101: note = Oligonucleotide probe
  misc_feature 36..41: note = n is a, c, g, or t
  source 1..101: mol_type = other DNA
atgtgactggcacgggagttgatcctggttttcacnnnnnnaccgagctgctgggaggagacatggtgaaccagagtttcatctgcgacccggacgacgag

SEQ ID NO: 711 - DNA, 101 bp, synthetic construct
  misc_feature 1..101: note = Oligonucleotide probe
  misc_feature 36..41: note = n is a, c, g, or t
  source 1..101: mol_type = other DNA
atgtgactggcacgggagttgatcctggttttcacnnnnnngccgccgcctcagagtgcatcgacccctcggtggtcttcccctaccctctcaacgacagc

SEQ ID NO: 712 - DNA, 101 bp, synthetic construct
  misc_feature 1..101: note = Oligonucleotide probe
  misc_feature 36..41: note = n is a, c, g, or t
  source 1..101: mol_type = other DNA
atgtgactggcacgggagttgatcctggttttcacnnnnnnggcggctaggggacaggggcggggtgggcagcagctcgaatttcttccagatatcctcgc

SEQ ID NO: 713 - DNA, 101 bp, synthetic construct
  misc_feature 1..101: note = Oligonucleotide probe
  misc_feature 36..41: note = n is a, c, g, or t
  source 1..101: mol_type = other DNA
atgtgactggcacgggagttgatcctggttttcacnnnnnnagacgagcttggcggcggccgagaagccgctccacatacagtcctggatgatgatgtttt

SEQ ID NO: 714 - DNA, 101 bp, synthetic construct
  misc_feature 1..101: note = Oligonucleotide probe
  misc_feature 36..41: note = n is a, c, g, or t
  source 1..101: mol_type = other DNA
atgtgactggcacgggagttgatcctggttttcacnnnnnnaggagagcagagaatccgaggacggagagaaggcgctggagtcttgcgaggcgcaggact

SEQ ID NO: 715 - DNA, 101 bp, synthetic construct
  misc_feature 1..101: note = Oligonucleotide probe
  misc_feature 36..41: note = n is a, c, g, or t
  source 1..101: mol_type = other DNA
atgtgactggcacgggagttgatcctggttttcacnnnnnntaagagtggcccgttaaataagctgccaatgaaaatgggaaaggtatccagccgcccact

SEQ ID NO: 716 - DNA, 101 bp, synthetic construct
  misc_feature 1..101: note = Oligonucleotide probe
  misc_feature 36..41: note = n is a, c, g, or t
  source 1..101: mol_type = other DNA
atgtgactggcacgggagttgatcctggttttcacnnnnnnttgtatttgtacagcattaatctggtaattgattattttaatgtaaccttgctaaaggag

SEQ ID NO: 717 - DNA, 101 bp, synthetic construct
  misc_feature 1..101: note = Oligonucleotide probe
  misc_feature 36..41: note = n is a, c, g, or t
  source 1..101: mol_type = other DNA
atgtgactggcacgggagttgatcctggttttcacnnnnnngaggccacagcaaacctcctcacagcccactggtcctcaagaggtgccacgtctccacac

SEQ ID NO: 718 - DNA, 101 bp, synthetic construct
  misc_feature 1..101: note = Oligonucleotide probe
  misc_feature 36..41: note = n is a, c, g, or t
  source 1..101: mol_type = other DNA
atgtgactggcacgggagttgatcctggttttcacnnnnnnagaggaggaacgagctaaaacggagcttttttgccctgcgtgaccagatcccggagttgg

SEQ ID NO: 719 - DNA, 101 bp, synthetic construct
  misc_feature 1..101: note = Oligonucleotide probe
  misc_feature 36..41: note = n is a, c, g, or t
  source 1..101: mol_type = other DNA
atgtgactggcacgggagttgatcctggttttcacnnnnnntccaacttgaccctcttggcagcaggatagtccttccgagtggagggaggcgctgcgtag

SEQ ID NO: 720 - DNA, 101 bp, synthetic construct
  misc_feature 1..101: note = Oligonucleotide probe
  misc_feature 36..41: note = n is a, c, g, or t
  source 1..101: mol_type = other DNA
atgtgactggcacgggagttgatcctggttttcacnnnnnngcttggacggacaggatgtatgctgtggcttttttaaggataactaccttgggggccttt

SEQ ID NO: 721 - DNA, 101 bp, synthetic construct
  misc_feature 1..101: note = Oligonucleotide probe
  misc_feature 36..41: note = n is a, c, g, or t
  source 1..101: mol_type = other DNA
atgtgactggcacgggagttgatcctggttttcacnnnnnngcatttgatcatgcatttgaaacaagttcataggtgattgctcaggacatttctgttaga

SEQ ID NO: 722 - DNA, 20 bp, synthetic construct
  misc_feature 1..20: note = poly- dT primer
  modified_base 20: mod_base = OTHER; note = n = any nucleotide
  misc_feature 20: note = n is a, c, g, or t
  source 1..20: mol_type = other DNA
ttttttttttttttttttvn

SEQ ID NO: 723 - DNA, 45 bp, synthetic construct
  misc_feature 1..45: note = oligonucleotide aptamer
  misc_feature 26..33: note = n is a, c, g, or t
  modified_base 36..43: mod_base = OTHER; note = n = any nucleotide
  source 1..45: mol_type = other DNA
tgcaggaccagagaattcgaatacannnnnnnngactccgatccc

SEQ ID NO: 724 - DNA, 12 bp, synthetic construct
  misc_feature 1..12: note = Oligonucleotide aptamer
  source 1..12: mol_type = other DNA
gggatcggagtc

SEQ ID NO: 725 - DNA, 45 bp, synthetic construct
  misc_feature 1..45: note = Oligonucleotide aptamer
  misc_feature 26..33: note = n is a, c, g, or t
  modified_base 36..43: mod_base = OTHER; note = n = any nucleotide
  source 1..45: mol_type = other DNA
tgcaggaccagagaattcgaatacannnnnnnncggaactcggag

SEQ ID NO: 726 - DNA, 12 bp, synthetic construct
  misc_feature 1..12: note = Oligonucleotide aptamer
  source 1..12: mol_type = other DNA
ctccgagttccg

SEQ ID NO: 727 - DNA, 101 bp, synthetic construct
  misc_feature 1..101: note = Oligonucleotide probe
  misc_feature 36..41: note = n is a, c, g, or t
  source 1..101: mol_type = other DNA
atgtgactggcacgggagttgatcctggttttcacnnnnnngccgaagaggaaatgctggaaaatgtcagcctggtctgtccaaaagatgcgacccgattc

SEQ ID NO: 728 - DNA, 100 bp, synthetic construct
  misc_feature 1..100: note = Oligonucleotide probe
  misc_feature 36..41: note = n is a, c, g, or t
  source 1..100: mol_type = other DNA
atgtgactggcacgggagttgatcctggttttcacnnnnnncagctgacctcatcgagattggcttggaaggaaaaggctttgagccaacattggaagct

SEQ ID NO: 729 - DNA, 101 bp, synthetic construct
  misc_feature 1..101: note = Oligonucleotide probe
  misc_feature 36..41: note = n is a, c, g, or t
  source 1..101: mol_type = other DNA
atgtgactggcacgggagttgatcctggttttcacnnnnnntactggagacaggctggactcagctacatccgatactcccagatctgtgcaaaagcagtg

SEQ ID NO: 730 - DNA, 101 bp, synthetic construct
  misc_feature 1..101: note = Oligonucleotide probe
  misc_feature 36..41: note = n is a, c, g, or t
  source 1..101: mol_type = other DNA
atgtgactggcacgggagttgatcctggttttcacnnnnnnctgaagacagaattcaaagcaaatgctgagaagacttctggcagcaacgtaaaaattgtg

SEQ ID NO: 731 - DNA, 101 bp, synthetic construct
  misc_feature 1..101: note = Oligonucleotide probe
  misc_feature 36..41: note = n is a, c, g, or t
  source 1..101: mol_type = other DNA
atgtgactggcacgggagttgatcctggttttcacnnnnnnacagagtccagcccattgagagaatcaactgccataggttttacacctgagttagaaagt

SEQ ID NO: 732 - DNA, 100 bp, synthetic construct
  misc_feature 1..100: note = Oligonucleotide probe
  misc_feature 36..41: note = n is a, c, g, or t
  source 1..100: mol_type = other DNA
atgtgactggcacgggagttgatcctggttttcacnnnnnnagccagctccagtgacagtgacgacggcttgcaccagtttcttcggggtacctccagca

SEQ ID NO: 733 - DNA, 100 bp, synthetic construct
  misc_feature 1..100: note = Oligonucleotide probe
  misc_feature 36..41: note = n is a, c, g, or t
  source 1..100: mol_type = other DNA
atgtgactggcacgggagttgatcctggttttcacnnnnnngacacgcagcacaaattgcgcagcgcggtggaagagatggaggcagaagaagctgctgc

SEQ ID NO: 734 - DNA, 100 bp, synthetic construct
  misc_feature 1..100: note = Oligonucleotide probe
  misc_feature 36..41: note = n is a, c, g, or t
  source 1..100: mol_type = other DNA
atgtgactggcacgggagttgatcctggttttcacnnnnnntggtgtatgtgtgcaagccgaccttcgtggggagccgtgaccaagatggggagatcctg

SEQ ID NO: 735 - DNA, 101 bp, synthetic construct
  misc_feature 1..101: note = Oligonucleotide probe
  misc_feature 36..41: note = n is a, c, g, or t
  source 1..101: mol_type = other DNA
atgtgactggcacgggagttgatcctggttttcacnnnnnnatgaggatcgtctgcctggtcctaagtgtggtgggcacagcatggactgcagatagtggt

SEQ ID NO: 736 - DNA, 100 bp, synthetic construct
  misc_feature 1..100: note = Oligonucleotide probe
  misc_feature 36..41: note = n is a, c, g, or t
  source 1..100: mol_type = other DNA
atgtgactggcacgggagttgatcctggttttcacnnnnnnattttttctgtttattgcgatcaagagaccagtttgggaggatggcttttgatccagca

SEQ ID NO: 737 - DNA, 101 bp, synthetic construct
  misc_feature 1..101: note = Oligonucleotide probe
  misc_feature 36..41: note = n is a, c, g, or t
  source 1..101: mol_type = other DNA
atgtgactggcacgggagttgatcctggttttcacnnnnnngtgttcagtttcatccttgttaccaccgctctgacaatgggcagggaaatttcggcgctc

SEQ ID NO: 738 - DNA, 100 bp, synthetic construct
  misc_feature 1..100: note = Oligonucleotide probe
  misc_feature 36..41: note = n is a, c, g, or t
  source 1..100: mol_type = other DNA
atgtgactggcacgggagttgatcctggttttcacnnnnnntgcaaacctgaatggtgtatactacagcggcccctacacggctaaaacagacaatggga

SEQ ID NO: 739 - DNA, 100 bp, synthetic construct
  misc_feature 1..100: note = Oligonucleotide probe
  misc_feature 36..41: note = n is a, c, g, or t
  source 1..100: mol_type = other DNA
atgtgactggcacgggagttgatcctggttttcacnnnnnncatccccaacgtacccgccgacaccaaactctccaaaatcaagaccctgcgcctggcca

SEQ ID NO: 740 - DNA, 100 bp, synthetic construct
  misc_feature 1..100: note = Oligonucleotide probe
  misc_feature 36..41: note = n is a, c, g, or t
  source 1..100: mol_type = other DNA
atgtgactggcacgggagttgatcctggttttcacnnnnnncgaccagaatggcgaggcggaggccttcaaggcagagatcaagaagaccgacgtgaaag

SEQ ID NO: 741 - DNA, 101 bp, synthetic construct
  misc_feature 1..101: note = Oligonucleotide probe
  misc_feature 36..41: note = n is a, c, g, or t
  source 1..101: mol_type = other DNA
atgtgactggcacgggagttgatcctggttttcacnnnnnnctgatccttcttgccatcctggccgccttagcggtagtaactttgtgttatgaatcacat

SEQ ID NO: 742 - DNA, 100 bp, synthetic construct
  misc_feature 1..100: note = Oligonucleotide probe
  misc_feature 36..41: note = n is a, c, g, or t
  source 1..100: mol_type = other DNA
atgtgactggcacgggagttgatcctggttttcacnnnnnncgagctcaatagggaagcctgtgatgactacagactttgcgaacgctacgccatggttt

SEQ ID NO: 743 - DNA, 100 bp, synthetic construct
  misc_feature 1..100: note = Oligonucleotide probe
  misc_feature 36..41: note = n is a, c, g, or t
  source 1..100: mol_type = other DNA
atgtgactggcacgggagttgatcctggttttcacnnnnnnaagaagtatcttcgaacagatgacagagtagaacgtgtacgcagagcccacctgaatga

SEQ ID NO: 744 - DNA, 100 bp, synthetic construct
  misc_feature 1..100: note = Oligonucleotide probe
  misc_feature 36..41: note = n is a, c, g, or t
  source 1..100: mol_type = other DNA
atgtgactggcacgggagttgatcctggttttcacnnnnnntattccttgagtggtcccgacccctctacagccatcctgcacttcagactatttgtcgg

SEQ ID NO: 745 - DNA, 101 bp, synthetic construct
  misc_feature 1..101: note = Oligonucleotide probe
  misc_feature 36..41: note = n is a, c, g, or t
  source 1..101: mol_type = other DNA
atgtgactggcacgggagttgatcctggttttcacnnnnnncagaccaggccttttgacctcaagaaggatgtcttcgtgcctgatgacaaacaggagttt

SEQ ID NO: 746 - DNA, 100 bp, synthetic construct
  misc_feature 1..100: note = Oligonucleotide probe
  misc_feature 36..41: note = n is a, c, g, or t
  source 1..100: mol_type = other DNA
atgtgactggcacgggagttgatcctggttttcacnnnnnnagagctcttcaaactcaagaacgcctatgaggagtccctggaacatctggagaccttca

SEQ ID NO: 747 - DNA, 101 bp, synthetic construct
  misc_feature 1..101: note = Oligonucleotide probe
  misc_feature 36..41: note = n is a, c, g, or t
  source 1..101: mol_type = other DNA
atgtgactggcacgggagttgatcctggttttcacnnnnnncaggtcttctataagcctgttattgaagacttaagcatggaattggccagaaaatgcacg

SEQ ID NO: 748 - DNA, 100 bp, synthetic construct
  misc_feature 1..100: note = Oligonucleotide probe
  misc_feature 36..41: note = n is a, c, g, or t
  source 1..100: mol_type = other DNA
atgtgactggcacgggagttgatcctggttttcacnnnnnnaaagagcaaaactacaaggccactccggtaagcatgaccccggagatagagagagtgag

SEQ ID NO: 749 - DNA, 101 bp, synthetic construct
  misc_feature 1..101: note = Oligonucleotide probe
  misc_feature 36..41: note = n is a, c, g, or t
  source 1..101: mol_type = other DNA
atgtgactggcacgggagttgatcctggttttcacnnnnnnggatatcgcactctgtcccagcacctcaatgacctgaagaaggagaacttcagcctcaag

SEQ ID NO: 750 - DNA, 100 bp, synthetic construct
  misc_feature 1..100: note = Oligonucleotide probe
  misc_feature 36..41: note = n is a, c, g, or t
  source 1..100: mol_type = other DNA
atgtgactggcacgggagttgatcctggttttcacnnnnnngaaagccaagctgctgcagagaagttggtgcaagccttaatggaaagaaattcagaatt

SEQ ID NO: 751 - DNA, 101 bp, synthetic construct
  misc_feature 1..101: note = Oligonucleotide probe
  misc_feature 36..41: note = n is a, c, g, or t
  source 1..101: mol_type = other DNA
atgtgactggcacgggagttgatcctggttttcacnnnnnnccggacgaggattcttctaacagagaaaatgccattgaggatgaagaggaggaggaggag

SEQ ID NO: 752 - DNA, 100 bp, synthetic construct
  misc_feature 1..100: note = Oligonucleotide probe
  misc_feature 36..41: note = n is a, c, g, or t
  source 1..100: mol_type = other DNA
atgtgactggcacgggagttgatcctggttttcacnnnnnncgtcaaggtcgtggtgggaaagacctttgactccattgtgatggaccccaagaaggacg

SEQ ID NO: 753 - DNA, 100 bp, synthetic construct
  misc_feature 1..100: note = Oligonucleotide probe
  misc_feature 36..41: note = n is a, c, g, or t
  source 1..100: mol_type = other DNA
atgtgactggcacgggagttgatcctggttttcacnnnnnnagatcacgagttatgaaaaacctcctcctgggcttatcaaggttggcattgcaaatggt

SEQ ID NO: 754 - DNA, 101 bp, synthetic construct
  misc_feature 1..101: note = Oligonucleotide probe
  misc_feature 36..41: note = n is a, c, g, or t
  source 1..101: mol_type = other DNA
atgtgactggcacgggagttgatcctggttttcacnnnnnnaaagtttcttcatcgttgtcctccctgctggtcacatgagtttacgattccttagaagtg

SEQ ID NO: 755 - DNA, 100 bp, synthetic construct
  misc_feature 1..100: note = Oligonucleotide probe
  misc_feature 36..41: note = n is a, c, g, or t
  source 1..100: mol_type = other DNA
atgtgactggcacgggagttgatcctggttttcacnnnnnncccggcgcgttccgactggctgccaggatgtacctgcagaaaggatttcccatcaaaga

SEQ ID NO: 756 - DNA, 100 bp, synthetic construct
  misc_feature 1..100: note = Oligonucleotide probe
  misc_feature 36..41: note = n is a, c, g, or t
  source 1..100: mol_type = other DNA
atgtgactggcacgggagttgatcctggttttcacnnnnnngcctgaaaggcttcccccgcggagacaagcttttcggccctgacttaaaacttgtgccc

SEQ ID NO: 757 - DNA, 100 bp, synthetic construct
  misc_feature 1..100: note = Oligonucleotide probe
  misc_feature 36..41: note = n is a, c, g, or t
  source 1..100: mol_type = other DNA
atgtgactggcacgggagttgatcctggttttcacnnnnnnaacaacctgaacgtcaccgaggagaagtaccaggaggcgttggccaagggagatgttac

SEQ ID NO: 758 - DNA, 100 bp, synthetic construct
  misc_feature 1..100: note = Oligonucleotide probe
  misc_feature 36..41: note = n is a, c, g, or t
  source 1..100: mol_type = other DNA
atgtgactggcacgggagttgatcctggttttcacnnnnnnaggagaagctgacggctgcatctgttggtgtccaaggctcaggttggggttggcttggt

SEQ ID NO: 759 - DNA, 101 bp, synthetic construct
  misc_feature 1..101: note = Oligonucleotide probe
  misc_feature 36..41: note = n is a, c, g, or t
  source 1..101: mol_type = other DNA
atgtgactggcacgggagttgatcctggttttcacnnnnnngaccaagactttcgcagcttccggtcagagtgtgaggctgaggtgggctggaacctgacc

SEQ ID NO: 760 - DNA, 101 bp, synthetic construct
  misc_feature 1..101: note = Oligonucleotide probe
  misc_feature 36..41: note = n is a, c, g, or t
  source 1..101: mol_type = other DNA
atgtgactggcacgggagttgatcctggttttcacnnnnnnagatgtacaaggcgtgcctcaagtaccccgagtggaaacagaagcacctgcctcacttca

SEQ ID NO: 761 - DNA, 101 bp, synthetic construct
  misc_feature 1..101: note = Oligonucleotide probe
  misc_feature 36..41: note = n is a, c, g, or t
  source 1..101: mol_type = other DNA
atgtgactggcacgggagttgatcctggttttcacnnnnnnttcagtgaagaattaaaagggcctgtgacagatgatgaagaagtggaaacatctgtgctc

SEQ ID NO: 762 - DNA, 100 bp, synthetic construct
  misc_feature 1..100: note = Oligonucleotide probe
  misc_feature 36..41: note = n is a, c, g, or t
  source 1..100: mol_type = other DNA
atgtgactggcacgggagttgatcctggttttcacnnnnnngaaaccaccttgcgtgggttcaagaagagtggaactccaggaaaaactggtggccaggc

SEQ ID NO: 763 - DNA, 101 bp, synthetic construct
  misc_feature 1..101: note = Oligonucleotide probe
  misc_feature 36..41: note = n is a, c, g, or t
  source 1..101: mol_type = other DNA
atgtgactggcacgggagttgatcctggttttcacnnnnnnctttggggtctattccagagagcgcaacaactgtccccaagatcctctcagaccgtctac

SEQ ID NO: 764 - DNA, 100 bp, synthetic construct
  misc_feature 1..100: note = Oligonucleotide probe
  misc_feature 36..41: note = n is a, c, g, or t
  source 1..100: mol_type = other DNA
atgtgactggcacgggagttgatcctggttttcacnnnnnnaggcctacccattcctgcacacaaaggaggacacttatgagaacctgcataaggtgctg

SEQ ID NO: 765 - DNA, 101 bp, synthetic construct
  misc_feature 1..101: note = Oligonucleotide probe
  misc_feature 36..41: note = n is a, c, g, or t
  source 1..101: mol_type = other DNA
atgtgactggcacgggagttgatcctggttttcacnnnnnnatcggttttggttatgcagccctcgtgacatttggaagcatttttggatataagcggaga

SEQ ID NO: 766 - DNA, 100 bp, synthetic construct
  misc_feature 1..100: note = Oligonucleotide probe
  misc_feature 36..41: note = n is a, c, g, or t
  source 1..100: mol_type = other DNA
atgtgactggcacgggagttgatcctggttttcacnnnnnngctttcttcctggctaccataatgggtgtgagatttaagaggtccaagaaaataatgcc

SEQ ID NO: 767 - DNA, 101 bp, synthetic construct
  misc_feature 1..101: note = Oligonucleotide probe
  misc_feature 36..41: note = n is a, c, g, or t
  source 1..101: mol_type = other DNA
atgtgactggcacgggagttgatcctggttttcacnnnnnncacaacctgtacctgtttgaccggaatggagtgtgtctgcactacagcgaatggcaccgc

SEQ ID NO: 768 - DNA, 100 bp, synthetic construct
  misc_feature 1..100: note = Oligonucleotide probe
  misc_feature 36..41: note = n is a, c, g, or t
  source 1..100: mol_type = other DNA
atgtgactggcacgggagttgatcctggttttcacnnnnnnatccgagatgtgctgcaccacatctacagtgcgctgtatgtggagctggtggtgaagaa

SEQ ID NO: 769 - DNA, 101 bp, synthetic construct; identical to SEQ ID NO: 727
  misc_feature 1..101: note = Oligonucleotide probe
  misc_feature 36..41: note = n is a, c, g, or t
  source 1..101: mol_type = other DNA

SEQ ID NO: 770 - DNA, 100 bp, synthetic construct; identical to SEQ ID NO: 728
  misc_feature 1..100: note = Oligonucleotide probe
  misc_feature 36..41: note = n is a, c, g, or t
  source 1..100: mol_type = other DNA

SEQ ID NO: 771 - DNA, 101 bp, synthetic construct; identical to SEQ ID NO: 729
  misc_feature 1..101: note = Oligonucleotide probe
  misc_feature 36..41: note = n is a, c, g, or t
  source 1..101: mol_type = other DNA

SEQ ID NO: 772 - DNA, 101 bp, synthetic construct; identical to SEQ ID NO: 730
  misc_feature 1..101: note = Oligonucleotide probe
  misc_feature 36..41: note = n is a, c, g, or t
  source 1..101: mol_type = other DNA

SEQ ID NO: 773 - DNA, 101 bp, synthetic construct; identical to SEQ ID NO: 731
  misc_feature 1..101: note = Oligonucleotide probe
  misc_feature 36..41: note = n is a, c, g, or t
  source 1..101: mol_type = other DNA

SEQ ID NO: 774 - DNA, 100 bp, synthetic construct; identical to SEQ ID NO: 732
  misc_feature 1..100: note = Oligonucleotide probe
  misc_feature 36..41: note = n is a, c, g, or t
  source 1..100: mol_type = other DNA

SEQ ID NO: 775 - DNA, 100 bp, synthetic construct; identical to SEQ ID NO: 733
  misc_feature 1..100: note = Oligonucleotide probe
  misc_feature 36..41: note = n is a, c, g, or t
  source 1..100: mol_type = other DNA

SEQ ID NO: 776 - DNA, 100 bp, synthetic construct; identical to SEQ ID NO: 734
  misc_feature 1..100: note = Oligonucleotide probe
  misc_feature 36..41: note = n is a, c, g, or t
  source 1..100: mol_type = other DNA

SEQ ID NO: 777 - DNA, 101 bp, synthetic construct; identical to SEQ ID NO: 735
  misc_feature 1..101: note = Oligonucleotide probe
  misc_feature 36..41: note = n is a, c, g, or t
  source 1..101: mol_type = other DNA

SEQ ID NO: 778 - DNA, 100 bp, synthetic construct; identical to SEQ ID NO: 736
  misc_feature 1..100: note = Oligonucleotide probe
  misc_feature 36..41: note = n is a, c, g, or t
  source 1..100: mol_type = other DNA

SEQ ID NO: 779 - DNA, 101 bp, synthetic construct; identical to SEQ ID NO: 737
  misc_feature 1..101: note = Oligonucleotide probe
  misc_feature 36..41: note = n is a, c, g, or t
  source 1..101: mol_type = other DNA

SEQ ID NO: 780 - DNA, 100 bp, synthetic construct; identical to SEQ ID NO: 738
  misc_feature 1..100: note = Oligonucleotide probe
  misc_feature 36..41: note = n is a, c, g, or t
  source 1..100: mol_type = other DNA

SEQ ID NO: 781 - DNA, 100 bp, synthetic construct; identical to SEQ ID NO: 739
  misc_feature 1..100: note = Oligonucleotide probe
  misc_feature 36..41: note = n is a, c, g, or t
  source 1..100: mol_type = other DNA

SEQ ID NO: 782 - DNA, 100 bp, synthetic construct; identical to SEQ ID NO: 740
  misc_feature 1..100: note = Oligonucleotide probe
  misc_feature 36..41: note = n is a, c, g, or t
  source 1..100: mol_type = other DNA

SEQ ID NO: 783 - DNA, 101 bp, synthetic construct; identical to SEQ ID NO: 741
  misc_feature 1..101: note = Oligonucleotide probe
  misc_feature 36..41: note = n is a, c, g, or t
  source 1..101: mol_type = other DNA

SEQ ID NO: 784 - DNA, 100 bp, synthetic construct; identical to SEQ ID NO: 742
  misc_feature 1..100: note = Oligonucleotide probe
  misc_feature 36..41: note = n is a, c, g, or t
  source 1..100: mol_type = other DNA

SEQ ID NO: 785 - DNA, 100 bp, synthetic construct; identical to SEQ ID NO: 743
  misc_feature 1..100: note = Oligonucleotide probe
  misc_feature 36..41: note = n is a, c, g, or t
  source 1..100: mol_type = other DNA

SEQ ID NO: 786 - DNA, 100 bp, synthetic construct; identical to SEQ ID NO: 744
  misc_feature 1..100: note = Oligonucleotide probe
  misc_feature 36..41: note = n is a, c, g, or t
  source 1..100: mol_type = other DNA

SEQ ID NO: 787 - DNA, 101 bp, synthetic construct; identical to SEQ ID NO: 745
  misc_feature 1..101: note = Oligonucleotide probe
  misc_feature 36..41: note = n is a, c, g, or t
  source 1..101: mol_type = other DNA

SEQ ID NO: 788 - DNA, 100 bp, synthetic construct; identical to SEQ ID NO: 746
  misc_feature 1..100: note = Oligonucleotide probe
  misc_feature 36..41: note = n is a, c, g, or t
  source 1..100: mol_type = other DNA

SEQ ID NO: 789 - DNA, 101 bp, synthetic construct; identical to SEQ ID NO: 747
  misc_feature 1..101: note = Oligonucleotide probe
  misc_feature 36..41: note = n is a, c, g, or t
  source 1..101: mol_type = other DNA

SEQ ID NO: 790 - DNA, 100 bp, synthetic construct; identical to SEQ ID NO: 748
  misc_feature 1..100: note = Oligonucleotide probe
  misc_feature 36..41: note = n is a, c, g, or t
  source 1..100: mol_type = other DNA

SEQ ID NO: 791 - DNA, 101 bp, synthetic construct; identical to SEQ ID NO: 749
  misc_feature 1..101: note = Oligonucleotide probe
  misc_feature 36..41: note = n is a, c, g, or t
  source 1..101: mol_type = other DNA

SEQ ID NO: 792 - DNA, 100 bp, synthetic construct; identical to SEQ ID NO: 750
  misc_feature 1..100: note = Oligonucleotide probe
  misc_feature 36..41: note = n is a, c, g, or t
  source 1..100: mol_type = other DNA

SEQ ID NO: 793 - DNA, 101 bp, synthetic construct; identical to SEQ ID NO: 751
  misc_feature 1..101: note = Oligonucleotide probe
  misc_feature 36..41: note = n is a, c, g, or t
  source 1..101: mol_type = other DNA

SEQ ID NO: 794 - DNA, 100 bp, synthetic construct; identical to SEQ ID NO: 752
  misc_feature 1..100: note = Oligonucleotide probe
  misc_feature 36..41: note = n is a, c, g, or t
  source 1..100: mol_type = other DNA

SEQ ID NO: 795 - DNA, 100 bp, synthetic construct; identical to SEQ ID NO: 753
  misc_feature 1..100: note = Oligonucleotide probe
  misc_feature 36..41: note = n is a, c, g, or t
  source 1..100: mol_type = other DNA

SEQ ID NO: 796 - DNA, 101 bp, synthetic construct; identical to SEQ ID NO: 754
  misc_feature 1..101: note = Oligonucleotide probe
  misc_feature 36..41: note = n is a, c, g, or t
  source 1..101: mol_type = other DNA

SEQ ID NO: 797 - DNA, 100 bp, synthetic construct; identical to SEQ ID NO: 755
  misc_feature 1..100: note = Oligonucleotide probe
  misc_feature 36..41: note = n is a, c, g, or t
  source 1..100: mol_type = other DNA

SEQ ID NO: 798 - DNA, 100 bp, synthetic construct; identical to SEQ ID NO: 756
  misc_feature 1..100: note = Oligonucleotide probe
  misc_feature 36..41: note = n is a, c, g, or t
  source 1..100: mol_type = other DNA

SEQ ID NO: 799 - DNA, 100 bp, synthetic construct; identical to SEQ ID NO: 757
  misc_feature 1..100: note = Oligonucleotide probe
  misc_feature 36..41: note = n is a, c, g, or t
  source 1..100: mol_type = other DNA

SEQ ID NO: 800 - DNA, 100 bp, synthetic construct; identical to SEQ ID NO: 758
  misc_feature 1..100: note = Oligonucleotide probe
  misc_feature 36..41: note = n is a, c, g, or t
  source 1..100: mol_type = other DNA

SEQ ID NO: 801 - DNA, 101 bp, synthetic construct; identical to SEQ ID NO: 759
  misc_feature 1..101: note = Oligonucleotide probe
  misc_feature 36..41: note = n is a, c, g, or t
  source 1..101: mol_type = other DNA

SEQ ID NO: 802 - DNA, 101 bp, synthetic construct; identical to SEQ ID NO: 760
  misc_feature 1..101: note = Oligonucleotide probe
  misc_feature 36..41: note = n is a, c, g, or t
  source 1..101: mol_type = other DNA

SEQ ID NO: 803 - DNA, 101 bp, synthetic construct; identical to SEQ ID NO: 761
  misc_feature 1..101: note = Oligonucleotide probe
  misc_feature 36..41: note = n is a, c, g, or t
  source 1..101: mol_type = other DNA

SEQ ID NO: 804 - DNA, 100 bp, synthetic construct; identical to SEQ ID NO: 762
  misc_feature 1..100: note = Oligonucleotide probe
  misc_feature 36..41: note = n is a, c, g, or t
  source 1..100: mol_type = other DNA

SEQ ID NO: 805 - DNA, 101 bp, synthetic construct; identical to SEQ ID NO: 763
  misc_feature 1..101: note = Oligonucleotide probe
  misc_feature 36..41: note = n is a, c, g, or t
  source 1..101: mol_type = other DNA

SEQ ID NO: 806 - DNA, 100 bp, synthetic construct; identical to SEQ ID NO: 764
  misc_feature 1..100: note = Oligonucleotide probe
  misc_feature 36..41: note = n is a, c, g, or t
  source 1..100: mol_type = other DNA

SEQ ID NO: 807 - DNA, 101 bp, synthetic construct; identical to SEQ ID NO: 765
  misc_feature 1..101: note = Oligonucleotide probe
  misc_feature 36..41: note = n is a, c, g, or t
  source 1..101: mol_type = other DNA

SEQ ID NO: 808 - DNA, 100 bp, synthetic construct; identical to SEQ ID NO: 766
  misc_feature 1..100: note = Oligonucleotide probe
  misc_feature 36..41: note = n is a, c, g, or t
  source 1..100: mol_type = other DNA

SEQ ID NO: 809 - DNA, 101 bp, synthetic construct; identical to SEQ ID NO: 767
  misc_feature 1..101: note = Oligonucleotide probe
  misc_feature 36..41: note = n is a, c, g, or t
  source 1..101: mol_type = other DNA

SEQ ID NO: 810 - DNA, 100 bp, synthetic construct; identical to SEQ ID NO: 768
  misc_feature 1..100: note = Oligonucleotide probe
  misc_feature 36..41: note = n is a, c, g, or t
  source 1..100: mol_type = other DNA